European Patent Specification EP 3 495 487 B1, published April 29, 2026. Title: PROMOTER WITH A REGION RICH IN CYTOSINE-GUANINE DINUCLEOTIDES, VECTORS, CELLULAR LINES, METHOD FOR PRODUCING RECOMBINANT PROTEIN. Applicant: UNIVERSIDAD DE CHILE BPH S.A. INGENIERIA ORBICORP LTDA. Application EP 17818793.6. The sequence listing filed with the application follows.

SEQUENCE LISTING (45 sequences)

SEQ ID NO: 1 - DNA, 5599 bp, Artificial Sequence
  Plasmid
ggcctaactggccggtacctgagctcgctagcctcgaggatatcaagatctggcctcggcggccaagcttggcaatccggtactgttggtaaagccaccatggaagatgccaaaaacattaagaagggcccagcgccattctacccactcgaagacgggaccgccggcgagcagctgcacaaagccatgaagcgctacgccctggtgcccggcaccatcgcctttaccgacgcacatatcgaggtggacattacctacgccgagtacttcgagatgagcgttcggctggcagaagctatgaagcgctatgggctgaatacaaaccatcggatcgtggtgtgcagcgagaatagcttgcagttcttcatgcccgtgttgggtgccctgttcatcggtgtggctgtggccccagctaacgacatctacaacgagcgcgagctgctgaacagcatgggcatcagccagcccaccgtcgtattcgtgagcaagaaagggctgcaaaagatcctcaacgtgcaaaagaagctaccgatcatacaaaagatcatcatcatggatagcaagaccgactaccagggcttccaaagcatgtacaccttcgtgacttcccatttgccacccggcttcaacgagtacgacttcgtgcccgagagcttcgaccgggacaaaaccatcgccctgatcatgaacagtagtggcagtaccggattgcccaagggcgtagccctaccgcaccgcaccgcttgtgtccgattcagtcatgcccgcgaccccatcttcggcaaccagatcatccccgacaccgctatcctcagcgtggtgccatttcaccacggcttcggcatgttcaccacgctgggctacttgatctgcggctttcgggtcgtgctcatgtaccgcttcgaggaggagctattcttgcgcagcttgcaagactataagattcaatctgccctgctggtgcccacactatttagcttcttcgctaagagcactctcatcgacaagtacgacctaagcaacttgcacgagatcgccagcggcggggcgccgctcagcaaggaggtaggtgaggccgtggccaaacgcttccacctaccaggcatccgccagggctacggcctgacagaaacaaccagcgccattctgatcacccccgaaggggacgacaagcctggcgcagtaggcaaggtggtgcccttcttcgaggctaaggtggtggacttggacaccggtaagacactgggtgtgaaccagcgcggcgagctgtgcgtccgtggccccatgatcatgagcggctacgttaacaaccccgaggctacaaacgctctcatcgacaaggacggctggctgcacagcggcgacatcgcctactgggacgaggacgagcacttcttcatcgtggaccggctgaagagcctgatcaaatacaagggctaccaggtagccccagccgaactggagagcatcctgctgcaacaccccaacatcttcgacgccggggtcgccggcctgcccgacgacgatgccggcgagctgcccgccgcagtcgtcgtgctggaacacggtaaaaccatgaccgagaaggagatcgtggactatgtggccagccaggttacaaccgccaagaagctgcgcggtggtgttgtgttcgtggacgaggtgcctaaaggactgaccggcaagttggacgcccgcaagatccgcgagattctcattaaggccaagaagggcggcaagatcgccgtgtaataattctagagtcggggcggccggccgcttcgagcagacatgataagatacattgatgagtttggacaaaccacaactagaatgcagtgaaaaaaatgctttatttgtgaaatttgtgatgctattgctttatttgtaaccattataagctgcaataaacaagttaacaacaacaattgcattcattttatgtttcaggttcagggggaggtgtgggaggttttttaaagcaagtaaaacctctacaaatgtggtaaaatcgataaggatccgtttgcgtattgggcgctcttccgctgatctgcgcagcaccatggcctgaaataacctctgaaagaggaacttggttagctaccttctgaggcggaaagaaccagctgtggaatgtgtgtcagttagggtgtggaaagtccccaggctccccagcaggcagaagtatgcaaagcatgcatctcaattagtcagcaaccaggtgtggaaagtccccaggctccccagcaggcagaagtatgcaaagcatgcatctcaattagtcagcaaccatagtcccgcccctaactccgcccatcccgcccctaactccgcccagttccgcccattctccgccccatggctgactaattttttttatttatgcagaggccgaggccgcctctgcctctgagctattccagaagtagtgaggaggcttttttggaggcctaggcttttgcaaaaagctcgattcttctgacactagcgccaccatgatcgaacaagacggcctccatgctggcagtcccgcagcttgggtcgaacgcttgttcgggtacgactgggcccagcagaccatcggatgtagcgatgcggccgtgttccgtctaagcgctcaaggccggcccgtgctgttcgtgaagaccgacctgagcggcgccctgaacgagcttcaagacgaggctgcccgcctgagctggctggccaccaccggcgtaccctgcgccgctgtgttggatgttgtgaccgaagccggccgggactggctgctgctgggcgaggtccctggccaggatctgctgagcagccaccttgcccccgctgagaaggtttctatcatggccgatgcaatgcggcgcctgcacaccctggaccccgctacctgccccttcgaccaccaggctaagcatcggatcgagcgtgctcggacccgcatggaggccggcctggtggaccaggacgacctggacgaggagcatcagggcctggcccccgctgaactgttcgcccgactgaaagcccgcatgccggacggtgaggacctggttgtcacacacggagatgcctgcctccctaacatcatggtcgagaatggccgcttctccggcttcatcgactgcggtcgcctaggagttgccgaccgctaccaggacatcgccctggccacccgcgacatcgctgaggagcttggcggcgagtgggccgaccgcttcttagtcttgtacggcatcgcagctcccgacagccagcgcatcgccttctaccgcttgctcgacgagttcttttaatgatctagaaccggtcatggccgcaataaaatatctttattttcattacatctgtgtgttggttttttgtgtgttcgaactagatgctgtcgaccgatgcccttgagagccttcaacccagtcagctccttccggtgggcgcggggcatgactatcgtcgccgcacttatgactgtcttctttatcatgcaactcgtaggacaggtgccggcagcgctcttccgcttcctcgctcactgactcgctgcgctcggtcgttcggctgcggcgagcggtatcagctcactcaaaggcggtaatacggttatccacagaatcaggggataacgcaggaaagaacatgtgagcaaaaggccagcaaaaggccaggaaccgtaaaaaggccgcgttgctggcgtttttccataggctccgcccccctgacgagcatcacaaaaatcgacgctcaagtcagaggtggcgaaacccgacaggactataaagataccaggcgtttccccctggaagctccctcgtgcgctctcctgttccgaccctgccgcttaccggatacctgtccgcctttctcccttcgggaagcgtggcgctttctcatagctcacgctgtaggtatctcagttcggtgtaggtcgttcgctccaagctgggctgtgtgcacgaaccccccgttcagcccgaccgctgcgccttatccggtaactatcgtcttgagtccaacccggtaagacacgacttatcgccactggcagcagccactggtaacaggattagcagagcgaggtatgtaggcggtgctacagagttcttgaagtggtggcctaactacggctacactagaagaacagtatttggtatctgcgctctgctgaagccagttaccttcggaaaaagagttggtagctcttgatccggcaaacaaaccaccgctggtagcggtggtttttttgtttgcaagcagcagattacgcgcagaaaaaaaggatctcaagaagatcctttgatcttttctacggggtctgacgctcagtggaacgaaaactcacgttaagggattttggtcatgagattatcaaaaaggatcttcacctagatccttttaaattaaaaatgaagttttaaatcaatctaaagtatatatgagtaaacttggtctgacagcggccgcaaatgctaaaccactgcagtggttaccagtgcttgatcagtgaggcaccgatctcagcgatctgcctatttcgttcgtccatagtggcctgactccccgtcgtgtagatcactacgattcgtgagggcttaccatcaggccccagcgcagcaatgatgccgcgagagccgcgttcaccggcccccgatttgtcagcaatgaaccagccagcagggagggccgagcgaagaagtggtcctgctactttgtccgcctccatccagtctatgagctgctgtcgtgatgctagagtaagaagttcgccagtgagtagtttccgaagagttgtggccattgctactggcatcgtggtatcacgctcgtcgttcggtatggcttcgttcaactctggttcccagcggtcaagccgggtcacatgatcacccatattatgaagaaatgcagtcagctccttagggcctccgatcgttgtcagaagtaagttggccgcggtgttgtcgctcatggtaatggcagcactacacaattctcttaccgtcatgccatccgtaagatgcttttccgtgaccggcgagtactcaaccaagtcgttttgtgagtagtgtatacggcgaccaagctgctcttgcccggcgtctatacgggacaacaccgcgccacatagcagtactttgaaagtgctcatcatcgggaatcgttcttcggggcggaaagactcaaggatcttgccgctattgagatccagttcgatatagcccactcttgcacccagttgatcttcagcatcttttactttcaccagcgtttcggggtgtgcaaaaacaggcaagcaaaatgccgcaaagaagggaatgagtgcgacacgaaaatgttggatgctcatactcgtcctttttcaatattattgaagcatttatcagggttactagtacgtctctcaaggataagtaagtaatattaaggtacgggaggtattggacaggccgcaataaaatatctttattttcattacatctgtgtgttggttttttgtgtgaatcgatagtactaacatacgctctccatcaaaacaaaacgaaacaaaacaaactagcaaaataggctgtccccagtgcaagtgcaggtgccagaacatttctct

SEQ ID NO: 2 - DNA, 6214 bp, Artificial Sequence
  Plasmid
ggcctaactggccggtacctgagctcgctagcctcgaggatatcaagatctgttgacattgattattgactagttattaatagtaatcaattacggggtcattagttcatagcccatatatggagttccgcgttacataacttacggtaaatggcccgcctggctgaccgcccaacgacccccgcccattgacgtcaataatgacgtatgttcccatagtaacgccaatagggactttccattgacgtcaatgggtggagtatttacggtaaactgcccacttggcagtacatcaagtgtatcatatgccaagtacgccccctattgacgtcaatgacggtaaatggcccgcctggcattatgcccagtacatgaccttatgggactttcctacttggcagtacatctacgtattagtcatcgctattaccatggtgatgcggttttggcagtacatcaatgggcgtggatagcggtttgactcacggggatttccaagtctccaccccattgacgtcaatgggagtttgttttggcaccaaaatcaacgggactttccaaaatgtcgtaacaactccgccccattgacgcaaatgggcggtaggcgtgtacggtgggaggtctatataagcagagctctctggctaactagagaacccactgcttactggcttatcgaaagcttggcaatccggtactgttggtaaagccaccatggaagatgccaaaaacattaagaagggcccagcgccattctacccactcgaagacgggaccgccggcgagcagctgcacaaagccatgaagcgctacgccctggtgcccggcaccatcgcctttaccgacgcacatatcgaggtggacattacctacgccgagtacttcgagatgagcgttcggctggcagaagctatgaagcgctatgggctgaatacaaaccatcggatcgtggtgtgcagcgagaatagcttgcagttcttcatgcccgtgttgggtgccctgttcatcggtgtggctgtggccccagctaacgacatctacaacgagcgcgagctgctgaacagcatgggcatcagccagcccaccgtcgtattcgtgagcaagaaagggctgcaaaagatcctcaacgtgcaaaagaagctaccgatcatacaaaagatcatcatcatggatagcaagaccgactaccagggcttccaaagcatgtacaccttcgtgacttcccatttgccacccggcttcaacgagtacgacttcgtgcccgagagcttcgaccgggacaaaaccatcgccctgatcatgaacagtagtggcagtaccggattgcccaagggcgtagccctaccgcaccgcaccgcttgtgtccgattcagtcatgcccgcgaccccatcttcggcaaccagatcatccccgacaccgctatcctcagcgtggtgccatttcaccacggcttcggcatgttcaccacgctgggctacttgatctgcggctttcgggtcgtgctcatgtaccgcttcgaggaggagctattcttgcgcagcttgcaagactataagattcaatctgccctgctggtgcccacactatttagcttcttcgctaagagcactctcatcgacaagtacgacctaagcaacttgcacgagatcgccagcggcggggcgccgctcagcaaggaggtaggtgaggccgtggccaaacgcttccacctaccaggcatccgccagggctacggcctgacagaaacaaccagcgccattctgatcacccccgaaggggacgacaagcctggcgcagtaggcaaggtggtgcccttcttcgaggctaaggtggtggacttggacaccggtaagacactgggtgtgaaccagcgcggcgagctgtgcgtccgtggccccatgatcatgagcggctacgttaacaaccccgaggctacaaacgctctcatcgacaaggacggctggctgcacagcggcgacatcgcctactgggacgaggacgagcacttcttcatcgtggaccggctgaagagcctgatcaaatacaagggctaccaggtagccccagccgaactggagagcatcctgctgcaacaccccaacatcttcgacgccggggtcgccggcctgcccgacgacgatgccggcgagctgcccgccgcagtcgtcgtgctggaacacggtaaaaccatgaccgagaaggagatcgtggactatgtggccagccaggttacaaccgccaagaagctgcgcggtggtgttgtgttcgtggacgaggtgcctaaaggactgaccggcaagttggacgcccgcaagatccgcgagattctcattaaggccaagaagggcggcaagatcgccgtgtaataattctagagtcggggcggccggccgcttcgagcagacatgataagatacattgatgagtttggacaaaccacaactagaatgcagtgaaaaaaatgctttatttgtgaaatttgtgatgctattgctttatttgtaaccattataagctgcaataaacaagttaacaacaacaattgcattcattttatgtttcaggttcagggggaggtgtgggaggttttttaaagcaagtaaaacctctacaaatgtggtaaaatcgataaggatccgtttgcgtattgggcgctcttccgctgatctgcgcagcaccatggcctgaaataacctctgaaagaggaacttggttagctaccttctgaggcggaaagaaccagctgtggaatgtgtgtcagttagggtgtggaaagtccccaggctccccagcaggcagaagtatgcaaagcatgcatctcaattagtcagcaaccaggtgtggaaagtccccaggctccccagcaggcagaagtatgcaaagcatgcatctcaattagtcagcaaccatagtcccgcccctaactccgcccatcccgcccctaactccgcccagttccgcccattctccgccccatggctgactaattttttttatttatgcagaggccgaggccgcctctgcctctgagctattccagaagtagtgaggaggcttttttggaggcctaggcttttgcaaaaagctcgattcttctgacactagcgccaccatgatcgaacaagacggcctccatgctggcagtcccgcagcttgggtcgaacgcttgttcgggtacgactgggcccagcagaccatcggatgtagcgatgcggccgtgttccgtctaagcgctcaaggccggcccgtgctgttcgtgaagaccgacctgagcggcgccctgaacgagcttcaagacgaggctgcccgcctgagctggctggccaccaccggcgtaccctgcgccgctgtgttggatgttgtgaccgaagccggccgggactggctgctgctgggcgaggtccctggccaggatctgctgagcagccaccttgcccccgctgagaaggtttctatcatggccgatgcaatgcggcgcctgcacaccctggaccccgctacctgccccttcgaccaccaggctaagcatcggatcgagcgtgctcggacccgcatggaggccggcctggtggaccaggacgacctggacgaggagcatcagggcctggcccccgctgaactgttcgcccgactgaaagcccgcatgccggacggtgaggacctggttgtcacacacggagatgcctgcctccctaacatcatggtcgagaatggccgcttctccggcttcatcgactgcggtcgcctaggagttgccgaccgctaccaggacatcgccctggccacccgcgacatcgctgaggagcttggcggcgagtgggccgaccgcttcttagtcttgtacggcatcgcagctcccgacagccagcgcatcgccttctaccgcttgctcgacgagttcttttaatgatctagaaccggtcatggccgcaataaaatatctttattttcattacatctgtgtgttggttttttgtgtgttcgaactagatgctgtcgaccgatgcccttgagagccttcaacccagtcagctccttccggtgggcgcggggcatgactatcgtcgccgcacttatgactgtcttctttatcatgcaactcgtaggacaggtgccggcagcgctcttccgcttcctcgctcactgactcgctgcgctcggtcgttcggctgcggcgagcggtatcagctcactcaaaggcggtaatacggttatccacagaatcaggggataacgcaggaaagaacatgtgagcaaaaggccagcaaaaggccaggaaccgtaaaaaggccgcgttgctggcgtttttccataggctccgcccccctgacgagcatcacaaaaatcgacgctcaagtcagaggtggcgaaacccgacaggactataaagataccaggcgtttccccctggaagctccctcgtgcgctctcctgttccgaccctgccgcttaccggatacctgtccgcctttctcccttcgggaagcgtggcgctttctcatagctcacgctgtaggtatctcagttcggtgtaggtcgttcgctccaagctgggctgtgtgcacgaaccccccgttcagcccgaccgctgcgccttatccggtaactatcgtcttgagtccaacccggtaagacacgacttatcgccactggcagcagccactggtaacaggattagcagagcgaggtatgtaggcggtgctacagagttcttgaagtggtggcctaactacggctacactagaagaacagtatttggtatctgcgctctgctgaagccagttaccttcggaaaaagagttggtagctcttgatccggcaaacaaaccaccgctggtagcggtggtttttttgtttgcaagcagcagattacgcgcagaaaaaaaggatctcaagaagatcctttgatcttttctacggggtctgacgctcagtggaacgaaaactcacgttaagggattttggtcatgagattatcaaaaaggatcttcacctagatccttttaaattaaaaatgaagttttaaatcaatctaaagtatatatgagtaaacttggtctgacagcggccgcaaatgctaaaccactgcagtggttaccagtgcttgatcagtgaggcaccgatctcagcgatctgcctatttcgttcgtccatagtggcctgactccccgtcgtgtagatcactacgattcgtgagggcttaccatcaggccccagcgcagcaatgatgccgcgagagccgcgttcaccggcccccgatttgtcagcaatgaaccagccagcagggagggccgagcgaagaagtggtcctgctactttgtccgcctccatccagtctatgagctgctgtcgtgatgctagagtaagaagttcgccagtgagtagtttccgaagagttgtggccattgctactggcatcgtggtatcacgctcgtcgttcggtatggcttcgttcaactctggttcccagcggtcaagccgggtcacatgatcacccatattatgaagaaatgcagtcagctccttagggcctccgatcgttgtcagaagtaagttggccgcggtgttgtcgctcatggtaatggcagcactacacaattctcttaccgtcatgccatccgtaagatgcttttccgtgaccggcgagtactcaaccaagtcgttttgtgagtagtgtatacggcgaccaagctgctcttgcccggcgtctatacgggacaacaccgcgccacatagcagtactttgaaagtgctcatcatcgggaatcgttcttcggggcggaaagactcaaggatcttgccgctattgagatccagttcgatatagcccactcttgcacccagttgatcttcagcatcttttactttcaccagcgtttcggggtgtgcaaaaacaggcaagcaaaatgccgcaaagaagggaatgagtgcgacacgaaaatgttggatgctcatactcgtcctttttcaatattattgaagcatttatcagggttactagtacgtctctcaaggataagtaagtaatattaaggtacgggaggtattggacaggccgcaataaaatatctttattttcattacatctgtgtgttggttttttgtgtgaatcgatagtactaacatacgctctccatcaaaacaaaacgaaacaaaacaaactagcaaaataggctgtccccagtgcaagtgcaggtgccagaacatttctct

SEQ ID NO: 3 - DNA, 628 bp, Artificial Sequence
  Plasmid
gttgacattgattattgactagttattaatagtaatcaattacggggtcattagttcatagcccatatatggagttccgcgttacataacttacggtaaatggcccgcctggctgaccgcccaacgacccccgcccattgacgtcaataatgacgtatgttcccatagtaacgccaatagggactttccattgacgtcaatgggtggagtatttacggtaaactgcccacttggcagtacatcaagtgtatcatatgccaagtacgccccctattgacgtcaatgacggtaaatggcccgcctggcattatgcccagtacatgaccttatgggactttcctacttggcagtacatctacgtattagtcatcgctattaccatggtgatgcggttttggcagtacatcaatgggcgtggatagcggtttgactcacggggatttccaagtctccaccccattgacgtcaatgggagtttgttttggcaccaaaatcaacgggactttccaaaatgtcgtaacaactccgccccattgacgcaaatgggcggtaggcgtgtacggtgggaggtctatataagcagagctctctggctaactagagaacccactgcttactggcttatcga

SEQ ID NO: 4 - DNA, 7376 bp, Artificial Sequence
  Plasmid
ggcctaactggccggtaccggagagggggtaaaaaaatgctgcactgtgcggctaggccggtgagtgagcggcgcggagccaatcagcgctcgccgttccgaaagttgccttttatggctcgagtggccgctgtggcgtcctataaaacccggcggcgcaacgcgcagccactgtcgagtccgcgtccacccgcgagcacaggcctttcgcagctctttcttcgccgctccacacccgccaccaggtaagcagggacaacaggcccagccggccacagccctcccgtgggcagtgaccgcgctgcagggtcgcgggggacactcggcgcggacaccggggaaggctggagggtggtgccgggccgcggagcggacactttcagatccaactttcagtccagggtgtagaccctttacagccgcattgccacggtgtagacaccggtggacccgctctggctcagagcacgcggcttgggggaacccattagggtcgcagtgtgggcgctatgagagccgatgcagctttcgggtgttgaaccgtatctgcccaccttggggggaggacacaaggtcgggagccaaacgccacgatcatgccttggtggcccatgggtctttgtctaaaccggtttgcccatttggcttgccgggcgggcgggcgcggcgggcccggctcggccgggttgggggctgggttgccactgcgcttgcgcgctctatggctgggtattggggcgcgtgcacgctggggagggagcccttcctcttccccctctcccaagttaaacttgcgcgtgcgtattgagacttggagcgcggccaccggggttgggcgagggcggggccgttgtccggaaggggcggggtcgcagcggcttcggggcgcctgctcgcgcttcctgctgggtgtggtcgcctcccgcgcgcgcactagccgcccgccggcggggcgaaggcggggcttgcgcccgtttggggagggggcggaggcctggcttcctgccgtggggccgcctccggaccagcgtttgcctcttatggtaataacgcggccggcctgggcttcctttgtcccctgagtttgggcgcgcgccccctggcggcccgaggccgcggcttgccggaagtgggcagggcggcagcggctgcgcctagtggcccgccagtgaccgcgaccctcttttgtgccctgatatagttcgccagatctgttgacattgattattgactagttattaatagtaatcaattacggggtcattagttcatagcccatatatggagttccgcgttacataacttacggtaaatggcccgcctggctgaccgcccaacgacccccgcccattgacgtcaataatgacgtatgttcccatagtaacgccaatagggactttccattgacgtcaatgggtggagtatttacggtaaactgcccacttggcagtacatcaagtgtatcatatgccaagtacgccccctattgacgtcaatgacggtaaatggcccgcctggcattatgcccagtacatgaccttatgggactttcctacttggcagtacatctacgtattagtcatcgctattaccatggtgatgcggttttggcagtacatcaatgggcgtggatagcggtttgactcacggggatttccaagtctccaccccattgacgtcaatgggagtttgttttggcaccaaaatcaacgggactttccaaaatgtcgtaacaactccgccccattgacgcaaatgggcggtaggcgtgtacggtgggaggtctatataagcagagctctctggctaactagagaacccactgcttactggcttatcgaaagcttggcaatccggtactgttggtaaagccaccatggaagatgccaaaaacattaagaagggcccagcgccattctacccactcgaagacgggaccgccggcgagcagctgcacaaagccatgaagcgctacgccctggtgcccggcaccatcgcctttaccgacgcacatatcgaggtggacattacctacgccgagtacttcgagatgagcgttcggctggcagaagctatgaagcgctatgggctgaatacaaaccatcggatcgtggtgtgcagcgagaatagcttgcagttcttcatgcccgtgttgggtgccctgttcatcggtgtggctgtggccccagctaacgacatctacaacgagcgcgagctgctgaacagcatgggcatcagccagcccaccgtcgtattcgtgagcaagaaagggctgcaaaagatcctcaacgtgcaaaagaagctaccgatcatacaaaagatcatcatcatggatagcaagaccgactaccagggcttccaaagcatgtacaccttcgtgacttcccatttgccacccggcttcaacgagtacgacttcgtgcccgagagcttcgaccgggacaaaaccatcgccctgatcatgaacagtagtggcagtaccggattgcccaagggcgtagccctaccgcaccgcaccgcttgtgtccgattcagtcatgcccgcgaccccatcttcggcaaccagatcatccccgacaccgctatcctcagcgtggtgccatttcaccacggcttcggcatgttcaccacgctgggctacttgatctgcggctttcgggtcgtgctcatgtaccgcttcgaggaggagctattcttgcgcagcttgcaagactataagattcaatctgccctgctggtgcccacactatttagcttcttcgctaagagcactctcatcgacaagtacgacctaagcaacttgcacgagatcgccagcggcggggcgccgctcagcaaggaggtaggtgaggccgtggccaaacgcttccacctaccaggcatccgccagggctacggcctgacagaaacaaccagcgccattctgatcacccccgaaggggacgacaagcctggcgcagtaggcaaggtggtgcccttcttcgaggctaaggtggtggacttggacaccggtaagacactgggtgtgaaccagcgcggcgagctgtgcgtccgtggccccatgatcatgagcggctacgttaacaaccccgaggctacaaacgctctcatcgacaaggacggctggctgcacagcggcgacatcgcctactgggacgaggacgagcacttcttcatcgtggaccggctgaagagcctgatcaaatacaagggctaccaggtagccccagccgaactggagagcatcctgctgcaacaccccaacatcttcgacgccggggtcgccggcctgcccgacgacgatgccggcgagctgcccgccgcagtcgtcgtgctggaacacggtaaaaccatgaccgagaaggagatcgtggactatgtggccagccaggttacaaccgccaagaagctgcgcggtggtgttgtgttcgtggacgaggtgcctaaaggactgaccggcaagttggacgcccgcaagatccgcgagattctcattaaggccaagaagggcggcaagatcgccgtgtaataattctagagtcggggcggccggccgcttcgagcagacatgataagatacattgatgagtttggacaaaccacaactagaatgcagtgaaaaaaatgctttatttgtgaaatttgtgatgctattgctttatttgtaaccattataagctgcaataaacaagttaacaacaacaattgcattcattttatgtttcaggttcagggggaggtgtgggaggttttttaaagcaagtaaaacctctacaaatgtggtaaaatcgataaggatccgtttgcgtattgggcgctcttccgctgatctgcgcagcaccatggcctgaaataacctctgaaagaggaacttggttagctaccttctgaggcggaaagaaccagctgtggaatgtgtgtcagttagggtgtggaaagtccccaggctccccagcaggcagaagtatgcaaagcatgcatctcaattagtcagcaaccaggtgtggaaagtccccaggctccccagcaggcagaagtatgcaaagcatgcatctcaattagtcagcaaccatagtcccgcccctaactccgcccatcccgcccctaactccgcccagttccgcccattctccgccccatggctgactaattttttttatttatgcagaggccgaggccgcctctgcctctgagctattccagaagtagtgaggaggcttttttggaggcctaggcttttgcaaaaagctcgattcttctgacactagcgccaccatgatcgaacaagacggcctccatgctggcagtcccgcagcttgggtcgaacgcttgttcgggtacgactgggcccagcagaccatcggatgtagcgatgcggccgtgttccgtctaagcgctcaaggccggcccgtgctgttcgtgaagaccgacctgagcggcgccctgaacgagcttcaagacgaggctgcccgcctgagctggctggccaccaccggcgtaccctgcgccgctgtgttggatgttgtgaccgaagccggccgggactggctgctgctgggcgaggtccctggccaggatctgctgagcagccaccttgcccccgctgagaaggtttctatcatggccgatgcaatgcggcgcctgcacaccctggaccccgctacctgccccttcgaccaccaggctaagcatcggatcgagcgtgctcggacccgcatggaggccggcctggtggaccaggacgacctggacgaggagcatcagggcctggcccccgctgaactgttcgcccgactgaaagcccgcatgccggacggtgaggacctggttgtcacacacggagatgcctgcctccctaacatcatggtcgagaatggccgcttctccggcttcatcgactgcggtcgcctaggagttgccgaccgctaccaggacatcgccctggccacccgcgacatcgctgaggagcttggcggcgagtgggccgaccgcttcttagtcttgtacggcatcgcagctcccgacagccagcgcatcgccttctaccgcttgctcgacgagttcttttaatgatctagaaccggtcatggccgcaataaaatatctttattttcattacatctgtgtgttggttttttgtgtgttcgaactagatgctgtcgaccgatgcccttgagagccttcaacccagtcagctccttccggtgggcgcggggcatgactatcgtcgccgcacttatgactgtcttctttatcatgcaactcgtaggacaggtgccggcagcgctcttccgcttcctcgctcactgactcgctgcgctcggtcgttcggctgcggcgagcggtatcagctcactcaaaggcggtaatacggttatccacagaatcaggggataacgcaggaaagaacatgtgagcaaaaggccagcaaaaggccaggaaccgtaaaaaggccgcgttgctggcgtttttccataggctccgcccccctgacgagcatcacaaaaatcgacgctcaagtcagaggtggcgaaacccgacaggactataaagataccaggcgtttccccctggaagctccctcgtgcgctctcctgttccgaccctgccgcttaccggatacctgtccgcctttctcccttcgggaagcgtggcgctttctcatagctcacgctgtaggtatctcagttcggtgtaggtcgttcgctccaagctgggctgtgtgcacgaaccccccgttcagcccgaccgctgcgccttatccggtaactatcgtcttgagtccaacccggtaagacacgacttatcgccactggcagcagccactggtaacaggattagcagagcgaggtatgtaggcggtgctacagagttcttgaagtggtggcctaactacggctacactagaagaacagtatttggtatctgcgctctgctgaagccagttaccttcggaaaaagagttggtagctcttgatccggcaaacaaaccaccgctggtagcggtggtttttttgtttgcaagcagcagattacgcgcagaaaaaaaggatctcaagaagatcctttgatcttttctacggggtctgacgctcagtggaacgaaaactcacgttaagggattttggtcatgagattatcaaaaaggatcttcacctagatccttttaaattaaaaatgaagttttaaatcaatctaaagtatatatgagtaaacttggtctgacagcggccgcaaatgctaaaccactgcagtggttaccagtgcttgatcagtgaggcaccgatctcagcgatctgcctatttcgttcgtccatagtggcctgactccccgtcgtgtagatcactacgattcgtgagggcttaccatcaggccccagcgcagcaatgatgccgcgagagccgcgttcaccggcccccgatttgtcagcaatgaaccagccagcagggagggccgagcgaagaagtggtcctgctactttgtccgcctccatccagtctatgagctgctgtcgtgatgctagagtaagaagttcgccagtgagtagtttccgaagagttgtggccattgctactggcatcgtggtatcacgctcgtcgttcggtatggcttcgttcaactctggttcccagcggtcaagccgggtcacatgatcacccatattatgaagaaatgcagtcagctccttagggcctccgatcgttgtcagaagtaagttggccgcggtgttgtcgctcatggtaatggcagcactacacaattctcttaccgtcatgccatccgtaagatgcttttccgtgaccggcgagtactcaaccaagtcgttttgtgagtagtgtatacggcgaccaagctgctcttgcccggcgtctatacgggacaacaccgcgccacatagcagtactttgaaagtgctcatcatcgggaatcgttcttcggggcggaaagactcaaggatcttgccgctattgagatccagttcgatatagcccactcttgcacccagttgatcttcagcatcttttactttcaccagcgtttcggggtgtgcaaaaacaggcaagcaaaatgccgcaaagaagggaatgagtgcgacacgaaaatgttggatgctcatactcgtcctttttcaatattattgaagcatttatcagggttactagtacgtctctcaaggataagtaagtaatattaaggtacgggaggtattggacaggccgcaataaaatatctttattttcattacatctgtgtgttggttttttgtgtgaatcgatagtactaacatacgctctccatcaaaacaaaacgaaacaaaacaaactagcaaaataggctgtccccagtgcaagtgcaggtgccagaacatttctct

SEQ ID NO: 5 - DNA, 1188 bp, Cricetulus griseus
ggagagggggtaaaaaaatgctgcactgtgcggctaggccggtgagtgagcggcgcggagccaatcagcgctcgccgttccgaaagttgccttttatggctcgagtggccgctgtggcgtcctataaaacccggcggcgcaacgcgcagccactgtcgagtccgcgtccacccgcgagcacaggcctttcgcagctctttcttcgccgctccacacccgccaccaggtaagcagggacaacaggcccagccggccacagccctcccgtgggcagtgaccgcgctgcagggtcgcgggggacactcggcgcggacaccggggaaggctggagggtggtgccgggccgcggagcggacactttcagatccaactttcagtccagggtgtagaccctttacagccgcattgccacggtgtagacaccggtggacccgctctggctcagagcacgcggcttgggggaacccattagggtcgcagtgtgggcgctatgagagccgatgcagctttcgggtgttgaaccgtatctgcccaccttggggggaggacacaaggtcgggagccaaacgccacgatcatgccttggtggcccatgggtctttgtctaaaccggtttgcccatttggcttgccgggcgggcgggcgcggcgggcccggctcggccgggttgggggctgggttgccactgcgcttgcgcgctctatggctgggtattggggcgcgtgcacgctggggagggagcccttcctcttccccctctcccaagttaaacttgcgcgtgcgtattgagacttggagcgcggccaccggggttgggcgagggcggggccgttgtccggaaggggcggggtcgcagcggcttcggggcgcctgctcgcgcttcctgctgggtgtggtcgcctcccgcgcgcgcactagccgcccgccggcggggcgaaggcggggcttgcgcccgtttggggagggggcggaggcctggcttcctgccgtggggccgcctccggaccagcgtttgcctcttatggtaataacgcggccggcctgggcttcctttgtcccctgagtttgggcgcgcgccccctggcggcccgaggccgcggcttgccggaagtgggcagggcggcagcggctgcgcctagtggcccgccagtgaccgcgaccctcttttgtgccctgatatagttcgcc

SEQ ID NO: 6 - DNA, 1822 bp, Artificial Sequence
  Promoter
ggagagggggtaaaaaaatgctgcactgtgcggctaggccggtgagtgagcggcgcggagccaatcagcgctcgccgttccgaaagttgccttttatggctcgagtggccgctgtggcgtcctataaaacccggcggcgcaacgcgcagccactgtcgagtccgcgtccacccgcgagcacaggcctttcgcagctctttcttcgccgctccacacccgccaccaggtaagcagggacaacaggcccagccggccacagccctcccgtgggcagtgaccgcgctgcagggtcgcgggggacactcggcgcggacaccggggaaggctggagggtggtgccgggccgcggagcggacactttcagatccaactttcagtccagggtgtagaccctttacagccgcattgccacggtgtagacaccggtggacccgctctggctcagagcacgcggcttgggggaacccattagggtcgcagtgtgggcgctatgagagccgatgcagctttcgggtgttgaaccgtatctgcccaccttggggggaggacacaaggtcgggagccaaacgccacgatcatgccttggtggcccatgggtctttgtctaaaccggtttgcccatttggcttgccgggcgggcgggcgcggcgggcccggctcggccgggttgggggctgggttgccactgcgcttgcgcgctctatggctgggtattggggcgcgtgcacgctggggagggagcccttcctcttccccctctcccaagttaaacttgcgcgtgcgtattgagacttggagcgcggccaccggggttgggcgagggcggggccgttgtccggaaggggcggggtcgcagcggcttcggggcgcctgctcgcgcttcctgctgggtgtggtcgcctcccgcgcgcgcactagccgcccgccggcggggcgaaggcggggcttgcgcccgtttggggagggggcggaggcctggcttcctgccgtggggccgcctccggaccagcgtttgcctcttatggtaataacgcggccggcctgggcttcctttgtcccctgagtttgggcgcgcgccccctggcggcccgaggccgcggcttgccggaagtgggcagggcggcagcggctgcgcctagtggcccgccagtgaccgcgaccctcttttgtgccctgatatagttcgccagatctgttgacattgattattgactagttattaatagtaatcaattacggggtcattagttcatagcccatatatggagttccgcgttacataacttacggtaaatggcccgcctggctgaccgcccaacgacccccgcccattgacgtcaataatgacgtatgttcccatagtaacgccaatagggactttccattgacgtcaatgggtggagtatttacggtaaactgcccacttggcagtacatcaagtgtatcatatgccaagtacgccccctattgacgtcaatgacggtaaatggcccgcctggcattatgcccagtacatgaccttatgggactttcctacttggcagtacatctacgtattagtcatcgctattaccatggtgatgcggttttggcagtacatcaatgggcgtggatagcggtttgactcacggggatttccaagtctccaccccattgacgtcaatgggagtttgttttggcaccaaaatcaacgggactttccaaaatgtcgtaacaactccgccccattgacgcaaatgggcggtaggcgtgtacggtgggaggtctatataagcagagctctctggctaactagagaacccactgcttactggcttatcga

SEQ ID NO: 7 - DNA, 7565 bp, Artificial Sequence
  Plasmid
ggcctaactggccggtaccggagagggggtaaaaaaatgctgcactgtgcggctaggccggtgagtgagcggcgcggagccaatcagcgctcgccgttccgaaagttgccttttatggctcgagtggccgctgtggcgtcctataaaacccggcggcgcaacgcgcagccactgtcgagtccgcgtccacccgcgagcacaggcctttcgcagctctttcttcgccgctccacacccgccaccaggtaagcagggacaacaggcccagccggccacagccctcccgtgggcagtgaccgcgctgcagggtcgcgggggacactcggcgcggacaccggggaaggctggagggtggtgccgggccgcggagcggacactttcagatccaactttcagtccagggtgtagaccctttacagccgcattgccacggtgtagacaccggtggacccgctctggctcagagcacgcggcttgggggaacccattagggtcgcagtgtgggcgctatgagagccgatgcagctttcgggtgttgaaccgtatctgcccaccttggggggaggacacaaggtcgggagccaaacgccacgatcatgccttggtggcccatgggtctttgtctaaaccggtttgcccatttggcttgccgggcgggcgggcgcggcgggcccggctcggccgggttgggggctgggttgccactgcgcttgcgcgctctatggctgggtattggggcgcgtgcacgctggggagggagcccttcctcttccccctctcccaagttaaacttgcgcgtgcgtattgagacttggagcgcggccaccggggttgggcgagggcggggccgttgtccggaaggggcggggtcgcagcggcttcggggcgcctgctcgcgcttcctgctgggtgtggtcgcctcccgcgcgcgcactagccgcccgccggcggggcgaaggcggggcttgcgcccgtttggggagggggcggaggcctggcttcctgccgtggggccgcctccggaccagcgtttgcctcttatggtaataacgcggccggcctgggcttcctttgtcccctgagtttgggcgcgcgccccctggcggcccgaggccgcggcttgccggaagtgggcagggcggcagcggctgcgcctagtggcccgccagtgaccgcgaccctcttttgtgccctgatatagttcgccgaattcgctagcagaacaggatgttctgatcaaagagatccaaagtcagaacacgttgttctagctaaaataacacattcagagaacatgctgttctgatcaaagagatccaaagtcagaacaaggtgttctagctaaaataacacattcagagaacatgatgttctgatcaaagagatccaaagtcgcggccgcgttgacattgattattgactagttattaatagtaatcaattacggggtcattagttcatagcccatatatggagttccgcgttacataacttacggtaaatggcccgcctggctgaccgcccaacgacccccgcccattgacgtcaataatgacgtatgttcccatagtaacgccaatagggactttccattgacgtcaatgggtggagtatttacggtaaactgcccacttggcagtacatcaagtgtatcatatgccaagtacgccccctattgacgtcaatgacggtaaatggcccgcctggcattatgcccagtacatgaccttatgggactttcctacttggcagtacatctacgtattagtcatcgctattaccatggtgatgcggttttggcagtacatcaatgggcgtggatagcggtttgactcacggggatttccaagtctccaccccattgacgtcaatgggagtttgttttggcaccaaaatcaacgggactttccaaaatgtcgtaacaactccgccccattgacgcaaatgggcggtaggcgtgtacggtgggaggtctatataagcagagctctctggctaactagagaacccactgcttactggcttatcgaaagcttggcaatccggtactgttggtaaagccaccatggaagatgccaaaaacattaagaagggcccagcgccattctacccactcgaagacgggaccgccggcgagcagctgcacaaagccatgaagcgctacgccctggtgcccggcaccatcgcctttaccgacgcacatatcgaggtggacattacctacgccgagtacttcgagatgagcgttcggctggcagaagctatgaagcgctatgggctgaatacaaaccatcggatcgtggtgtgcagcgagaatagcttgcagttcttcatgcccgtgttgggtgccctgttcatcggtgtggctgtggccccagctaacgacatctacaacgagcgcgagctgctgaacagcatgggcatcagccagcccaccgtcgtattcgtgagcaagaaagggctgcaaaagatcctcaacgtgcaaaagaagctaccgatcatacaaaagatcatcatcatggatagcaagaccgactaccagggcttccaaagcatgtacaccttcgtgacttcccatttgccacccggcttcaacgagtacgacttcgtgcccgagagcttcgaccgggacaaaaccatcgccctgatcatgaacagtagtggcagtaccggattgcccaagggcgtagccctaccgcaccgcaccgcttgtgtccgattcagtcatgcccgcgaccccatcttcggcaaccagatcatccccgacaccgctatcctcagcgtggtgccatttcaccacggcttcggcatgttcaccacgctgggctacttgatctgcggctttcgggtcgtgctcatgtaccgcttcgaggaggagctattcttgcgcagcttgcaagactataagattcaatctgccctgctggtgcccacactatttagcttcttcgctaagagcactctcatcgacaagtacgacctaagcaacttgcacgagatcgccagcggcggggcgccgctcagcaaggaggtaggtgaggccgtggccaaacgcttccacctaccaggcatccgccagggctacggcctgacagaaacaaccagcgccattctgatcacccccgaaggggacgacaagcctggcgcagtaggcaaggtggtgcccttcttcgaggctaaggtggtggacttggacaccggtaagacactgggtgtgaaccagcgcggcgagctgtgcgtccgtggccccatgatcatgagcggctacgttaacaaccccgaggctacaaacgctctcatcgacaaggacggctggctgcacagcggcgacatcgcctactgggacgaggacgagcacttcttcatcgtggaccggctgaagagcctgatcaaatacaagggctaccaggtagccccagccgaactggagagcatcctgctgcaacaccccaacatcttcgacgccggggtcgccggcctgcccgacgacgatgccggcgagctgcccgccgcagtcgtcgtgctggaacacggtaaaaccatgaccgagaaggagatcgtggactatgtggccagccaggttacaaccgccaagaagctgcgcggtggtgttgtgttcgtggacgaggtgcctaaaggactgaccggcaagttggacgcccgcaagatccgcgagattctcattaaggccaagaagggcggcaagatcgccgtgtaataattctagagtcggggcggccggccgcttcgagcagacatgataagatacattgatgagtttggacaaaccacaactagaatgcagtgaaaaaaatgctttatttgtgaaatttgtgatgctattgctttatttgtaaccattataagctgcaataaacaagttaacaacaacaattgcattcattttatgtttcaggttcagggggaggtgtgggaggttttttaaagcaagtaaaacctctacaaatgtggtaaaatcgataaggatccgtttgcgtattgggcgctcttccgctgatctgcgcagcaccatggcctgaaataacctctgaaagaggaacttggttagctaccttctgaggcggaaagaaccagctgtggaatgtgtgtcagttagggtgtggaaagtccccaggctccccagcaggcagaagtatgcaaagcatgcatctcaattagtcagcaaccaggtgtggaaagtccccaggctccccagcaggcagaagtatgcaaagcatgcatctcaattagtcagcaaccatagtcccgcccctaactccgcccatcccgcccctaactccgcccagttccgcccattctccgccccatggctgactaattttttttatttatgcagaggccgaggccgcctctgcctctgagctattccagaagtagtgaggaggcttttttggaggcctaggcttttgcaaaaagctcgattcttctgacactagcgccaccatgatcgaacaagacggcctccatgctggcagtcccgcagcttgggtcgaacgcttgttcgggtacgactgggcccagcagaccatcggatgtagcgatgcggccgtgttccgtctaagcgctcaaggccggcccgtgctgttcgtgaagaccgacctgagcggcgccctgaacgagcttcaagacgaggctgcccgcctgagctggctggccaccaccggcgtaccctgcgccgctgtgttggatgttgtgaccgaagccggccgggactggctgctgctgggcgaggtccctggccaggatctgctgagcagccaccttgcccccgctgagaaggtttctatcatggccgatgcaatgcggcgcctgcacaccctggaccccgctacctgccccttcgaccaccaggctaagcatcggatcgagcgtgctcggacccgcatggaggccggcctggtggaccaggacgacctggacgaggagcatcagggcctggcccccgctgaactgttcgcccgactgaaagcccgcatgccggacggtgaggacctggttgtcacacacggagatgcctgcctccctaacatcatggtcgagaatggccgcttctccggcttcatcgactgcggtcgcctaggagttgccgaccgctaccaggacatcgccctggccacccgcgacatcgctgaggagcttggcggcgagtgggccgaccgcttcttagtcttgtacggcatcgcagctcccgacagccagcgcatcgccttctaccgcttgctcgacgagttcttttaatgatctagaaccggtcatggccgcaataaaatatctttattttcattacatctgtgtgttggttttttgtgtgttcgaactagatgctgtcgaccgatgcccttgagagccttcaacccagtcagctccttccggtgggcgcggggcatgactatcgtcgccgcacttatgactgtcttctttatcatgcaactcgtaggacaggtgccggcagcgctcttccgcttcctcgctcactgactcgctgcgctcggtcgttcggctgcggcgagcggtatcagctcactcaaaggcggtaatacggttatccacagaatcaggggataacgcaggaaagaacatgtgagcaaaaggccagcaaaaggccaggaaccgtaaaaaggccgcgttgctggcgtttttccataggctccgcccccctgacgagcatcacaaaaatcgacgctcaagtcagaggtggcgaaacccgacaggactataaagataccaggcgtttccccctggaagctccctcgtgcgctctcctgttccgaccctgccgcttaccggatacctgtccgcctttctcccttcgggaagcgtggcgctttctcatagctcacgctgtaggtatctcagttcggtgtaggtcgttcgctccaagctgggctgtgtgcacgaaccccccgttcagcccgaccgctgcgccttatccggtaactatcgtcttgagtccaacccggtaagacacgacttatcgccactggcagcagccactggtaacaggattagcagagcgaggtatgtaggcggtgctacagagttcttgaagtggtggcctaactacggctacactagaagaacagtatttggtatctgcgctctgctgaagccagttaccttcggaaaaagagttggtagctcttgatccggcaaacaaaccaccgctggtagcggtggtttttttgtttgcaagcagcagattacgcgcagaaaaaaaggatctcaagaagatcctttgatcttttctacggggtctgacgctcagtggaacgaaaactcacgttaagggattttggtcatgagattatcaaaaaggatcttcacctagatccttttaaattaaaaatgaagttttaaatcaatctaaagtatatatgagtaaacttggtctgacagcggccgcaaatgctaaaccactgcagtggttaccagtgcttgatcagtgaggcaccgatctcagcgatctgcctatttcgttcgtccatagtggcctgactccccgtcgtgtagatcactacgattcgtgagggcttaccatcaggccccagcgcagcaatgatgccgcgagagccgcgttcaccggcccccgatttgtcagcaatgaaccagccagcagggagggccgagcgaagaagtggtcctgctactttgtccgcctccatccagtctatgagctgctgtcgtgatgctagagtaagaagttcgccagtgagtagtttccgaagagttgtggccattgctactggcatcgtggtatcacgctcgtcgttcggtatggcttcgttcaactctggttcccagcggtcaagccgggtcacatgatcacccatattatgaagaaatgcagtcagctccttagggcctccgatcgttgtcagaagtaagttggccgcggtgttgtcgctcatggtaatggcagcactacacaattctcttaccgtcatgccatccgtaagatgcttttccgtgaccggcgagtactcaaccaagtcgttttgtgagtagtgtatacggcgaccaagctgctcttgcccggcgtctatacgggacaacaccgcgccacatagcagtactttgaaagtgctcatcatcgggaatcgttcttcggggcggaaagactcaaggatcttgccgctattgagatccagttcgatatagcccactcttgcacccagttgatcttcagcatcttttactttcaccagcgtttcggggtgtgcaaaaacaggcaagcaaaatgccgcaaagaagggaatgagtgcgacacgaaaatgttggatgctcatactcgtcctttttcaatattattgaagcatttatcagggttactagtacgtctctcaaggataagtaagtaatattaaggtacgggaggtattggacaggccgcaataaaatatctttattttcattacatctgtgtgttggttttttgtgtgaatcgatagtactaacatacgctctccatcaaaacaaaacgaaacaaaacaaactagcaaaataggctgtccccagtgcaagtgcaggtgccagaacatttctct

SEQ ID NO: 8 - DNA, 175 bp, Artificial Sequence
  Tandem Sequence
agaacaggatgttctgatcaaagagatccaaagtcagaacacgttgttctagctaaaataacacattcagagaacatgctgttctgatcaaagagatccaaagtcagaacaaggtgttctagctaaaataacacattcagagaacatgatgttctgatcaaagagatccaaagtc

SEQ ID NO: 9 - DNA, 2011 bp, Artificial Sequence
  Promoter
ggagagggggtaaaaaaatgctgcactgtgcggctaggccggtgagtgagcggcgcggagccaatcagcgctcgccgttccgaaagttgccttttatggctcgagtggccgctgtggcgtcctataaaacccggcggcgcaacgcgcagccactgtcgagtccgcgtccacccgcgagcacaggcctttcgcagctctttcttcgccgctccacacccgccaccaggtaagcagggacaacaggcccagccggccacagccctcccgtgggcagtgaccgcgctgcagggtcgcgggggacactcggcgcggacaccggggaaggctggagggtggtgccgggccgcggagcggacactttcagatccaactttcagtccagggtgtagaccctttacagccgcattgccacggtgtagacaccggtggacccgctctggctcagagcacgcggcttgggggaacccattagggtcgcagtgtgggcgctatgagagccgatgcagctttcgggtgttgaaccgtatctgcccaccttggggggaggacacaaggtcgggagccaaacgccacgatcatgccttggtggcccatgggtctttgtctaaaccggtttgcccatttggcttgccgggcgggcgggcgcggcgggcccggctcggccgggttgggggctgggttgccactgcgcttgcgcgctctatggctgggtattggggcgcgtgcacgctggggagggagcccttcctcttccccctctcccaagttaaacttgcgcgtgcgtattgagacttggagcgcggccaccggggttgggcgagggcggggccgttgtccggaaggggcggggtcgcagcggcttcggggcgcctgctcgcgcttcctgctgggtgtggtcgcctcccgcgcgcgcactagccgcccgccggcggggcgaaggcggggcttgcgcccgtttggggagggggcggaggcctggcttcctgccgtggggccgcctccggaccagcgtttgcctcttatggtaataacgcggccggcctgggcttcctttgtcccctgagtttgggcgcgcgccccctggcggcccgaggccgcggcttgccggaagtgggcagggcggcagcggctgcgcctagtggcccgccagtgaccgcgaccctcttttgtgccctgatatagttcgccgaattcgctagcagaacaggatgttctgatcaaagagatccaaagtcagaacacgttgttctagctaaaataacacattcagagaacatgctgttctgatcaaagagatccaaagtcagaacaaggtgttctagctaaaataacacattcagagaacatgatgttctgatcaaagagatccaaagtcgcggccgcgttgacattgattattgactagttattaatagtaatcaattacggggtcattagttcatagcccatatatggagttccgcgttacataacttacggtaaatggcccgcctggctgaccgcccaacgacccccgcccattgacgtcaataatgacgtatgttcccatagtaacgccaatagggactttccattgacgtcaatgggtggagtatttacggtaaactgcccacttggcagtacatcaagtgtatcatatgccaagtacgccccctattgacgtcaatgacggtaaatggcccgcctggcattatgcccagtacatgaccttatgggactttcctacttggcagtacatctacgtattagtcatcgctattaccatggtgatgcggttttggcagtacatcaatgggcgtggatagcggtttgactcacggggatttccaagtctccaccccattgacgtcaatgggagtttgttttggcaccaaaatcaacgggactttccaaaatgtcgtaacaactccgccccattgacgcaaatgggcggtaggcgtgtacggtgggaggtctatataagcagagctctctggctaactagagaacccactgcttactggcttatcga

SEQ ID NO: 10 - DNA, 7609 bp, Artificial Sequence
  Plasmid
ggcctaactggccggtacctgagctcgctagcggagagggggtaaaaaaatgctgcactgtgcggctaggccggtgagtgagcggcgcggagccaatcagcgctcgccgttccgaaagttgccttttatggctcgagtggccgctgtggcgtcctataaaacccggcggcgcaacgcgcagccactgtcgagtccgcgtccacccgcgagcacaggcctttcgcagctctttcttcgccgctccacacccgccaccaggtaagcagggacaacaggcccagccggccacagccctcccgtgggcagtgaccgcgctgcagggtcgcgggggacactcggcgcggacaccggggaaggctggagggtggtgccgggccgcggagcggacactttcagatccaactttcagtccagggtgtagaccctttacagccgcattgccacggtgtagacaccggtggacccgctctggctcagagcacgcggcttgggggaacccattagggtcgcagtgtgggcgctatgagagccgatgcagctttcgggtgttgaaccgtatctgcccaccttggggggaggacacaaggtcgggagccaaacgccacgatcatgccttggtggcccatgggtctttgtctaaaccggtttgcccatttggcttgccgggcgggcgggcgcggcgggcccggctcggccgggttgggggctgggttgccactgcgcttgcgcgctctatggctgggtattggggcgcgtgcacgctggggagggagcccttcctcttccccctctcccaagttaaacttgcgcgtgcgtattgagacttggagcgcggccaccggggttgggcgagggcggggccgttgtccggaaggggcggggtcgcagcggcttcggggcgcctgctcgcgcttcctgctgggtgtggtcgcctcccgcgcgcgcactagccgcccgccggcggggcgaaggcggggcttgcgcccgtttggggagggggcggaggcctggcttcctgccgtggggccgcctccggaccagcgtttgcctcttatggtaataacgcggccggcctgggcttcctttgtcccctgagtttgggcgcgcgccccctggcggcccgaggccgcggcttgccggaagtgggcagggcggcagcggctgcgcctagtggcccgccagtgaccgcgaccctcttttgtgccctgatatagttcgccgaattcttttttgcggccgcgttgacattgattattgactagttattaatagtaatcaattacggggtcattagttcatagcccatatatggagttccgcgttacataacttacggtaaatggcccgcctggctgaccgcccaacgacccccgcccattgacgtcaataatgacgtatgttcccatagtaacgccaatagggactttccattgacgtcaatgggtggagtatttacggtaaactgcccacttggcagtacatcaagtgtatcatatgccaagtacgccccctattgacgtcaatgacggtaaatggcccgcctggcattatgcccagtacatgaccttatgggactttcctacttggcagtacatctacgtattagtcatcgctattaccatggtgatgcggttttggcagtacatcaatgggcgtggatagcggtttgactcacggggatttccaagtctccaccccattgacgtcaatgggagtttgttttggcaccaaaatcaacgggactttccaaaatgtcgtaacaactccgccccattgacggctagcagaacaggatgttctgatcaaagagatccaaagtcagaacacgttgttctagctaaaataacacattcagagaacatgctgttctgatcaaagagatccaaagtcagaacaaggtgttctagctaaaataacacattcagagaacatgatgttctgatcaaagagatccaaagtcctcgaggatatcaagatctgcaaatcaaatgggcggtaggcgtgtacggtgggaggtctatataagcagagctctctggctaactagagaacccactgcttactggcttatcgaaagcttggcaatccggtactgttggtaaagccaccatggaagatgccaaaaacattaagaagggcccagcgccattctacccactcgaagacgggaccgccggcgagcagctgcacaaagccatgaagcgctacgccctggtgcccggcaccatcgcctttaccgacgcacatatcgaggtggacattacctacgccgagtacttcgagatgagcgttcggctggcagaagctatgaagcgctatgggctgaatacaaaccatcggatcgtggtgtgcagcgagaatagcttgcagttcttcatgcccgtgttgggtgccctgttcatcggtgtggctgtggccccagctaacgacatctacaacgagcgcgagctgctgaacagcatgggcatcagccagcccaccgtcgtattcgtgagcaagaaagggctgcaaaagatcctcaacgtgcaaaagaagctaccgatcatacaaaagatcatcatcatggatagcaagaccgactaccagggcttccaaagcatgtacaccttcgtgacttcccatttgccacccggcttcaacgagtacgacttcgtgcccgagagcttcgaccgggacaaaaccatcgccctgatcatgaacagtagtggcagtaccggattgcccaagggcgtagccctaccgcaccgcaccgcttgtgtccgattcagtcatgcccgcgaccccatcttcggcaaccagatcatccccgacaccgctatcctcagcgtggtgccatttcaccacggcttcggcatgttcaccacgctgggctacttgatctgcggctttcgggtcgtgctcatgtaccgcttcgaggaggagctattcttgcgcagcttgcaagactataagattcaatctgccctgctggtgcccacactatttagcttcttcgctaagagcactctcatcgacaagtacgacctaagcaacttgcacgagatcgccagcggcggggcgccgctcagcaaggaggtaggtgaggccgtggccaaacgcttccacctaccaggcatccgccagggctacggcctgacagaaacaaccagcgccattctgatcacccccgaaggggacgacaagcctggcgcagtaggcaaggtggtgcccttcttcgaggctaaggtggtggacttggacaccggtaagacactgggtgtgaaccagcgcggcgagctgtgcgtccgtggccccatgatcatgagcggctacgttaacaaccccgaggctacaaacgctctcatcgacaaggacggctggctgcacagcggcgacatcgcctactgggacgaggacgagcacttcttcatcgtggaccggctgaagagcctgatcaaatacaagggctaccaggtagccccagccgaactggagagcatcctgctgcaacaccccaacatcttcgacgccggggtcgccggcctgcccgacgacgatgccggcgagctgcccgccgcagtcgtcgtgctggaacacggtaaaaccatgaccgagaaggagatcgtggactatgtggccagccaggttacaaccgccaagaagctgcgcggtggtgttgtgttcgtggacgaggtgcctaaaggactgaccggcaagttggacgcccgcaagatccgcgagattctcattaaggccaagaagggcggcaagatcgccgtgtaataattctagagtcggggcggccggccgcttcgagcagacatgataagatacattgatgagtttggacaaaccacaactagaatgcagtgaaaaaaatgctttatttgtgaaatttgtgatgctattgctttatttgtaaccattataagctgcaataaacaagttaacaacaacaattgcattcattttatgtttcaggttcagggggaggtgtgggaggttttttaaagcaagtaaaacctctacaaatgtggtaaaatcgataaggatccgtttgcgtattgggcgctcttccgctgatctgcgcagcaccatggcctgaaataacctctgaaagaggaacttggttagctaccttctgaggcggaaagaaccagctgtggaatgtgtgtcagttagggtgtggaaagtccccaggctccccagcaggcagaagtatgcaaagcatgcatctcaattagtcagcaaccaggtgtggaaagtccccaggctccccagcaggcagaagtatgcaaagcatgcatctcaattagtcagcaaccatagtcccgcccctaactccgcccatcccgcccctaactccgcccagttccgcccattctccgccccatggctgactaattttttttatttatgcagaggccgaggccgcctctgcctctgagctattccagaagtagtgaggaggcttttttggaggcctaggcttttgcaaaaagctcgattcttctgacactagcgccaccatgatcgaacaagacggcctccatgctggcagtcccgcagcttgggtcgaacgcttgttcgggtacgactgggcccagcagaccatcggatgtagcgatgcggccgtgttccgtctaagcgctcaaggccggcccgtgctgttcgtgaagaccgacctgagcggcgccctgaacgagcttcaagacgaggctgcccgcctgagctggctggccaccaccggcgtaccctgcgccgctgtgttggatgttgtgaccgaagccggccgggactggctgctgctgggcgaggtccctggccaggatctgctgagcagccaccttgcccccgctgagaaggtttctatcatggccgatgcaatgcggcgcctgcacaccctggaccccgctacctgccccttcgaccaccaggctaagcatcggatcgagcgtgctcggacccgcatggaggccggcctggtggaccaggacgacctggacgaggagcatcagggcctggcccccgctgaactgttcgcccgactgaaagcccgcatgccggacggtgaggacctggttgtcacacacggagatgcctgcctccctaacatcatggtcgagaatggccgcttctccggcttcatcgactgcggtcgcctaggagttgccgaccgctaccaggacatcgccctggccacccgcgacatcgctgaggagcttggcggcgagtgggccgaccgcttcttagtcttgtacggcatcgcagctcccgacagccagcgcatcgccttctaccgcttgctcgacgagttcttttaatgatctagaaccggtcatggccgcaataaaatatctttattttcattacatctgtgtgttggttttttgtgtgttcgaactagatgctgtcgaccgatgcccttgagagccttcaacccagtcagctccttccggtgggcgcggggcatgactatcgtcgccgcacttatgactgtcttctttatcatgcaactcgtaggacaggtgccggcagcgctcttccgcttcctcgctcactgactcgctgcgctcggtcgttcggctgcggcgagcggtatcagctcactcaaaggcggtaatacggttatccacagaatcaggggataacgcaggaaagaacatgtgagcaaaaggccagcaaaaggccaggaaccgtaaaaaggccgcgttgctggcgtttttccataggctccgcccccctgacgagcatcacaaaaatcgacgctcaagtcagaggtggcgaaacccgacaggactataaagataccaggcgtttccccctggaagctccctcgtgcgctctcctgttccgaccctgccgcttaccggatacctgtccgcctttctcccttcgggaagcgtggcgctttctcatagctcacgctgtaggtatctcagttcggtgtaggtcgttcgctccaagctgggctgtgtgcacgaaccccccgttcagcccgaccgctgcgccttatccggtaactatcgtcttgagtccaacccggtaagacacgacttatcgccactggcagcagccactggtaacaggattagcagagcgaggtatgtaggcggtgctacagagttcttgaagtggtggcctaactacggctacactagaagaacagtatttggtatctgcgctctgctgaagccagttaccttcggaaaaagagttggtagctcttgatccggcaaacaaaccaccgctggtagcggtggtttttttgtttgcaagcagcagattacgcgcagaaaaaaaggatctcaagaagatcctttgatcttttctacggggtctgacgctcagtggaacgaaaactcacgttaagggattttggtcatgagattatcaaaaaggatcttcacctagatccttttaaattaaaaatgaagttttaaatcaatctaaagtatatatgagtaaacttggtctgacagcggccgcaaatgctaaaccactgcagtggttaccagtgcttgatcagtgaggcaccgatctcagcgatctgcctatttcgttcgtccatagtggcctgactccccgtcgtgtagatcactacgattcgtgagggcttaccatcaggccccagcgcagcaatgatgccgcgagagccgcgttcaccggcccccgatttgtcagcaatgaaccagccagcagggagggccgagcgaagaagtggtcctgctactttgtccgcctccatccagtctatgagctgctgtcgtgatgctagagtaagaagttcgccagtgagtagtttccgaagagttgtggccattgctactggcatcgtggtatcacgctcgtcgttcggtatggcttcgttcaactctggttcccagcggtcaagccgggtcacatgatcacccatattatgaagaaatgcagtcagctccttagggcctccgatcgttgtcagaagtaagttggccgcggtgttgtcgctcatggtaatggcagcactacacaattctcttaccgtcatgccatccgtaagatgcttttccgtgaccggcgagtactcaaccaagtcgttttgtgagtagtgtatacggcgaccaagctgctcttgcccggcgtctatacgggacaacaccgcgccacatagcagtactttgaaagtgctcatcatcgggaatcgttcttcggggcggaaagactcaaggatcttgccgctattgagatccagttcgatatagcccactcttgcacccagttgatcttcagcatcttttactttcaccagcgtttcggggtgtgcaaaaacaggcaagcaaaatgccgcaaagaagggaatgagtgcgacacgaaaatgttggatgctcatactcgtcctttttcaatattattgaagcatttatcagggttactagtacgtctctcaaggataagtaagtaatattaaggtacgggaggtattggacaggccgcaataaaatatctttattttcattacatctgtgtgttggttttttgtgtgaatcgatagtactaacatacgctctccatcaaaacaaaacgaaacaaaacaaactagcaaaataggctgtccccagtgcaagtgcaggtgccagaacatttctct

SEQ ID NO: 11 - DNA, 2042 bp, Artificial Sequence
  Promoter
ggagagggggtaaaaaaatgctgcactgtgcggctaggccggtgagtgagcggcgcggagccaatcagcgctcgccgttccgaaagttgccttttatggctcgagtggccgctgtggcgtcctataaaacccggcggcgcaacgcgcagccactgtcgagtccgcgtccacccgcgagcacaggcctttcgcagctctttcttcgccgctccacacccgccaccaggtaagcagggacaacaggcccagccggccacagccctcccgtgggcagtgaccgcgctgcagggtcgcgggggacactcggcgcggacaccggggaaggctggagggtggtgccgggccgcggagcggacactttcagatccaactttcagtccagggtgtagaccctttacagccgcattgccacggtgtagacaccggtggacccgctctggctcagagcacgcggcttgggggaacccattagggtcgcagtgtgggcgctatgagagccgatgcagctttcgggtgttgaaccgtatctgcccaccttggggggaggacacaaggtcgggagccaaacgccacgatcatgccttggtggcccatgggtctttgtctaaaccggtttgcccatttggcttgccgggcgggcgggcgcggcgggcccggctcggccgggttgggggctgggttgccactgcgcttgcgcgctctatggctgggtattggggcgcgtgcacgctggggagggagcccttcctcttccccctctcccaagttaaacttgcgcgtgcgtattgagacttggagcgcggccaccggggttgggcgagggcggggccgttgtccggaaggggcggggtcgcagcggcttcggggcgcctgctcgcgcttcctgctgggtgtggtcgcctcccgcgcgcgcactagccgcccgccggcggggcgaaggcggggcttgcgcccgtttggggagggggcggaggcctggcttcctgccgtggggccgcctccggaccagcgtttgcctcttatggtaataacgcggccggcctgggcttcctttgtcccctgagtttgggcgcgcgccccctggcggcccgaggccgcggcttgccggaagtgggcagggcggcagcggctgcgcctagtggcccgccagtgaccgcgaccctcttttgtgccctgatatagttcgccgaattcttttttgcggccgcgttgacattgattattgactagttattaatagtaatcaattacggggtcattagttcatagcccatatatggagttccgcgttacataacttacggtaaatggcccgcctggctgaccgcccaacgacccccgcccattgacgtcaataatgacgtatgttcccatagtaacgccaatagggactttccattgacgtcaatgggtggagtatttacggtaaactgcccacttggcagtacatcaagtgtatcatatgccaagtacgccccctattgacgtcaatgacggtaaatggcccgcctggcattatgcccagtacatgaccttatgggactttcctacttggcagtacatctacgtattagtcatcgctattaccatggtgatgcggttttggcagtacatcaatgggcgtggatagcggtttgactcacggggatttccaagtctccaccccattgacgtcaatgggagtttgttttggcaccaaaatcaacgggactttccaaaatgtcgtaacaactccgccccattgacggctagcagaacaggatgttctgatcaaagagatccaaagtcagaacacgttgttctagctaaaataacacattcagagaacatgctgttctgatcaaagagatccaaagtcagaacaaggtgttctagctaaaataacacattcagagaacatgatgttctgatcaaagagatccaaagtcctcgaggatatcaagatctgcaaatcaaatgggcggtaggcgtgtacggtgggaggtctatataagcagagctctctggctaactagagaacccactgcttactggcttatcga

SEQ ID NO: 12 - DNA, 7786 bp, Artificial Sequence
  Plasmid
ggcctaactggccggtacctgagctcgctagcggagagggggtaaaaaaatgctgcactgtgcggctaggccggtgagtgagcggcgcggagccaatcagcgctcgccgttccgaaagttgccttttatggctcgagtggccgctgtggcgtcctataaaacccggcggcgcaacgcgcagccactgtcgagtccgcgtccacccgcgagcacaggcctttcgcagctctttcttcgccgctccacacccgccaccaggtaagcagggacaacaggcccagccggccacagccctcccgtgggcagtgaccgcgctgcagggtcgcgggggacactcggcgcggacaccggggaaggctggagggtggtgccgggccgcggagcggacactttcagatccaactttcagtccagggtgtagaccctttacagccgcattgccacggtgtagacaccggtggacccgctctggctcagagcacgcggcttgggggaacccattagggtcgcagtgtgggcgctatgagagccgatgcagctttcgggtgttgaaccgtatctgcccaccttggggggaggacacaaggtcgggagccaaacgccacgatcatgccttggtggcccatgggtctttgtctaaaccggtttgcccatttggcttgccgggcgggcgggcgcggcgggcccggctcggccgggttgggggctgggttgccactgcgcttgcgcgctctatggctgggtattggggcgcgtgcacgctggggagggagcccttcctcttccccctctcccaagttaaacttgcgcgtgcgtattgagacttggagcgcggccaccggggttgggcgagggcggggccgttgtccggaaggggcggggtcgcagcggcttcggggcgcctgctcgcgcttcctgctgggtgtggtcgcctcccgcgcgcgcactagccgcccgccggcggggcgaaggcggggcttgcgcccgtttggggagggggcggaggcctggcttcctgccgtggggccgcctccggaccagcgtttgcctcttatggtaataacgcggccggcctgggcttcctttgtcccctgagtttgggcgcgcgccccctggcggcccgaggccgcggcttgccggaagtgggcagggcggcagcggctgcgcctagtggcccgccagtgaccgcgaccctcttttgtgccctgatatagttcgccgaattcagaacaggatgttctgatcaaagagatccaaagtcagaacacgttgttctagctaaaataacacattcagagaacatgctgttctgatcaaagagatccaaagtcagaacaaggtgttctagctaaaataacacattcagagaacatgatgttctgatcaaagagatccaaagtcctcgaggatatcagcggccgcgttgacattgattattgactagttattaatagtaatcaattacggggtcattagttcatagcccatatatggagttccgcgttacataacttacggtaaatggcccgcctggctgaccgcccaacgacccccgcccattgacgtcaataatgacgtatgttcccatagtaacgccaatagggactttccattgacgtcaatgggtggagtatttacggtaaactgcccacttggcagtacatcaagtgtatcatatgccaagtacgccccctattgacgtcaatgacggtaaatggcccgcctggcattatgcccagtacatgaccttatgggactttcctacttggcagtacatctacgtattagtcatcgctattaccatggtgatgcggttttggcagtacatcaatgggcgtggatagcggtttgactcacggggatttccaagtctccaccccattgacgtcaatgggagtttgttttggcaccaaaatcaacgggactttccaaaatgtcgtaacaactccgccccattgacggctagcagaacaggatgttctgatcaaagagatccaaagtcagaacacgttgttctagctaaaataacacattcagagaacatgctgttctgatcaaagagatccaaagtcagaacaaggtgttctagctaaaataacacattcagagaacatgatgttctgatcaaagagatccaaagtcctcgaggatatcaagatctgcaaatgggcggtaggcgtgtacggtgggaggtctatataagcagagctctctggctaactagagaacccactgcttactggcttatcgaaagcttggcaatccggtactgttggtaaagccaccatggaagatgccaaaaacattaagaagggcccagcgccattctacccactcgaagacgggaccgccggcgagcagctgcacaaagccatgaagcgctacgccctggtgcccggcaccatcgcctttaccgacgcacatatcgaggtggacattacctacgccgagtacttcgagatgagcgttcggctggcagaagctatgaagcgctatgggctgaatacaaaccatcggatcgtggtgtgcagcgagaatagcttgcagttcttcatgcccgtgttgggtgccctgttcatcggtgtggctgtggccccagctaacgacatctacaacgagcgcgagctgctgaacagcatgggcatcagccagcccaccgtcgtattcgtgagcaagaaagggctgcaaaagatcctcaacgtgcaaaagaagctaccgatcatacaaaagatcatcatcatggatagcaagaccgactaccagggcttccaaagcatgtacaccttcgtgacttcccatttgccacccggcttcaacgagtacgacttcgtgcccgagagcttcgaccgggacaaaaccatcgccctgatcatgaacagtagtggcagtaccggattgcccaagggcgtagccctaccgcaccgcaccgcttgtgtccgattcagtcatgcccgcgaccccatcttcggcaaccagatcatccccgacaccgctatcctcagcgtggtgccatttcaccacggcttcggcatgttcaccacgctgggctacttgatctgcggctttcgggtcgtgctcatgtaccgcttcgaggaggagctattcttgcgcagcttgcaagactataagattcaatctgccctgctggtgcccacactatttagcttcttcgctaagagcactctcatcgacaagtacgacctaagcaacttgcacgagatcgccagcggcggggcgccgctcagcaaggaggtaggtgaggccgtggccaaacgcttccacctaccaggcatccgccagggctacggcctgacagaaacaaccagcgccattctgatcacccccgaaggggacgacaagcctggcgcagtaggcaaggtggtgcccttcttcgaggctaaggtggtggacttggacaccggtaagacactgggtgtgaaccagcgcggcgagctgtgcgtccgtggccccatgatcatgagcggctacgttaacaaccccgaggctacaaacgctctcatcgacaaggacggctggctgcacagcggcgacatcgcctactgggacgaggacgagcacttcttcatcgtggaccggctgaagagcctgatcaaatacaagggctaccaggtagccccagccgaactggagagcatcctgctgcaacaccccaacatcttcgacgccggggtcgccggcctgcccgacgacgatgccggcgagctgcccgccgcagtcgtcgtgctggaacacggtaaaaccatgaccgagaaggagatcgtggactatgtggccagccaggttacaaccgccaagaagctgcgcggtggtgttgtgttcgtggacgaggtgcctaaaggactgaccggcaagttggacgcccgcaagatccgcgagattctcattaaggccaagaagggcggcaagatcgccgtgtaataattctagagtcggggcggccggccgcttcgagcagacatgataagatacattgatgagtttggacaaaccacaactagaatgcagtgaaaaaaatgctttatttgtgaaatttgtgatgctattgctttatttgtaaccattataagctgcaataaacaagttaacaacaacaattgcattcattttatgtttcaggttcagggggaggtgtgggaggttttttaaagcaagtaaaacctctacaaatgtggtaaaatcgataaggatccgtttgcgtattgggcgctcttccgctgatctgcgcagcaccatggcctgaaataacctctgaaagaggaacttggttagctaccttctgaggcggaaagaaccagctgtggaatgtgtgtcagttagggtgtggaaagtccccaggctccccagcaggcagaagtatgcaaagcatgcatctcaattagtcagcaaccaggtgtggaaagtccccaggctccccagcaggcagaagtatgcaaagcatgcatctcaattagtcagcaaccatagtcccgcccctaactccgcccatcccgcccctaactccgcccagttccgcccattctccgccccatggctgactaattttttttatttatgcagaggccgaggccgcctctgcctctgagctattccagaagtagtgaggaggcttttttggaggcctaggcttttgcaaaaagctcgattcttctgacactagcgccaccatgatcgaacaagacggcctccatgctggcagtcccgcagcttgggtcgaacgcttgttcgggtacgactgggcccagcagaccatcggatgtagcgatgcggccgtgttccgtctaagcgctcaaggccggcccgtgctgttcgtgaagaccgacctgagcggcgccctgaacgagcttcaagacgaggctgcccgcctgagctggctggccaccaccggcgtaccctgcgccgctgtgttggatgttgtgaccgaagccggccgggactggctgctgctgggcgaggtccctggccaggatctgctgagcagccaccttgcccccgctgagaaggtttctatcatggccgatgcaatgcggcgcctgcacaccctggaccccgctacctgccccttcgaccaccaggctaagcatcggatcgagcgtgctcggacccgcatggaggccggcctggtggaccaggacgacctggacgaggagcatcagggcctggcccccgctgaactgttcgcccgactgaaagcccgcatgccggacggtgaggacctggttgtcacacacggagatgcctgcctccctaacatcatggtcgagaatggccgcttctccggcttcatcgactgcggtcgcctaggagttgccgaccgctaccaggacatcgccctggccacccgcgacatcgctgaggagcttggcggcgagtgggccgaccgcttcttagtcttgtacggcatcgcagctcccgacagccagcgcatcgccttctaccgcttgctcgacgagttcttttaatgatctagaaccggtcatggccgcaataaaatatctttattttcattacatctgtgtgttggttttttgtgtgttcgaactagatgctgtcgaccgatgcccttgagagccttcaacccagtcagctccttccggtgggcgcggggcatgactatcgtcgccgcacttatgactgtcttctttatcatgcaactcgtaggacaggtgccggcagcgctcttccgcttcctcgctcactgactcgctgcgctcggtcgttcggctgcggcgagcggtatcagctcactcaaaggcggtaatacggttatccacagaatcaggggataacgcaggaaagaacatgtgagcaaaaggccagcaaaaggccaggaaccgtaaaaaggccgcgttgctggcgtttttccataggctccgcccccctgacgagcatcacaaaaatcgacgctcaagtcagaggtggcgaaacccgacaggactataaagataccaggcgtttccccctggaagctccctcgtgcgctctcctgttccgaccctgccgcttaccggatacctgtccgcctttctcccttcgggaagcgtggcgctttctcatagctcacgctgtaggtatctcagttcggtgtaggtcgttcgctccaagctgggctgtgtgcacgaaccccccgttcagcccgaccgctgcgccttatccggtaactatcgtcttgagtccaacccggtaagacacgacttatcgccactggcagcagccactggtaacaggattagcagagcgaggtatgtaggcggtgctacagagttcttgaagtggtggcctaactacggctacactagaagaacagtatttggtatctgcgctctgctgaagccagttaccttcggaaaaagagttggtagctcttgatccggcaaacaaaccaccgctggtagcggtggtttttttgtttgcaagcagcagattacgcgcagaaaaaaaggatctcaagaagatcctttgatcttttctacggggtctgacgctcagtggaacgaaaactcacgttaagggattttggtcatgagattatcaaaaaggatcttcacctagatccttttaaattaaaaatgaagttttaaatcaatctaaagtatatatgagtaaacttggtctgacagcggccgcaaatgctaaaccactgcagtggttaccagtgcttgatcagtgaggcaccgatctcagcgatctgcctatttcgttcgtccatagtggcctgactccccgtcgtgtagatcactacgattcgtgagggcttaccatcaggccccagcgcagcaatgatgccgcgagagccgcgttcaccggcccccgatttgtcagcaatgaaccagccagcagggagggccgagcgaagaagtggtcctgctactttgtccgcctccatccagtctatgagctgctgtcgtgatgctagagtaagaagttcgccagtgagtagtttccgaagagttgtggccattgctactggcatcgtggtatcacgctcgtcgttcggtatggcttcgttcaactctggttcccagcggtcaagccgggtcacatgatcacccatattatgaagaaatgcagtcagctccttagggcctccgatcgttgtcagaagtaagttggccgcggtgttgtcgctcatggtaatggcagcactacacaattctcttaccgtcatgccatccgtaagatgcttttccgtgaccggcgagtactcaaccaagtcgttttgtgagtagtgtatacggcgaccaagctgctcttgcccggcgtctatacgggacaacaccgcgccacatagcagtactttgaaagtgctcatcatcgggaatcgttcttcggggcggaaagactcaaggatcttgccgctattgagatccagttcgatatagcccactcttgcacccagttgatcttcagcatcttttactttcaccagcgtttcggggtgtgcaaaaacaggcaagcaaaatgccgcaaagaagggaatgagtgcgacacgaaaatgttggatgctcatactcgtcctttttcaatattattgaagcatttatcagggttactagtacgtctctcaaggataagtaagtaatattaaggtacgggaggtattggacaggccgcaataaaatatctttattttcattacatctgtgtgttggttttttgtgtgaatcgatagtactaacatacgctctccatcaaaacaaaacgaaacaaaacaaactagcaaaataggctgtccccagtgcaagtgcaggtgccagaacatttctct

SEQ ID NO: 13 - DNA, 2219 bp, Artificial Sequence
  Promoter
ggagagggggtaaaaaaatgctgcactgtgcggctaggccggtgagtgagcggcgcggagccaatcagcgctcgccgttccgaaagttgccttttatggctcgagtggccgctgtggcgtcctataaaacccggcggcgcaacgcgcagccactgtcgagtccgcgtccacccgcgagcacaggcctttcgcagctctttcttcgccgctccacacccgccaccaggtaagcagggacaacaggcccagccggccacagccctcccgtgggcagtgaccgcgctgcagggtcgcgggggacactcggcgcggacaccggggaaggctggagggtggtgccgggccgcggagcggacactttcagatccaactttcagtccagggtgtagaccctttacagccgcattgccacggtgtagacaccggtggacccgctctggctcagagcacgcggcttgggggaacccattagggtcgcagtgtgggcgctatgagagccgatgcagctttcgggtgttgaaccgtatctgcccaccttggggggaggacacaaggtcgggagccaaacgccacgatcatgccttggtggcccatgggtctttgtctaaaccggtttgcccatttggcttgccgggcgggcgggcgcggcgggcccggctcggccgggttgggggctgggttgccactgcgcttgcgcgctctatggctgggtattggggcgcgtgcacgctggggagggagcccttcctcttccccctctcccaagttaaacttgcgcgtgcgtattgagacttggagcgcggccaccggggttgggcgagggcggggccgttgtccggaaggggcggggtcgcagcggcttcggggcgcctgctcgcgcttcctgctgggtgtggtcgcctcccgcgcgcgcactagccgcccgccggcggggcgaaggcggggcttgcgcccgtttggggagggggcggaggcctggcttcctgccgtggggccgcctccggaccagcgtttgcctcttatggtaataacgcggccggcctgggcttcctttgtcccctgagtttgggcgcgcgccccctggcggcccgaggccgcggcttgccggaagtgggcagggcggcagcggctgcgcctagtggcccgccagtgaccgcgaccctcttttgtgccctgatatagttcgccgaattcagaacaggatgttctgatcaaagagatccaaagtcagaacacgttgttctagctaaaataacacattcagagaacatgctgttctgatcaaagagatccaaagtcagaacaaggtgttctagctaaaataacacattcagagaacatgatgttctgatcaaagagatccaaagtcctcgaggatatcagcggccgcgttgacattgattattgactagttattaatagtaatcaattacggggtcattagttcatagcccatatatggagttccgcgttacataacttacggtaaatggcccgcctggctgaccgcccaacgacccccgcccattgacgtcaataatgacgtatgttcccatagtaacgccaatagggactttccattgacgtcaatgggtggagtatttacggtaaactgcccacttggcagtacatcaagtgtatcatatgccaagtacgccccctattgacgtcaatgacggtaaatggcccgcctggcattatgcccagtacatgaccttatgggactttcctacttggcagtacatctacgtattagtcatcgctattaccatggtgatgcggttttggcagtacatcaatgggcgtggatagcggtttgactcacggggatttccaagtctccaccccattgacgtcaatgggagtttgttttggcaccaaaatcaacgggactttccaaaatgtcgtaacaactccgccccattgacggctagcagaacaggatgttctgatcaaagagatccaaagtcagaacacgttgttctagctaaaataacacattcagagaacatgctgttctgatcaaagagatccaaagtcagaacaaggtgttctagctaaaataacacattcagagaacatgatgttctgatcaaagagatccaaagtcctcgaggatatcaagatctgcaaatgggcggtaggcgtgtacggtgggaggtctatataagcagagctctctggctaactagagaacccactgcttactggcttatcga

SEQ ID NO: 14 - DNA, 5427 bp, Artificial Sequence
  Plasmid
gacggatcgggagatctcccgatcccctatggtgcactctcagtacaatctgctctgatgccgcatagttaagccagtatctgctccctgcttgtgtgttggaggtcgctgagtagtgcgcgagcaaaatttaagctacaacaaggcaaggcttgaccgacaattgcatgaagaatctgcttagggttaggcgttttgcgctgcttcgcgatgtacgggccagatatacgcgttgacattgattattgactagttattaatagtaatcaattacggggtcattagttcatagcccatatatggagttccgcgttacataacttacggtaaatggcccgcctggctgaccgcccaacgacccccgcccattgacgtcaataatgacgtatgttcccatagtaacgccaatagggactttccattgacgtcaatgggtggagtatttacggtaaactgcccacttggcagtacatcaagtgtatcatatgccaagtacgccccctattgacgtcaatgacggtaaatggcccgcctggcattatgcccagtacatgaccttatgggactttcctacttggcagtacatctacgtattagtcatcgctattaccatggtgatgcggttttggcagtacatcaatgggcgtggatagcggtttgactcacggggatttccaagtctccaccccattgacgtcaatgggagtttgttttggcaccaaaatcaacgggactttccaaaatgtcgtaacaactccgccccattgacgcaaatgggcggtaggcgtgtacggtgggaggtctatataagcagagctctctggctaactagagaacccactgcttactggcttatcgaaattaatacgactcactatagggagacccaagctggctagcgtttaaacgggccctctagactcgagcggccgccactgtgctggatatctgcagaattccaccacactggactagtggatccgagctcggtaccaagcttaagtttaaaccgctgatcagcctcgactgtgccttctagttgccagccatctgttgtttgcccctcccccgtgccttccttgaccctggaaggtgccactcccactgtcctttcctaataaaatgaggaaattgcatcgcattgtctgagtaggtgtcattctattctggggggtggggtggggcaggacagcaagggggaggattgggaagacaatagcaggcatgctggggatgcggtgggctctatggcttctgaggcggaaagaaccagctggggctctagggggtatccccacgcgccctgtagcggcgcattaagcgcggcgggtgtggtggttacgcgcagcgtgaccgctacacttgccagcgccctagcgcccgctcctttcgctttcttcccttcctttctcgccacgttcgccggctttccccgtcaagctctaaatcgggggctccctttagggttccgatttagtgctttacggcacctcgaccccaaaaaacttgattagggtgatggttcacgtagtgggccatcgccctgatagacggtttttcgccctttgacgttggagtccacgttctttaatagtggactcttgttccaaactggaacaacactcaaccctatctcggtctattcttttgatttataagggattttgccgatttcggcctattggttaaaaaatgagctgatttaacaaaaatttaacgcgaattaattctgtggaatgtgtgtcagttagggtgtggaaagtccccaggctccccagcaggcagaagtatgcaaagcatgcatctcaattagtcagcaaccaggtgtggaaagtccccaggctccccagcaggcagaagtatgcaaagcatgcatctcaattagtcagcaaccatagtcccgcccctaactccgcccatcccgcccctaactccgcccagttccgcccattctccgccccatggctgactaattttttttatttatgcagaggccgaggccgcctctgcctctgagctattccagaagtagtgaggaggcttttttggaggcctaggcttttgcaaaaagctcccgggagcttgtatatccattttcggatctgatcaagagacaggatgaggatcgtttcgcatgattgaacaagatggattgcacgcaggttctccggccgcttgggtggagaggctattcggctatgactgggcacaacagacaatcggctgctctgatgccgccgtgttccggctgtcagcgcaggggcgcccggttctttttgtcaagaccgacctgtccggtgccctgaatgaactgcaggacgaggcagcgcggctatcgtggctggccacgacgggcgttccttgcgcagctgtgctcgacgttgtcactgaagcgggaagggactggctgctattgggcgaagtgccggggcaggatctcctgtcatctcaccttgctcctgccgagaaagtatccatcatggctgatgcaatgcggcggctgcatacgcttgatccggctacctgcccattcgaccaccaagcgaaacatcgcatcgagcgagcacgtactcggatggaagccggtcttgtcgatcaggatgatctggacgaagagcatcaggggctcgcgccagccgaactgttcgccaggctcaaggcgcgcatgcccgacggcgaggatctcgtcgtgacccatggcgatgcctgcttgccgaatatcatggtggaaaatggccgcttttctggattcatcgactgtggccggctgggtgtggcggaccgctatcaggacatagcgttggctacccgtgatattgctgaagagcttggcggcgaatgggctgaccgcttcctcgtgctttacggtatcgccgctcccgattcgcagcgcatcgccttctatcgccttcttgacgagttcttctgagcgggactctggggttcgaaatgaccgaccaagcgacgcccaacctgccatcacgagatttcgattccaccgccgccttctatgaaaggttgggcttcggaatcgttttccgggacgccggctggatgatcctccagcgcggggatctcatgctggagttcttcgcccaccccaacttgtttattgcagcttataatggttacaaataaagcaatagcatcacaaatttcacaaataaagcatttttttcactgcattctagttgtggtttgtccaaactcatcaatgtatcttatcatgtctgtataccgtcgacctctagctagagcttggcgtaatcatggtcatagctgtttcctgtgtgaaattgttatccgctcacaattccacacaacatacgagccggaagcataaagtgtaaagcctggggtgcctaatgagtgagctaactcacattaattgcgttgcgctcactgcccgctttccagtcgggaaacctgtcgtgccagctgcattaatgaatcggccaacgcgcggggagaggcggtttgcgtattgggcgctcttccgcttcctcgctcactgactcgctgcgctcggtcgttcggctgcggcgagcggtatcagctcactcaaaggcggtaatacggttatccacagaatcaggggataacgcaggaaagaacatgtgagcaaaaggccagcaaaaggccaggaaccgtaaaaaggccgcgttgctggcgtttttccataggctccgcccccctgacgagcatcacaaaaatcgacgctcaagtcagaggtggcgaaacccgacaggactataaagataccaggcgtttccccctggaagctccctcgtgcgctctcctgttccgaccctgccgcttaccggatacctgtccgcctttctcccttcgggaagcgtggcgctttctcatagctcacgctgtaggtatctcagttcggtgtaggtcgttcgctccaagctgggctgtgtgcacgaaccccccgttcagcccgaccgctgcgccttatccggtaactatcgtcttgagtccaacccggtaagacacgacttatcgccactggcagcagccactggtaacaggattagcagagcgaggtatgtaggcggtgctacagagttcttgaagtggtggcctaactacggctacactagaagaacagtatttggtatctgcgctctgctgaagccagttaccttcggaaaaagagttggtagctcttgatccggcaaacaaaccaccgctggtagcggtttttttgtttgcaagcagcagattacgcgcagaaaaaaaggatctcaagaagatcctttgatcttttctacggggtctgacgctcagtggaacgaaaactcacgttaagggattttggtcatgagattatcaaaaaggatcttcacctagatccttttaaattaaaaatgaagttttaaatcaatctaaagtatatatgagtaaacttggtctgacagttaccaatgcttaatcagtgaggcacctatctcagcgatctgtctatttcgttcatccatagttgcctgactccccgtcgtgtagataactacgatacgggagggcttaccatctggccccagtgctgcaatgataccgcgagacccacgctcaccggctccagatttatcagcaataaaccagccagccggaagggccgagcgcagaagtggtcctgcaactttatccgcctccatccagtctattaattgttgccgggaagctagagtaagtagttcgccagttaatagtttgcgcaacgttgttgccattgctacaggcatcgtggtgtcacgctcgtcgtttggtatggcttcattcagctccggttcccaacgatcaaggcgagttacatgatcccccatgttgtgcaaaaaagcggttagctccttcggtcctccgatcgttgtcagaagtaagttggccgcagtgttatcactcatggttatggcagcactgcataattctcttactgtcatgccatccgtaagatgcttttctgtgactggtgagtactcaaccaagtcattctgagaatagtgtatgcggcgaccgagttgctcttgcccggcgtcaatacgggataataccgcgccacatagcagaactttaaaagtgctcatcattggaaaacgttcttcggggcgaaaactctcaaggatcttaccgctgttgagatccagttcgatgtaacccactcgtgcacccaactgatcttcagcatcttttactttcaccagcgtttctgggtgagcaaaaacaggaaggcaaaatgccgcaaaaaagggaataagggcgacacggaaatgttgaatactcatactcttcctttttcaatattattgaagcatttatcagggttattgtctcatgagcggatacatatttgaatgtatttagaaaaataaacaaataggggttccgcgcacatttccccgaaaagtgccacctgacgtc

SEQ ID NO: 15 - DNA, 1413 bp, Artificial Sequence
  Heavy chain aCD20 (Ab1)
atgggatggagtctgatattgttattccttgttgctgtcgcaacgcgggtcctgagtcaagtgcagctgcaacaacctggcgcagaactcgtgaagcccggtgcttccgttaagatgagctgtaaggcgtccggttataccttcacatcttacaacatgcattgggtgaagcagacccccggacgaggcctcgaatggatcggggccatttacccagggaatggagatactagctataatcagaagttcaaagggaaggccaccttgacagccgacaagtctagcagcaccgcctatatgcagctatcatcacttactagcgaagattccgccgtctactactgtgctaggtccacctactacggcggagattggtattttaacgtgtggggcgcaggcactacagtaaccgtgtctgcagcctcaaccaagggcccatcggtcttccccctggcaccctcctccaagagcacctctgggggcacagcggccctgggctgcctggtcaaggactacttccccgaaccggtgacggtgtcgtggaactcaggcgccctgaccagcggcgtgcacaccttcccggctgtcctacagtcctcaggactctactccctcagcagcgtggtgaccgtgccctccagcagcttgggcacccagacctacatctgcaacgtgaatcacaagcccagcaacaccaaggtggacaagaaagttgagcccaaatcttgtgacaaaactcacacatgcccaccgtgcccagcacctgaactcctggggggaccgtcagtcttcctcttccccccaaaacccaaggacaccctcatgatctcccggacccctgaggtcacatgcgtggtggtggacgtgagccacgaagaccctgaggtcaagttcaactggtacgtggacggcgtggaggtgcataatgccaagacaaagccgcgggaggagcagtacaacagcacgtaccgtgtggtcagcgtcctcaccgtcctgcaccaggactggctgaatggcaaggagtacaagtgcaaggtctccaacaaagccctcccagcccccatcgagaaaaccatctccaaagccaaagggcagccccgagaaccacaggtgtacaccctgcccccatcccgggatgagctgaccaagaaccaggtcagcctgacctgcctggtcaaaggcttctatcccagcgacatcgccgtggagtgggagagcaatgggcagccggagaacaactacaagaccacgcctcccgttctggactccgacggctccttcttcctctacagcaagctcaccgtggacaagagcaggtggcagcaggggaacgtcttctcatgctccgtgatgcatgaggctctgcacaaccactacacacagaagagcctctccctgtctccgggtaaatga

SEQ ID NO: 16 - DNA, 708 bp, Artificial Sequence
  Light chain aCD20 (Ab1)
atggattttcaggtgcaaatcatttccttcctattgatcagtgcttcagttattatgtcaaggggccagatcgtgctctctcagagccccgctatcttaagtgcatcccctggcgaaaaggtaacaatgacttgtcgagcctcctcttccgttagttatatccactggttccagcagaaacccggaagctcacctaagccatggatatacgcgaccagcaatcttgcaagcggggtgcctgtcagattcagcggcagcggaagcggtacctcttattctctcaccatctcccgggtcgaagccgaggacgcagccacgtactactgccagcagtggacatccaatccacccactttcggtgggggaaccaagctggaaatcaaacggactgttgcggcaccatctgtcttcatcttcccgccatctgatgagcagttgaaatctggaactgcctctgttgtgtgcctgctgaataacttctatcccagagaggccaaagtacagtggaaggtggataacgccctccaatcgggtaactcccaggagagtgtcacagagcaggacagcaaggacagcacctacagcctcagcagcaccctgacgctgagcaaagcagactacgagaaacacaaagtctacgcctgcgaagtcacccatcagggcctgagctcgcccgtcacaaagagcttcaacaggggagagtgttga

SEQ ID NO: 17 - DNA, 588 bp, Artificial Sequence
  IRES sequence
gccgcccctctccctcccccccccctaacgttactggccgaagccgcttggaataaggccggtgtgcgtttgtctatatgttattttccaccatattgccgtcttttggcaatgtgagggcccggaaacctggccctgtcttcttgacgagcattcctaggggtctttcccctctcgccaaaggaatgcaaggtctgttgaatgtcgtgaaggaagcagttcctctggaagcttcttgaagacaaacaacgtctgtagcgaccctttgcaggcagcggaaccccccacctggcgacaggtgcctctgcggccaaaagccacgtgtataagatacacctgcaaaggcggcacaaccccagtgccacgttgtgagttggatagttgtggaaagagtcaaatggctctcctcaagcgtattcaacaaggggctgaaggatgcccagaaggtaccccattgtatgggatctgatctggggcctcggtacacatgctttacatgtgtttagtcgaggttaaaaaaacgtctaggccccccgaaccacggggacgtggttttcctttgaaaaacacgatgataatatggccaca

SEQ ID NO: 18 - DNA, 2765 bp, Artificial Sequence
  Heavy Chain aCD20(Ab1)-IRES-Light Chain aCD20(Ab1)
atgggatggagtctgatattgttattccttgttgctgtcgcaacgcgggtcctgagtcaagtgcagctgcaacaacctggcgcagaactcgtgaagcccggtgcttccgttaagatgagctgtaaggcgtccggttataccttcacatcttacaacatgcattgggtgaagcagacccccggacgaggcctcgaatggatcggggccatttacccagggaatggagatactagctataatcagaagttcaaagggaaggccaccttgacagccgacaagtctagcagcaccgcctatatgcagctatcatcacttactagcgaagattccgccgtctactactgtgctaggtccacctactacggcggagattggtattttaacgtgtggggcgcaggcactacagtaaccgtgtctgcagcctcaaccaagggcccatcggtcttccccctggcaccctcctccaagagcacctctgggggcacagcggccctgggctgcctggtcaaggactacttccccgaaccggtgacggtgtcgtggaactcaggcgccctgaccagcggcgtgcacaccttcccggctgtcctacagtcctcaggactctactccctcagcagcgtggtgaccgtgccctccagcagcttgggcacccagacctacatctgcaacgtgaatcacaagcccagcaacaccaaggtggacaagaaagttgagcccaaatcttgtgacaaaactcacacatgcccaccgtgcccagcacctgaactcctggggggaccgtcagtcttcctcttccccccaaaacccaaggacaccctcatgatctcccggacccctgaggtcacatgcgtggtggtggacgtgagccacgaagaccctgaggtcaagttcaactggtacgtggacggcgtggaggtgcataatgccaagacaaagccgcgggaggagcagtacaacagcacgtaccgtgtggtcagcgtcctcaccgtcctgcaccaggactggctgaatggcaaggagtacaagtgcaaggtctccaacaaagccctcccagcccccatcgagaaaaccatctccaaagccaaagggcagccccgagaaccacaggtgtacaccctgcccccatcccgggatgagctgaccaagaaccaggtcagcctgacctgcctggtcaaaggcttctatcccagcgacatcgccgtggagtgggagagcaatgggcagccggagaacaactacaagaccacgcctcccgttctggactccgacggctccttcttcctctacagcaagctcaccgtggacaagagcaggtggcagcaggggaacgtcttctcatgctccgtgatgcatgaggctctgcacaaccactacacacagaagagcctctccctgtctccgggtaaatgaacgcgtggttggatccctaccggtgctgcggccgcgcagttaacgccgcccctctccctcccccccccctaacgttactggccgaagccgcttggaataaggccggtgtgcgtttgtctatatgttattttccaccatattgccgtcttttggcaatgtgagggcccggaaacctggccctgtcttcttgacgagcattcctaggggtctttcccctctcgccaaaggaatgcaaggtctgttgaatgtcgtgaaggaagcagttcctctggaagcttcttgaagacaaacaacgtctgtagcgaccctttgcaggcagcggaaccccccacctggcgacaggtgcctctgcggccaaaagccacgtgtataagatacacctgcaaaggcggcacaaccccagtgccacgttgtgagttggatagttgtggaaagagtcaaatggctctcctcaagcgtattcaacaaggggctgaaggatgcccagaaggtaccccattgtatgggatctgatctggggcctcggtacacatgctttacatgtgtttagtcgaggttaaaaaaacgtctaggccccccgaaccacggggacgtggttttcctttgaaaaacacgatgataatatggccacacatatggccaccatggattttcaggtgcaaatcatttccttcctattgatcagtgcttcagttattatgtcaaggggccagatcgtgctctctcagagccccgctatcttaagtgcatcccctggcgaaaaggtaacaatgacttgtcgagcctcctcttccgttagttatatccactggttccagcagaaacccggaagctcacctaagccatggatatacgcgaccagcaatcttgcaagcggggtgcctgtcagattcagcggcagcggaagcggtacctcttattctctcaccatctcccgggtcgaagccgaggacgcagccacgtactactgccagcagtggacatccaatccacccactttcggtgggggaaccaagctggaaatcaaacggactgttgcggcaccatctgtcttcatcttcccgccatctgatgagcagttgaaatctggaactgcctctgttgtgtgcctgctgaataacttctatcccagagaggccaaagtacagtggaaggtggataacgccctccaatcgggtaactcccaggagagtgtcacagagcaggacagcaaggacagcacctacagcctcagcagcaccctgacgctgagcaaagcagactacgagaaacacaaagtctacgcctgcgaagtcacccatcagggcctgagctcgcccgtcacaaagagcttcaacaggggagagtgttga

SEQ ID NO: 19 - DNA, 7485 bp, Artificial Sequence
  Plasmid
gttggttttttgtgtgaatcgatagtactaacatacgctctccatcaaaacaaaacgaaacaaaacaaactagcaaaataggctgtccccagtgcaagtgcaggtgccagaacatttctctggcctaactggccggtacctgagctcgctagcctcgaggatatcaagatctgttgacattgattattgactagttattaatagtaatcaattacggggtcattagttcatagcccatatatggagttccgcgttacataacttacggtaaatggcccgcctggctgaccgcccaacgacccccgcccattgacgtcaataatgacgtatgttcccatagtaacgccaatagggactttccattgacgtcaatgggtggagtatttacggtaaactgcccacttggcagtacatcaagtgtatcatatgccaagtacgccccctattgacgtcaatgacggtaaatggcccgcctggcattatgcccagtacatgaccttatgggactttcctacttggcagtacatctacgtattagtcatcgctattaccatggtgatgcggttttggcagtacatcaatgggcgtggatagcggtttgactcacggggatttccaagtctccaccccattgacgtcaatgggagtttgttttggcaccaaaatcaacgggactttccaaaatgtcgtaacaactccgccccattgacgcaaatgggcggtaggcgtgtacggtgggaggtctatataagcagagctctctggctaactagagaacccactgcttactggcttatcgaaagcttcactatagggagacccaagctggctagccaccatgggatggagtctgatattgttattccttgttgctgtcgcaacgcgggtcctgagtcaagtgcagctgcaacaacctggcgcagaactcgtgaagcccggtgcttccgttaagatgagctgtaaggcgtccggttataccttcacatcttacaacatgcattgggtgaagcagacccccggacgaggcctcgaatggatcggggccatttacccagggaatggagatactagctataatcagaagttcaaagggaaggccaccttgacagccgacaagtctagcagcaccgcctatatgcagctatcatcacttactagcgaagattccgccgtctactactgtgctaggtccacctactacggcggagattggtattttaacgtgtggggcgcaggcactacagtaaccgtgtctgcagcctcaaccaagggcccatcggtcttccccctggcaccctcctccaagagcacctctgggggcacagcggccctgggctgcctggtcaaggactacttccccgaaccggtgacggtgtcgtggaactcaggcgccctgaccagcggcgtgcacaccttcccggctgtcctacagtcctcaggactctactccctcagcagcgtggtgaccgtgccctccagcagcttgggcacccagacctacatctgcaacgtgaatcacaagcccagcaacaccaaggtggacaagaaagttgagcccaaatcttgtgacaaaactcacacatgcccaccgtgcccagcacctgaactcctggggggaccgtcagtcttcctcttccccccaaaacccaaggacaccctcatgatctcccggacccctgaggtcacatgcgtggtggtggacgtgagccacgaagaccctgaggtcaagttcaactggtacgtggacggcgtggaggtgcataatgccaagacaaagccgcgggaggagcagtacaacagcacgtaccgtgtggtcagcgtcctcaccgtcctgcaccaggactggctgaatggcaaggagtacaagtgcaaggtctccaacaaagccctcccagcccccatcgagaaaaccatctccaaagccaaagggcagccccgagaaccacaggtgtacaccctgcccccatcccgggatgagctgaccaagaaccaggtcagcctgacctgcctggtcaaaggcttctatcccagcgacatcgccgtggagtgggagagcaatgggcagccggagaacaactacaagaccacgcctcccgttctggactccgacggctccttcttcctctacagcaagctcaccgtggacaagagcaggtggcagcaggggaacgtcttctcatgctccgtgatgcatgaggctctgcacaaccactacacacagaagagcctctccctgtctccgggtaaatgaacgcgtggttggatccctaccggtgctgcggccgcgcagttaacgccgcccctctccctcccccccccctaacgttactggccgaagccgcttggaataaggccggtgtgcgtttgtctatatgttattttccaccatattgccgtcttttggcaatgtgagggcccggaaacctggccctgtcttcttgacgagcattcctaggggtctttcccctctcgccaaaggaatgcaaggtctgttgaatgtcgtgaaggaagcagttcctctggaagcttcttgaagacaaacaacgtctgtagcgaccctttgcaggcagcggaaccccccacctggcgacaggtgcctctgcggccaaaagccacgtgtataagatacacctgcaaaggcggcacaaccccagtgccacgttgtgagttggatagttgtggaaagagtcaaatggctctcctcaagcgtattcaacaaggggctgaaggatgcccagaaggtaccccattgtatgggatctgatctggggcctcggtacacatgctttacatgtgtttagtcgaggttaaaaaaacgtctaggccccccgaaccacggggacgtggttttcctttgaaaaacacgatgataatatggccacacatatggccaccatggattttcaggtgcaaatcatttccttcctattgatcagtgcttcagttattatgtcaaggggccagatcgtgctctctcagagccccgctatcttaagtgcatcccctggcgaaaaggtaacaatgacttgtcgagcctcctcttccgttagttatatccactggttccagcagaaacccggaagctcacctaagccatggatatacgcgaccagcaatcttgcaagcggggtgcctgtcagattcagcggcagcggaagcggtacctcttattctctcaccatctcccgggtcgaagccgaggacgcagccacgtactactgccagcagtggacatccaatccacccactttcggtgggggaaccaagctggaaatcaaacggactgttgcggcaccatctgtcttcatcttcccgccatctgatgagcagttgaaatctggaactgcctctgttgtgtgcctgctgaataacttctatcccagagaggccaaagtacagtggaaggtggataacgccctccaatcgggtaactcccaggagagtgtcacagagcaggacagcaaggacagcacctacagcctcagcagcaccctgacgctgagcaaagcagactacgagaaacacaaagtctacgcctgcgaagtcacccatcagggcctgagctcgcccgtcacaaagagcttcaacaggggagagtgttgaggatccactagtccagtgtggtggaattcgtgtaataattctagagtcggggcggccggccgcttcgagcagacatgataagatacattgatgagtttggacaaaccacaactagaatgcagtgaaaaaaatgctttatttgtgaaatttgtgatgctattgctttatttgtaaccattataagctgcaataaacaagttaacaacaacaattgcattcattttatgtttcaggttcagggggaggtgtgggaggttttttaaagcaagtaaaacctctacaaatgtggtaaaatcgataaggatccgtttgcgtattgggcgctcttccgctgatctgcgcagcaccatggcctgaaataacctctgaaagaggaacttggttagctaccttctgaggcggaaagaaccagctgtggaatgtgtgtcagttagggtgtggaaagtccccaggctccccagcaggcagaagtatgcaaagcatgcatctcaattagtcagcaaccaggtgtggaaagtccccaggctccccagcaggcagaagtatgcaaagcatgcatctcaattagtcagcaaccatagtcccgcccctaactccgcccatcccgcccctaactccgcccagttccgcccattctccgccccatggctgactaattttttttatttatgcagaggccgaggccgcctctgcctctgagctattccagaagtagtgaggaggcttttttggaggcctaggcttttgcaaaaagctcgattcttctgacactagcgccaccatgatcgaacaagacggcctccatgctggcagtcccgcagcttgggtcgaacgcttgttcgggtacgactgggcccagcagaccatcggatgtagcgatgcggccgtgttccgtctaagcgctcaaggccggcccgtgctgttcgtgaagaccgacctgagcggcgccctgaacgagcttcaagacgaggctgcccgcctgagctggctggccaccaccggcgtaccctgcgccgctgtgttggatgttgtgaccgaagccggccgggactggctgctgctgggcgaggtccctggccaggatctgctgagcagccaccttgcccccgctgagaaggtttctatcatggccgatgcaatgcggcgcctgcacaccctggaccccgctacctgccccttcgaccaccaggctaagcatcggatcgagcgtgctcggacccgcatggaggccggcctggtggaccaggacgacctggacgaggagcatcagggcctggcccccgctgaactgttcgcccgactgaaagcccgcatgccggacggtgaggacctggttgtcacacacggagatgcctgcctccctaacatcatggtcgagaatggccgcttctccggcttcatcgactgcggtcgcctaggagttgccgaccgctaccaggacatcgccctggccacccgcgacatcgctgaggagcttggcggcgagtgggccgaccgcttcttagtcttgtacggcatcgcagctcccgacagccagcgcatcgccttctaccgcttgctcgacgagttcttttaatgatctagaaccggtcatggccgcaataaaatatctttattttcattacatctgtgtgttggttttttgtgtgttcgaactagatgctgtcgaccgatgcccttgagagccttcaacccagtcagctccttccggtgggcgcggggcatgactatcgtcgccgcacttatgactgtcttctttatcatgcaactcgtaggacaggtgccggcagcgctcttccgcttcctcgctcactgactcgctgcgctcggtcgttcggctgcggcgagcggtatcagctcactcaaaggcggtaatacggttatccacagaatcaggggataacgcaggaaagaacatgtgagcaaaaggccagcaaaaggccaggaaccgtaaaaaggccgcgttgctggcgtttttccataggctccgcccccctgacgagcatcacaaaaatcgacgctcaagtcagaggtggcgaaacccgacaggactataaagataccaggcgtttccccctggaagctccctcgtgcgctctcctgttccgaccctgccgcttaccggatacctgtccgcctttctcccttcgggaagcgtggcgctttctcatagctcacgctgtaggtatctcagttcggtgtaggtcgttcgctccaagctgggctgtgtgcacgaaccccccgttcagcccgaccgctgcgccttatccggtaactatcgtcttgagtccaacccggtaagacacgacttatcgccactggcagcagccactggtaacaggattagcagagcgaggtatgtaggcggtgctacagagttcttgaagtggtggcctaactacggctacactagaagaacagtatttggtatctgcgctctgctgaagccagttaccttcggaaaaagagttggtagctcttgatccggcaaacaaaccaccgctggtagcggtggtttttttgtttgcaagcagcagattacgcgcagaaaaaaaggatctcaagaagatcctttgatcttttctacggggtctgacgctcagtggaacgaaaactcacgttaagggattttggtcatgagattatcaaaaaggatcttcacctagatccttttaaattaaaaatgaagttttaaatcaatctaaagtatatatgagtaaacttggtctgacagcggccgcaaatgctaaaccactgcagtggttaccagtgcttgatcagtgaggcaccgatctcagcgatctgcctatttcgttcgtccatagtggcctgactccccgtcgtgtagatcactacgattcgtgagggcttaccatcaggccccagcgcagcaatgatgccgcgagagccgcgttcaccggcccccgatttgtcagcaatgaaccagccagcagggagggccgagcgaagaagtggtcctgctactttgtccgcctccatccagtctatgagctgctgtcgtgatgctagagtaagaagttcgccagtgagtagtttccgaagagttgtggccattgctactggcatcgtggtatcacgctcgtcgttcggtatggcttcgttcaactctggttcccagcggtcaagccgggtcacatgatcacccatattatgaagaaatgcagtcagctccttagggcctccgatcgttgtcagaagtaagttggccgcggtgttgtcgctcatggtaatggcagcactacacaattctcttaccgtcatgccatccgtaagatgcttttccgtgaccggcgagtactcaaccaagtcgttttgtgagtagtgtatacggcgaccaagctgctcttgcccggcgtctatacgggacaacaccgcgccacatagcagtactttgaaagtgctcatcatcgggaatcgttcttcggggcggaaagactcaaggatcttgccgctattgagatccagttcgatatagcccactcttgcacccagttgatcttcagcatcttttactttcaccagcgtttcggggtgtgcaaaaacaggcaagcaaaatgccgcaaagaagggaatgagtgcgacacgaaaatgttggatgctcatactcgtcctttttcaatattattgaagcatttatcagggttactagtacgtctctcaaggataagtaagtaatattaaggtacgggaggtattggacaggccgcaataaaatatctttattttcattacatctgtgtgttggttttttgtgtgaatcgatagtactaacatacgctctccatcaaaacaaaacgaaacaaaacaaactagcaaaataggctgtccccagtgcaagtgcaggtgccagaacatttctct

SEQ ID NO: 20 - DNA, 8647 bp, Artificial Sequence
  Plasmid
gttggttttttgtgtgaatcgatagtactaacatacgctctccatcaaaacaaaacgaaacaaaacaaactagcaaaataggctgtccccagtgcaagtgcaggtgccagaacatttctctggcctaactggccggtaccggagagggggtaaaaaaatgctgcactgtgcggctaggccggtgagtgagcggcgcggagccaatcagcgctcgccgttccgaaagttgccttttatggctcgagtggccgctgtggcgtcctataaaacccggcggcgcaacgcgcagccactgtcgagtccgcgtccacccgcgagcacaggcctttcgcagctctttcttcgccgctccacacccgccaccaggtaagcagggacaacaggcccagccggccacagccctcccgtgggcagtgaccgcgctgcagggtcgcgggggacactcggcgcggacaccggggaaggctggagggtggtgccgggccgcggagcggacactttcagatccaactttcagtccagggtgtagaccctttacagccgcattgccacggtgtagacaccggtggacccgctctggctcagagcacgcggcttgggggaacccattagggtcgcagtgtgggcgctatgagagccgatgcagctttcgggtgttgaaccgtatctgcccaccttggggggaggacacaaggtcgggagccaaacgccacgatcatgccttggtggcccatgggtctttgtctaaaccggtttgcccatttggcttgccgggcgggcgggcgcggcgggcccggctcggccgggttgggggctgggttgccactgcgcttgcgcgctctatggctgggtattggggcgcgtgcacgctggggagggagcccttcctcttccccctctcccaagttaaacttgcgcgtgcgtattgagacttggagcgcggccaccggggttgggcgagggcggggccgttgtccggaaggggcggggtcgcagcggcttcggggcgcctgctcgcgcttcctgctgggtgtggtcgcctcccgcgcgcgcactagccgcccgccggcggggcgaaggcggggcttgcgcccgtttggggagggggcggaggcctggcttcctgccgtggggccgcctccggaccagcgtttgcctcttatggtaataacgcggccggcctgggcttcctttgtcccctgagtttgggcgcgcgccccctggcggcccgaggccgcggcttgccggaagtgggcagggcggcagcggctgcgcctagtggcccgccagtgaccgcgaccctcttttgtgccctgatatagttcgccagatctgttgacattgattattgactagttattaatagtaatcaattacggggtcattagttcatagcccatatatggagttccgcgttacataacttacggtaaatggcccgcctggctgaccgcccaacgacccccgcccattgacgtcaataatgacgtatgttcccatagtaacgccaatagggactttccattgacgtcaatgggtggagtatttacggtaaactgcccacttggcagtacatcaagtgtatcatatgccaagtacgccccctattgacgtcaatgacggtaaatggcccgcctggcattatgcccagtacatgaccttatgggactttcctacttggcagtacatctacgtattagtcatcgctattaccatggtgatgcggttttggcagtacatcaatgggcgtggatagcggtttgactcacggggatttccaagtctccaccccattgacgtcaatgggagtttgttttggcaccaaaatcaacgggactttccaaaatgtcgtaacaactccgccccattgacgcaaatgggcggtaggcgtgtacggtgggaggtctatataagcagagctctctggctaactagagaacccactgcttactggcttatcgaaagcttcactatagggagacccaagctggctagccaccatgggatggagtctgatattgttattccttgttgctgtcgcaacgcgggtcctgagtcaagtgcagctgcaacaacctggcgcagaactcgtgaagcccggtgcttccgttaagatgagctgtaaggcgtccggttataccttcacatcttacaacatgcattgggtgaagcagacccccggacgaggcctcgaatggatcggggccatttacccagggaatggagatactagctataatcagaagttcaaagggaaggccaccttgacagccgacaagtctagcagcaccgcctatatgcagctatcatcacttactagcgaagattccgccgtctactactgtgctaggtccacctactacggcggagattggtattttaacgtgtggggcgcaggcactacagtaaccgtgtctgcagcctcaaccaagggcccatcggtcttccccctggcaccctcctccaagagcacctctgggggcacagcggccctgggctgcctggtcaaggactacttccccgaaccggtgacggtgtcgtggaactcaggcgccctgaccagcggcgtgcacaccttcccggctgtcctacagtcctcaggactctactccctcagcagcgtggtgaccgtgccctccagcagcttgggcacccagacctacatctgcaacgtgaatcacaagcccagcaacaccaaggtggacaagaaagttgagcccaaatcttgtgacaaaactcacacatgcccaccgtgcccagcacctgaactcctggggggaccgtcagtcttcctcttccccccaaaacccaaggacaccctcatgatctcccggacccctgaggtcacatgcgtggtggtggacgtgagccacgaagaccctgaggtcaagttcaactggtacgtggacggcgtggaggtgcataatgccaagacaaagccgcgggaggagcagtacaacagcacgtaccgtgtggtcagcgtcctcaccgtcctgcaccaggactggctgaatggcaaggagtacaagtgcaaggtctccaacaaagccctcccagcccccatcgagaaaaccatctccaaagccaaagggcagccccgagaaccacaggtgtacaccctgcccccatcccgggatgagctgaccaagaaccaggtcagcctgacctgcctggtcaaaggcttctatcccagcgacatcgccgtggagtgggagagcaatgggcagccggagaacaactacaagaccacgcctcccgttctggactccgacggctccttcttcctctacagcaagctcaccgtggacaagagcaggtggcagcaggggaacgtcttctcatgctccgtgatgcatgaggctctgcacaaccactacacacagaagagcctctccctgtctccgggtaaatgaacgcgtggttggatccctaccggtgctgcggccgcgcagttaacgccgcccctctccctcccccccccctaacgttactggccgaagccgcttggaataaggccggtgtgcgtttgtctatatgttattttccaccatattgccgtcttttggcaatgtgagggcccggaaacctggccctgtcttcttgacgagcattcctaggggtctttcccctctcgccaaaggaatgcaaggtctgttgaatgtcgtgaaggaagcagttcctctggaagcttcttgaagacaaacaacgtctgtagcgaccctttgcaggcagcggaaccccccacctggcgacaggtgcctctgcggccaaaagccacgtgtataagatacacctgcaaaggcggcacaaccccagtgccacgttgtgagttggatagttgtggaaagagtcaaatggctctcctcaagcgtattcaacaaggggctgaaggatgcccagaaggtaccccattgtatgggatctgatctggggcctcggtacacatgctttacatgtgtttagtcgaggttaaaaaaacgtctaggccccccgaaccacggggacgtggttttcctttgaaaaacacgatgataatatggccacacatatggccaccatggattttcaggtgcaaatcatttccttcctattgatcagtgcttcagttattatgtcaaggggccagatcgtgctctctcagagccccgctatcttaagtgcatcccctggcgaaaaggtaacaatgacttgtcgagcctcctcttccgttagttatatccactggttccagcagaaacccggaagctcacctaagccatggatatacgcgaccagcaatcttgcaagcggggtgcctgtcagattcagcggcagcggaagcggtacctcttattctctcaccatctcccgggtcgaagccgaggacgcagccacgtactactgccagcagtggacatccaatccacccactttcggtgggggaaccaagctggaaatcaaacggactgttgcggcaccatctgtcttcatcttcccgccatctgatgagcagttgaaatctggaactgcctctgttgtgtgcctgctgaataacttctatcccagagaggccaaagtacagtggaaggtggataacgccctccaatcgggtaactcccaggagagtgtcacagagcaggacagcaaggacagcacctacagcctcagcagcaccctgacgctgagcaaagcagactacgagaaacacaaagtctacgcctgcgaagtcacccatcagggcctgagctcgcccgtcacaaagagcttcaacaggggagagtgttgaggatccactagtccagtgtggtggaattcgtgtaataattctagagtcggggcggccggccgcttcgagcagacatgataagatacattgatgagtttggacaaaccacaactagaatgcagtgaaaaaaatgctttatttgtgaaatttgtgatgctattgctttatttgtaaccattataagctgcaataaacaagttaacaacaacaattgcattcattttatgtttcaggttcagggggaggtgtgggaggttttttaaagcaagtaaaacctctacaaatgtggtaaaatcgataaggatccgtttgcgtattgggcgctcttccgctgatctgcgcagcaccatggcctgaaataacctctgaaagaggaacttggttagctaccttctgaggcggaaagaaccagctgtggaatgtgtgtcagttagggtgtggaaagtccccaggctccccagcaggcagaagtatgcaaagcatgcatctcaattagtcagcaaccaggtgtggaaagtccccaggctccccagcaggcagaagtatgcaaagcatgcatctcaattagtcagcaaccatagtcccgcccctaactccgcccatcccgcccctaactccgcccagttccgcccattctccgccccatggctgactaattttttttatttatgcagaggccgaggccgcctctgcctctgagctattccagaagtagtgaggaggcttttttggaggcctaggcttttgcaaaaagctcgattcttctgacactagcgccaccatgatcgaacaagacggcctccatgctggcagtcccgcagcttgggtcgaacgcttgttcgggtacgactgggcccagcagaccatcggatgtagcgatgcggccgtgttccgtctaagcgctcaaggccggcccgtgctgttcgtgaagaccgacctgagcggcgccctgaacgagcttcaagacgaggctgcccgcctgagctggctggccaccaccggcgtaccctgcgccgctgtgttggatgttgtgaccgaagccggccgggactggctgctgctgggcgaggtccctggccaggatctgctgagcagccaccttgcccccgctgagaaggtttctatcatggccgatgcaatgcggcgcctgcacaccctggaccccgctacctgccccttcgaccaccaggctaagcatcggatcgagcgtgctcggacccgcatggaggccggcctggtggaccaggacgacctggacgaggagcatcagggcctggcccccgctgaactgttcgcccgactgaaagcccgcatgccggacggtgaggacctggttgtcacacacggagatgcctgcctccctaacatcatggtcgagaatggccgcttctccggcttcatcgactgcggtcgcctaggagttgccgaccgctaccaggacatcgccctggccacccgcgacatcgctgaggagcttggcggcgagtgggccgaccgcttcttagtcttgtacggcatcgcagctcccgacagccagcgcatcgccttctaccgcttgctcgacgagttcttttaatgatctagaaccggtcatggccgcaataaaatatctttattttcattacatctgtgtgttggttttttgtgtgttcgaactagatgctgtcgaccgatgcccttgagagccttcaacccagtcagctccttccggtgggcgcggggcatgactatcgtcgccgcacttatgactgtcttctttatcatgcaactcgtaggacaggtgccggcagcgctcttccgcttcctcgctcactgactcgctgcgctcggtcgttcggctgcggcgagcggtatcagctcactcaaaggcggtaatacggttatccacagaatcaggggataacgcaggaaagaacatgtgagcaaaaggccagcaaaaggccaggaaccgtaaaaaggccgcgttgctggcgtttttccataggctccgcccccctgacgagcatcacaaaaatcgacgctcaagtcagaggtggcgaaacccgacaggactataaagataccaggcgtttccccctggaagctccctcgtgcgctctcctgttccgaccctgccgcttaccggatacctgtccgcctttctcccttcgggaagcgtggcgctttctcatagctcacgctgtaggtatctcagttcggtgtaggtcgttcgctccaagctgggctgtgtgcacgaaccccccgttcagcccgaccgctgcgccttatccggtaactatcgtcttgagtccaacccggtaagacacgacttatcgccactggcagcagccactggtaacaggattagcagagcgaggtatgtaggcggtgctacagagttcttgaagtggtggcctaactacggctacactagaagaacagtatttggtatctgcgctctgctgaagccagttaccttcggaaaaagagttggtagctcttgatccggcaaacaaaccaccgctggtagcggtggtttttttgtttgcaagcagcagattacgcgcagaaaaaaaggatctcaagaagatcctttgatcttttctacggggtctgacgctcagtggaacgaaaactcacgttaagggattttggtcatgagattatcaaaaaggatcttcacctagatccttttaaattaaaaatgaagttttaaatcaatctaaagtatatatgagtaaacttggtctgacagcggccgcaaatgctaaaccactgcagtggttaccagtgcttgatcagtgaggcaccgatctcagcgatctgcctatttcgttcgtccatagtggcctgactccccgtcgtgtagatcactacgattcgtgagggcttaccatcaggccccagcgcagcaatgatgccgcgagagccgcgttcaccggcccccgatttgtcagcaatgaaccagccagcagggagggccgagcgaagaagtggtcctgctactttgtccgcctccatccagtctatgagctgctgtcgtgatgctagagtaagaagttcgccagtgagtagtttccgaagagttgtggccattgctactggcatcgtggtatcacgctcgtcgttcggtatggcttcgttcaactctggttcccagcggtcaagccgggtcacatgatcacccatattatgaagaaatgcagtcagctccttagggcctccgatcgttgtcagaagtaagttggccgcggtgttgtcgctcatggtaatggcagcactacacaattctcttaccgtcatgccatccgtaagatgcttttccgtgaccggcgagtactcaaccaagtcgttttgtgagtagtgtatacggcgaccaagctgctcttgcccggcgtctatacgggacaacaccgcgccacatagcagtactttgaaagtgctcatcatcgggaatcgttcttcggggcggaaagactcaaggatcttgccgctattgagatccagttcgatatagcccactcttgcacccagttgatcttcagcatcttttactttcaccagcgtttcggggtgtgcaaaaacaggcaagcaaaatgccgcaaagaagggaatgagtgcgacacgaaaatgttggatgctcatactcgtcctttttcaatattattgaagcatttatcagggttactagtacgtctctcaaggataagtaagtaatattaaggtacgggaggtattggacaggccgcaataaaatatctttattttcattacatctgtgtgttggttttttgtgtgaatcgatagtactaacatacgctctccatcaaaacaaaacgaaacaaaacaaactagcaaaataggctgtccccagtgcaagtgcaggtgccagaacatttctct

SEQ ID NO: 21 - DNA, 8836 bp, Artificial Sequence
  Plasmid
gttggttttttgtgtgaatcgatagtactaacatacgctctccatcaaaacaaaacgaaacaaaacaaactagcaaaataggctgtccccagtgcaagtgcaggtgccagaacatttctctggcctaactggccggtaccggagagggggtaaaaaaatgctgcactgtgcggctaggccggtgagtgagcggcgcggagccaatcagcgctcgccgttccgaaagttgccttttatggctcgagtggccgctgtggcgtcctataaaacccggcggcgcaacgcgcagccactgtcgagtccgcgtccacccgcgagcacaggcctttcgcagctctttcttcgccgctccacacccgccaccaggtaagcagggacaacaggcccagccggccacagccctcccgtgggcagtgaccgcgctgcagggtcgcgggggacactcggcgcggacaccggggaaggctggagggtggtgccgggccgcggagcggacactttcagatccaactttcagtccagggtgtagaccctttacagccgcattgccacggtgtagacaccggtggacccgctctggctcagagcacgcggcttgggggaacccattagggtcgcagtgtgggcgctatgagagccgatgcagctttcgggtgttgaaccgtatctgcccaccttggggggaggacacaaggtcgggagccaaacgccacgatcatgccttggtggcccatgggtctttgtctaaaccggtttgcccatttggcttgccgggcgggcgggcgcggcgggcccggctcggccgggttgggggctgggttgccactgcgcttgcgcgctctatggctgggtattggggcgcgtgcacgctggggagggagcccttcctcttccccctctcccaagttaaacttgcgcgtgcgtattgagacttggagcgcggccaccggggttgggcgagggcggggccgttgtccggaaggggcggggtcgcagcggcttcggggcgcctgctcgcgcttcctgctgggtgtggtcgcctcccgcgcgcgcactagccgcccgccggcggggcgaaggcggggcttgcgcccgtttggggagggggcggaggcctggcttcctgccgtggggccgcctccggaccagcgtttgcctcttatggtaataacgcggccggcctgggcttcctttgtcccctgagtttgggcgcgcgccccctggcggcccgaggccgcggcttgccggaagtgggcagggcggcagcggctgcgcctagtggcccgccagtgaccgcgaccctcttttgtgccctgatatagttcgccgaattcgctagcagaacaggatgttctgatcaaagagatccaaagtcagaacacgttgttctagctaaaataacacattcagagaacatgctgttctgatcaaagagatccaaagtcagaacaaggtgttctagctaaaataacacattcagagaacatgatgttctgatcaaagagatccaaagtcgcggccgcgttgacattgattattgactagttattaatagtaatcaattacggggtcattagttcatagcccatatatggagttccgcgttacataacttacggtaaatggcccgcctggctgaccgcccaacgacccccgcccattgacgtcaataatgacgtatgttcccatagtaacgccaatagggactttccattgacgtcaatgggtggagtatttacggtaaactgcccacttggcagtacatcaagtgtatcatatgccaagtacgccccctattgacgtcaatgacggtaaatggcccgcctggcattatgcccagtacatgaccttatgggactttcctacttggcagtacatctacgtattagtcatcgctattaccatggtgatgcggttttggcagtacatcaatgggcgtggatagcggtttgactcacggggatttccaagtctccaccccattgacgtcaatgggagtttgttttggcaccaaaatcaacgggactttccaaaatgtcgtaacaactccgccccattgacgcaaatgggcggtaggcgtgtacggtgggaggtctatataagcagagctctctggctaactagagaacccactgcttactggcttatcgaaagcttcactatagggagacccaagctggctagccaccatgggatggagtctgatattgttattccttgttgctgtcgcaacgcgggtcctgagtcaagtgcagctgcaacaacctggcgcagaactcgtgaagcccggtgcttccgttaagatgagctgtaaggcgtccggttataccttcacatcttacaacatgcattgggtgaagcagacccccggacgaggcctcgaatggatcggggccatttacccagggaatggagatactagctataatcagaagttcaaagggaaggccaccttgacagccgacaagtctagcagcaccgcctatatgcagctatcatcacttactagcgaagattccgccgtctactactgtgctaggtccacctactacggcggagattggtattttaacgtgtggggcgcaggcactacagtaaccgtgtctgcagcctcaaccaagggcccatcggtcttccccctggcaccctcctccaagagcacctctgggggcacagcggccctgggctgcctggtcaaggactacttccccgaaccggtgacggtgtcgtggaactcaggcgccctgaccagcggcgtgcacaccttcccggctgtcctacagtcctcaggactctactccctcagcagcgtggtgaccgtgccctccagcagcttgggcacccagacctacatctgcaacgtgaatcacaagcccagcaacaccaaggtggacaagaaagttgagcccaaatcttgtgacaaaactcacacatgcccaccgtgcccagcacctgaactcctggggggaccgtcagtcttcctcttccccccaaaacccaaggacaccctcatgatctcccggacccctgaggtcacatgcgtggtggtggacgtgagccacgaagaccctgaggtcaagttcaactggtacgtggacggcgtggaggtgcataatgccaagacaaagccgcgggaggagcagtacaacagcacgtaccgtgtggtcagcgtcctcaccgtcctgcaccaggactggctgaatggcaaggagtacaagtgcaaggtctccaacaaagccctcccagcccccatcgagaaaaccatctccaaagccaaagggcagccccgagaaccacaggtgtacaccctgcccccatcccgggatgagctgaccaagaaccaggtcagcctgacctgcctggtcaaaggcttctatcccagcgacatcgccgtggagtgggagagcaatgggcagccggagaacaactacaagaccacgcctcccgttctggactccgacggctccttcttcctctacagcaagctcaccgtggacaagagcaggtggcagcaggggaacgtcttctcatgctccgtgatgcatgaggctctgcacaaccactacacacagaagagcctctccctgtctccgggtaaatgaacgcgtggttggatccctaccggtgctgcggccgcgcagttaacgccgcccctctccctcccccccccctaacgttactggccgaagccgcttggaataaggccggtgtgcgtttgtctatatgttattttccaccatattgccgtcttttggcaatgtgagggcccggaaacctggccctgtcttcttgacgagcattcctaggggtctttcccctctcgccaaaggaatgcaaggtctgttgaatgtcgtgaaggaagcagttcctctggaagcttcttgaagacaaacaacgtctgtagcgaccctttgcaggcagcggaaccccccacctggcgacaggtgcctctgcggccaaaagccacgtgtataagatacacctgcaaaggcggcacaaccccagtgccacgttgtgagttggatagttgtggaaagagtcaaatggctctcctcaagcgtattcaacaaggggctgaaggatgcccagaaggtaccccattgtatgggatctgatctggggcctcggtacacatgctttacatgtgtttagtcgaggttaaaaaaacgtctaggccccccgaaccacggggacgtggttttcctttgaaaaacacgatgataatatggccacacatatggccaccatggattttcaggtgcaaatcatttccttcctattgatcagtgcttcagttattatgtcaaggggccagatcgtgctctctcagagccccgctatcttaagtgcatcccctggcgaaaaggtaacaatgacttgtcgagcctcctcttccgttagttatatccactggttccagcagaaacccggaagctcacctaagccatggatatacgcgaccagcaatcttgcaagcggggtgcctgtcagattcagcggcagcggaagcggtacctcttattctctcaccatctcccgggtcgaagccgaggacgcagccacgtactactgccagcagtggacatccaatccacccactttcggtgggggaaccaagctggaaatcaaacggactgttgcggcaccatctgtcttcatcttcccgccatctgatgagcagttgaaatctggaactgcctctgttgtgtgcctgctgaataacttctatcccagagaggccaaagtacagtggaaggtggataacgccctccaatcgggtaactcccaggagagtgtcacagagcaggacagcaaggacagcacctacagcctcagcagcaccctgacgctgagcaaagcagactacgagaaacacaaagtctacgcctgcgaagtcacccatcagggcctgagctcgcccgtcacaaagagcttcaacaggggagagtgttgaggatccactagtccagtgtggtggaattcgtgtaataattctagagtcggggcggccggccgcttcgagcagacatgataagatacattgatgagtttggacaaaccacaactagaatgcagtgaaaaaaatgctttatttgtgaaatttgtgatgctattgctttatttgtaaccattataagctgcaataaacaagttaacaacaacaattgcattcattttatgtttcaggttcagggggaggtgtgggaggttttttaaagcaagtaaaacctctacaaatgtggtaaaatcgataaggatccgtttgcgtattgggcgctcttccgctgatctgcgcagcaccatggcctgaaataacctctgaaagaggaacttggttagctaccttctgaggcggaaagaaccagctgtggaatgtgtgtcagttagggtgtggaaagtccccaggctccccagcaggcagaagtatgcaaagcatgcatctcaattagtcagcaaccaggtgtggaaagtccccaggctccccagcaggcagaagtatgcaaagcatgcatctcaattagtcagcaaccatagtcccgcccctaactccgcccatcccgcccctaactccgcccagttccgcccattctccgccccatggctgactaattttttttatttatgcagaggccgaggccgcctctgcctctgagctattccagaagtagtgaggaggcttttttggaggcctaggcttttgcaaaaagctcgattcttctgacactagcgccaccatgatcgaacaagacggcctccatgctggcagtcccgcagcttgggtcgaacgcttgttcgggtacgactgggcccagcagaccatcggatgtagcgatgcggccgtgttccgtctaagcgctcaaggccggcccgtgctgttcgtgaagaccgacctgagcggcgccctgaacgagcttcaagacgaggctgcccgcctgagctggctggccaccaccggcgtaccctgcgccgctgtgttggatgttgtgaccgaagccggccgggactggctgctgctgggcgaggtccctggccaggatctgctgagcagccaccttgcccccgctgagaaggtttctatcatggccgatgcaatgcggcgcctgcacaccctggaccccgctacctgccccttcgaccaccaggctaagcatcggatcgagcgtgctcggacccgcatggaggccggcctggtggaccaggacgacctggacgaggagcatcagggcctggcccccgctgaactgttcgcccgactgaaagcccgcatgccggacggtgaggacctggttgtcacacacggagatgcctgcctccctaacatcatggtcgagaatggccgcttctccggcttcatcgactgcggtcgcctaggagttgccgaccgctaccaggacatcgccctggccacccgcgacatcgctgaggagcttggcggcgagtgggccgaccgcttcttagtcttgtacggcatcgcagctcccgacagccagcgcatcgccttctaccgcttgctcgacgagttcttttaatgatctagaaccggtcatggccgcaataaaatatctttattttcattacatctgtgtgttggttttttgtgtgttcgaactagatgctgtcgaccgatgcccttgagagccttcaacccagtcagctccttccggtgggcgcggggcatgactatcgtcgccgcacttatgactgtcttctttatcatgcaactcgtaggacaggtgccggcagcgctcttccgcttcctcgctcactgactcgctgcgctcggtcgttcggctgcggcgagcggtatcagctcactcaaaggcggtaatacggttatccacagaatcaggggataacgcaggaaagaacatgtgagcaaaaggccagcaaaaggccaggaaccgtaaaaaggccgcgttgctggcgtttttccataggctccgcccccctgacgagcatcacaaaaatcgacgctcaagtcagaggtggcgaaacccgacaggactataaagataccaggcgtttccccctggaagctccctcgtgcgctctcctgttccgaccctgccgcttaccggatacctgtccgcctttctcccttcgggaagcgtggcgctttctcatagctcacgctgtaggtatctcagttcggtgtaggtcgttcgctccaagctgggctgtgtgcacgaaccccccgttcagcccgaccgctgcgccttatccggtaactatcgtcttgagtccaacccggtaagacacgacttatcgccactggcagcagccactggtaacaggattagcagagcgaggtatgtaggcggtgctacagagttcttgaagtggtggcctaactacggctacactagaagaacagtatttggtatctgcgctctgctgaagccagttaccttcggaaaaagagttggtagctcttgatccggcaaacaaaccaccgctggtagcggtggtttttttgtttgcaagcagcagattacgcgcagaaaaaaaggatctcaagaagatcctttgatcttttctacggggtctgacgctcagtggaacgaaaactcacgttaagggattttggtcatgagattatcaaaaaggatcttcacctagatccttttaaattaaaaatgaagttttaaatcaatctaaagtatatatgagtaaacttggtctgacagcggccgcaaatgctaaaccactgcagtggttaccagtgcttgatcagtgaggcaccgatctcagcgatctgcctatttcgttcgtccatagtggcctgactccccgtcgtgtagatcactacgattcgtgagggcttaccatcaggccccagcgcagcaatgatgccgcgagagccgcgttcaccggcccccgatttgtcagcaatgaaccagccagcagggagggccgagcgaagaagtggtcctgctactttgtccgcctccatccagtctatgagctgctgtcgtgatgctagagtaagaagttcgccagtgagtagtttccgaagagttgtggccattgctactggcatcgtggtatcacgctcgtcgttcggtatggcttcgttcaactctggttcccagcggtcaagccgggtcacatgatcacccatattatgaagaaatgcagtcagctccttagggcctccgatcgttgtcagaagtaagttggccgcggtgttgtcgctcatggtaatggcagcactacacaattctcttaccgtcatgccatccgtaagatgcttttccgtgaccggcgagtactcaaccaagtcgttttgtgagtagtgtatacggcgaccaagctgctcttgcccggcgtctatacgggacaacaccgcgccacatagcagtactttgaaagtgctcatcatcgggaatcgttcttcggggcggaaagactcaaggatcttgccgctattgagatccagttcgatatagcccactcttgcacccagttgatcttcagcatcttttactttcaccagcgtttcggggtgtgcaaaaacaggcaagcaaaatgccgcaaagaagggaatgagtgcgacacgaaaatgttggatgctcatactcgtcctttttcaatattattgaagcatttatcagggttactagtacgtctctcaaggataagtaagtaatattaaggtacgggaggtattggacaggccgcaataaaatatctttattttcattacatctgtgtgttggttttttgtgtgaatcgatagtactaacatacgctctccatcaaaacaaaacgaaacaaaacaaactagcaaaataggctgtccccagtgcaagtgcaggtgccagaacatttctct

SEQ ID NO: 22 - DNA, 1416 bp, Artificial Sequence
  Heavy chain Ab2
atggcctgggtgtggaccttgctattcctgatgacagctgcccagagtgcccaagcacagatccagttggaacagtctggacctgagctgaagaagcctggagagacagtcaagatctcctgcaaggcttctggatatatcttcacaaacaatggaatgagctgggtgaaacaggctccaggaaagggtttaaagtggatgggctgggtaaacacctacactggtaagtcaacatatgctgatgacttcaagggacggtttgccttctctttggaaacctcagccagcactgcctatttgcaaatcaacaacctcaaaaatgaggacacggctacatatttctgtgcaagagactctactacggtaatagctacgaatgctatggacttctggggtcaaggaacctcagtcaccgtctcctcagcctcaaccaagggcccatcggtcttccccctggcaccctcctccaagagcacctctgggggcacagcggccctgggctgcctggtcaaggactacttccccgaaccggtgacggtgtcgtggaactcaggcgccctgaccagcggcgtgcacaccttcccggctgtcctacagtcctcaggactctactccctcagcagcgtggtgaccgtgccctccagcagcttgggcacccagacctacatctgcaacgtgaatcacaagcccagcaacaccaaggtggacaagaaagttgagcccaaatcttgtgacaaaactcacacatgcccaccgtgcccagcacctgaactcctggggggaccgtcagtcttcctcttccccccaaaacccaaggacaccctcatgatctcccggacccctgaggtcacatgcgtggtggtggacgtgagccacgaagaccctgaggtcaagttcaactggtacgtggacggcgtggaggtgcataatgccaagacaaagccgcgggaggagcagtacaacagcacgtaccgtgtggtcagcgtcctcaccgtcctgcaccaggactggctgaatggcaaggagtacaagtgcaaggtctccaacaaagccctcccagcccccatcgagaaaaccatctccaaagccaaagggcagccccgagaaccacaggtgtacaccctgcccccatcccgggatgagctgaccaagaaccaggtcagcctgacctgcctggtcaaaggcttctatcccagcgacatcgccgtggagtgggagagcaatgggcagccggagaacaactacaagaccacgcctcccgttctggactccgacggctccttcttcctctacagcaagctcaccgtggacaagagcaggtggcagcaggggaacgtcttctcatgctccgtgatgcatgaggctctgcacaaccactacacacagaagagcctctccctgtctccgggtaaatga

SEQ ID NO: 23 - DNA, 720 bp, Artificial Sequence
  Light chain Ab2
atggattcacaggcccaggttcttatattgctgctgctatgggtatctggtacctgtggggacattgtgatgtcacagtctccatcctccctggctgtgtcagcaggagagaaggtcactatgagctgcaaatccagtcagagtctgctcaacagtagaacccgaaagaactacttggcttggtaccagcagaaaccagggcagtctcctaaactgctgatctactgggcatccattagggaatctggggtccctgatcgcttcacaggcagtggatctgggacagatttcactctcaccatcagcagtgtgcaggctgaagacctggcagtttattactgcaagcaatcttataatctgtggacgttcggtggaggcaccaagctggaaatcaaacggactgttgcggcaccatctgtcttcatcttcccgccatctgatgagcagttgaaatctggaactgcctctgttgtgtgcctgctgaataacttctatcccagagaggccaaagtacagtggaaggtggataacgccctccaatcgggtaactcccaggagagtgtcacagagcaggacagcaaggacagcacctacagcctcagcagcaccctgacgctgagcaaagcagactacgagaaacacaaagtctacgcctgcgaagtcacccatcagggcctgagctcgcccgtcacaaagagcttcaacaggggagagtgttga

SEQ ID NO: 24 - DNA, 7733 bp, Artificial Sequence
  Plasmid
gttggttttttgtgtgaatcgatagtactaacatacgctctccatcaaaacaaaacgaaacaaaacaaactagcaaaataggctgtccccagtgcaagtgcaggtgccagaacatttctctggcctaactggccggtaccggagagggggtaaaaaaatgctgcactgtgcggctaggccggtgagtgagcggcgcggagccaatcagcgctcgccgttccgaaagttgccttttatggctcgagtggccgctgtggcgtcctataaaacccggcggcgcaacgcgcagccactgtcgagtccgcgtccacccgcgagcacaggcctttcgcagctctttcttcgccgctccacacccgccaccaggtaagcagggacaacaggcccagccggccacagccctcccgtgggcagtgaccgcgctgcagggtcgcgggggacactcggcgcggacaccggggaaggctggagggtggtgccgggccgcggagcggacactttcagatccaactttcagtccagggtgtagaccctttacagccgcattgccacggtgtagacaccggtggacccgctctggctcagagcacgcggcttgggggaacccattagggtcgcagtgtgggcgctatgagagccgatgcagctttcgggtgttgaaccgtatctgcccaccttggggggaggacacaaggtcgggagccaaacgccacgatcatgccttggtggcccatgggtctttgtctaaaccggtttgcccatttggcttgccgggcgggcgggcgcggcgggcccggctcggccgggttgggggctgggttgccactgcgcttgcgcgctctatggctgggtattggggcgcgtgcacgctggggagggagcccttcctcttccccctctcccaagttaaacttgcgcgtgcgtattgagacttggagcgcggccaccggggttgggcgagggcggggccgttgtccggaaggggcggggtcgcagcggcttcggggcgcctgctcgcgcttcctgctgggtgtggtcgcctcccgcgcgcgcactagccgcccgccggcggggcgaaggcggggcttgcgcccgtttggggagggggcggaggcctggcttcctgccgtggggccgcctccggaccagcgtttgcctcttatggtaataacgcggccggcctgggcttcctttgtcccctgagtttgggcgcgcgccccctggcggcccgaggccgcggcttgccggaagtgggcagggcggcagcggctgcgcctagtggcccgccagtgaccgcgaccctcttttgtgccctgatatagttcgccgaattcgctagcagaacaggatgttctgatcaaagagatccaaagtcagaacacgttgttctagctaaaataacacattcagagaacatgctgttctgatcaaagagatccaaagtcagaacaaggtgttctagctaaaataacacattcagagaacatgatgttctgatcaaagagatccaaagtcgcggccgcgttgacattgattattgactagttattaatagtaatcaattacggggtcattagttcatagcccatatatggagttccgcgttacataacttacggtaaatggcccgcctggctgaccgcccaacgacccccgcccattgacgtcaataatgacgtatgttcccatagtaacgccaatagggactttccattgacgtcaatgggtggagtatttacggtaaactgcccacttggcagtacatcaagtgtatcatatgccaagtacgccccctattgacgtcaatgacggtaaatggcccgcctggcattatgcccagtacatgaccttatgggactttcctacttggcagtacatctacgtattagtcatcgctattaccatggtgatgcggttttggcagtacatcaatgggcgtggatagcggtttgactcacggggatttccaagtctccaccccattgacgtcaatgggagtttgttttggcaccaaaatcaacgggactttccaaaatgtcgtaacaactccgccccattgacgcaaatgggcggtaggcgtgtacggtgggaggtctatataagcagagctctctggctaactagagaacccactgcttactggcttatcgaaagcttcaccatggcctgggtgtggaccttgctattcctgatgacagctgcccagagtgcccaagcacagatccagttggaacagtctggacctgagctgaagaagcctggagagacagtcaagatctcctgcaaggcttctggatatatcttcacaaacaatggaatgagctgggtgaaacaggctccaggaaagggtttaaagtggatgggctgggtaaacacctacactggtaagtcaacatatgctgatgacttcaagggacggtttgccttctctttggaaacctcagccagcactgcctatttgcaaatcaacaacctcaaaaatgaggacacggctacatatttctgtgcaagagactctactacggtaatagctacgaatgctatggacttctggggtcaaggaacctcagtcaccgtctcctcagcctcaaccaagggcccatcggtcttccccctggcaccctcctccaagagcacctctgggggcacagcggccctgggctgcctggtcaaggactacttccccgaaccggtgacggtgtcgtggaactcaggcgccctgaccagcggcgtgcacaccttcccggctgtcctacagtcctcaggactctactccctcagcagcgtggtgaccgtgccctccagcagcttgggcacccagacctacatctgcaacgtgaatcacaagcccagcaacaccaaggtggacaagaaagttgagcccaaatcttgtgacaaaactcacacatgcccaccgtgcccagcacctgaactcctggggggaccgtcagtcttcctcttccccccaaaacccaaggacaccctcatgatctcccggacccctgaggtcacatgcgtggtggtggacgtgagccacgaagaccctgaggtcaagttcaactggtacgtggacggcgtggaggtgcataatgccaagacaaagccgcgggaggagcagtacaacagcacgtaccgtgtggtcagcgtcctcaccgtcctgcaccaggactggctgaatggcaaggagtacaagtgcaaggtctccaacaaagccctcccagcccccatcgagaaaaccatctccaaagccaaagggcagccccgagaaccacaggtgtacaccctgcccccatcccgggatgagctgaccaagaaccaggtcagcctgacctgcctggtcaaaggcttctatcccagcgacatcgccgtggagtgggagagcaatgggcagccggagaacaactacaagaccacgcctcccgttctggactccgacggctccttcttcctctacagcaagctcaccgtggacaagagcaggtggcagcaggggaacgtcttctcatgctccgtgatgcatgaggctctgcacaaccactacacacagaagagcctctccctgtctccgggtaaatgaacgcgtgactctggtgtgagcgaattcgtgtaataattctagagtcggggcggccggccgcttcgagcagacatgataagatacattgatgagtttggacaaaccacaactagaatgcagtgaaaaaaatgctttatttgtgaaatttgtgatgctattgctttatttgtaaccattataagctgcaataaacaagttaacaacaacaattgcattcattttatgtttcaggttcagggggaggtgtgggaggttttttaaagcaagtaaaacctctacaaatgtggtaaaatcgataaggatccgtttgcgtattgggcgctcttccgctgatctgcgtaataattctagagtcggggcggccggccgcttcgagcagacatgataagatacattgatgagtttggacaaaccacaactagaatgcagtgaaaaaaatgctttatttgtgaaatttgtgatgctattgctttatttgtaaccattataagctgcaataaacaagttaacaacaacaattgcattcattttatgtttcaggttcagggggaggtgtgggaggttttttaaagcaagtaaaacctctacaaatgtggtaaaatcgataaggatccgcagcaccatggcctgaaataacctctgaaagaggaacttggttagctaccttctgaggcggaaagaaccagctgtggaatgtgtgtcagttagggtgtggaaagtccccaggctccccagcaggcagaagtatgcaaagcatgcatctcaattagtcagcaaccaggtgtggaaagtccccaggctccccagcaggcagaagtatgcaaagcatgcatctcaattagtcagcaaccatagtcccgcccctaactccgcccatcccgcccctaactccgcccagttccgcccattctccgccccatggctgactaattttttttatttatgcagaggccgaggccgcctctgcctctgagctattccagaagtagtgaggaggcttttttggaggcctaggcttttgcaaaaagctcgattcttctgacactagcgccaccatgatcgaacaagacggcctccatgctggcagtcccgcagcttgggtcgaacgcttgttcgggtacgactgggcccagcagaccatcggatgtagcgatgcggccgtgttccgtctaagcgctcaaggccggcccgtgctgttcgtgaagaccgacctgagcggcgccctgaacgagcttcaagacgaggctgcccgcctgagctggctggccaccaccggcgtaccctgcgccgctgtgttggatgttgtgaccgaagccggccgggactggctgctgctgggcgaggtccctggccaggatctgctgagcagccaccttgcccccgctgagaaggtttctatcatggccgatgcaatgcggcgcctgcacaccctggaccccgctacctgccccttcgaccaccaggctaagcatcggatcgagcgtgctcggacccgcatggaggccggcctggtggaccaggacgacctggacgaggagcatcagggcctggcccccgctgaactgttcgcccgactgaaagcccgcatgccggacggtgaggacctggttgtcacacacggagatgcctgcctccctaacatcatggtcgagaatggccgcttctccggcttcatcgactgcggtcgcctaggagttgccgaccgctaccaggacatcgccctggccacccgcgacatcgctgaggagcttggcggcgagtgggccgaccgcttcttagtcttgtacggcatcgcagctcccgacagccagcgcatcgccttctaccgcttgctcgacgagttcttttaatgatctagaaccggtcatggccgcaataaaatatctttattttcattacatctgtgtgttggttttttgtgtgttcgaactagatgctgtcgaccgatgcccttgagagccttcaacccagtcagctccttccggtgggcgcggggcatgactatcgtcgccgcacttatgactgtcttctttatcatgcaactcgtaggacaggtgccggcagcgctcttccgcttcctcgctcactgactcgctgcgctcggtcgttcggctgcggcgagcggtatcagctcactcaaaggcggtaatacggttatccacagaatcaggggataacgcaggaaagaacatgtgagcaaaaggccagcaaaaggccaggaaccgtaaaaaggccgcgttgctggcgtttttccataggctccgcccccctgacgagcatcacaaaaatcgacgctcaagtcagaggtggcgaaacccgacaggactataaagataccaggcgtttccccctggaagctccctcgtgcgctctcctgttccgaccctgccgcttaccggatacctgtccgcctttctcccttcgggaagcgtggcgctttctcatagctcacgctgtaggtatctcagttcggtgtaggtcgttcgctccaagctgggctgtgtgcacgaaccccccgttcagcccgaccgctgcgccttatccggtaactatcgtcttgagtccaacccggtaagacacgacttatcgccactggcagcagccactggtaacaggattagcagagcgaggtatgtaggcggtgctacagagttcttgaagtggtggcctaactacggctacactagaagaacagtatttggtatctgcgctctgctgaagccagttaccttcggaaaaagagttggtagctcttgatccggcaaacaaaccaccgctggtagcggtggtttttttgtttgcaagcagcagattacgcgcagaaaaaaaggatctcaagaagatcctttgatcttttctacggggtctgacgctcagtggaacgaaaactcacgttaagggattttggtcatgagattatcaaaaaggatcttcacctagatccttttaaattaaaaatgaagttttaaatcaatctaaagtatatatgagtaaacttggtctgacagcggccgcaaatgctaaaccactgcagtggttaccagtgcttgatcagtgaggcaccgatctcagcgatctgcctatttcgttcgtccatagtggcctgactccccgtcgtgtagatcactacgattcgtgagggcttaccatcaggccccagcgcagcaatgatgccgcgagagccgcgttcaccggcccccgatttgtcagcaatgaaccagccagcagggagggccgagcgaagaagtggtcctgctactttgtccgcctccatccagtctatgagctgctgtcgtgatgctagagtaagaagttcgccagtgagtagtttccgaagagttgtggccattgctactggcatcgtggtatcacgctcgtcgttcggtatggcttcgttcaactctggttcccagcggtcaagccgggtcacatgatcacccatattatgaagaaatgcagtcagctccttagggcctccgatcgttgtcagaagtaagttggccgcggtgttgtcgctcatggtaatggcagcactacacaattctcttaccgtcatgccatccgtaagatgcttttccgtgaccggcgagtactcaaccaagtcgttttgtgagtagtgtatacggcgaccaagctgctcttgcccggcgtctatacgggacaacaccgcgccacatagcagtactttgaaagtgctcatcatcgggaatcgttcttcggggcggaaagactcaaggatcttgccgctattgagatccagttcgatatagcccactcttgcacccagttgatcttcagcatcttttactttcaccagcgtttcggggtgtgcaaaaacaggcaagcaaaatgccgcaaagaagggaatgagtgcgacacgaaaatgttggatgctcatactcgtcctttttcaatattattgaagcatttatcagggttactagtacgtctctcaaggataagtaagtaatattaaggtacgggaggtattggacaggccgcaataaaatatctttattttcattacatctgtgtgttggttttttgtgtgaatcgatagtactaacatacgctctccatcaaaacaaaacgaaacaaaacaaactagcaaaataggctgtccccagtgcaagtgcaggtgccagaacatttctct

SEQ ID NO: 25 - DNA, 6528 bp, Artificial Sequence
  Plasmid
ggatccctaccggtgctgcggccgcgcagttaacgccgcccctctccctcccccccccctaacgttactggccgaagccgcttggaataaggccggtgtgcgtttgtctatatgttattttccaccatattgccgtcttttggcaatgtgagggcccggaaacctggccctgtcttcttgacgagcattcctaggggtctttcccctctcgccaaaggaatgcaaggtctgttgaatgtcgtgaaggaagcagttcctctggaagcttcttgaagacaaacaacgtctgtagcgaccctttgcaggcagcggaaccccccacctggcgacaggtgcctctgcggccaaaagccacgtgtataagatacacctgcaaaggcggcacaaccccagtgccacgttgtgagttggatagttgtggaaagagtcaaatggctctcctcaagcgtattcaacaaggggctgaaggatgcccagaaggtaccccattgtatgggatctgatctggggcctcggtacacatgctttacatgtgtttagtcgaggttaaaaaaacgtctaggccccccgaaccacggggacgtggttttcctttgaaaaacacgatgataatatggccacaagatctgccaccatggttcgaccattgaactgcatcgtcgccgtgtcccaaaatatggggattggcaagaacggagacctaccctggcctccgctcaggaacgagttcaagtacttccaaagaatgaccacaacctcttcagtggaaggtaaacagaatctggtgattatgggtaggaaaacctggttctccattcctgagaagaatcgacctttaaaggacagaattaatatagttctcagtagagaactcaaagaaccaccacgaggagctcattttcttgccaaaagtttggatgatgccttaagacttattgaacaaccggaattggcaagtaaagtagacatggtttggatagtcggaggcagttctgtttaccaggaagccatgaatcaaccaggccacctcagactctttgtgacaaggatcatgcaggaatttgaaagtgacacgtttttcccagaaattgatttggggaaatataaacttctcccagaatacccaggcgtcctctctgaggtccaggaggaaaaaggcatcaagtataagtttgaagtctacgagaagaaagactaaaaccggttagtaatgagtttaaacgggggaggctaactgaaacacggaaggagacaataccggaaggaacccgcgctatgacggcaataaaaagacagaataaaacgcacgggtgttgggtcgtttgttcataaacgcggggttcggtcccagggctggcactctgtcgataccccaccgagaccccattggggccaatacgcccgcgtttcttccttttccccaccccaccccccaagttcgggtgaaggcccagggctcgcagccaacgtcggggcggcaggccctgccattaccgtcgacctctagctagagcttggcgtaatcatggtcatagctgtttcctgtgtgaaattgttatccgctcacaattccacacaacatacgagccggaagcataaagtgtaaagcctggggtgcctaatgagtgagctaactcacattaattgcgttgcgctcactgcccgctttccagtcgggaaacctgtcgtgccagctgcattaatgaatcggccaacgcgcggggagaggcggtttgcgtattgggcgctcttccgcttcctcgctcactgactcgctgcgctcggtcgttcggctgcggcgagcggtatcagctcactcaaaggcggtaatacggttatccacagaatcaggggataacgcaggaaagaacatgtgagcaaaaggccagcaaaaggccaggaaccgtaaaaaggccgcgttgctggcgtttttccataggctccgcccccctgacgagcatcacaaaaatcgacgctcaagtcagaggtggcgaaacccgacaggactataaagataccaggcgtttccccctggaagctccctcgtgcgctctcctgttccgaccctgccgcttaccggatacctgtccgcctttctcccttcgggaagcgtggcgctttctcatagctcacgctgtaggtatctcagttcggtgtaggtcgttcgctccaagctgggctgtgtgcacgaaccccccgttcagcccgaccgctgcgccttatccggtaactatcgtcttgagtccaacccggtaagacacgacttatcgccactggcagcagccactggtaacaggattagcagagcgaggtatgtaggcggtgctacagagttcttgaagtggtggcctaactacggctacactagaagaacagtatttggtatctgcgctctgctgaagccagttaccttcggaaaaagagttggtagctcttgatccggcaaacaaaccaccgctggtagcggtttttttgtttgcaagcagcagattacgcgcagaaaaaaaggatctcaagaagatcctttgatcttttctacggggtctgacgctcagtggaacgaaaactcacgttaagggattttggtcatgagattatcaaaaaggatcttcacctagatccttttaaattaaaaatgaagttttaaatcaatctaaagtatatatgagtaaacttggtctgacagttaccaatgcttaatcagtgaggcacctatctcagcgatctgtctatttcgttcatccatagttgcctgactccccgtcgtgtagataactacgatacgggagggcttaccatctggccccagtgctgcaatgataccgcgagacccacgctcaccggctccagatttatcagcaataaaccagccagccggaagggccgagcgcagaagtggtcctgcaactttatccgcctccatccagtctattaattgttgccgggaagctagagtaagtagttcgccagttaatagtttgcgcaacgttgttgccattgctacaggcatcgtggtgtcacgctcgtcgtttggtatggcttcattcagctccggttcccaacgatcaaggcgagttacatgatcccccatgttgtgcaaaaaagcggttagctccttcggtcctccgatcgttgtcagaagtaagttggccgcagtgttatcactcatggttatggcagcactgcataattctcttactgtcatgccatccgtaagatgcttttctgtgactggtgagtactcaaccaagtcattctgagaatagtgtatgcggcgaccgagttgctcttgcccggcgtcaatacgggataataccgcgccacatagcagaactttaaaagtgctcatcattggaaaacgttcttcggggcgaaaactctcaaggatcttaccgctgttgagatccagttcgatgtaacccactcgtgcacccaactgatcttcagcatcttttactttcaccagcgtttctgggtgagcaaaaacaggaaggcaaaatgccgcaaaaaagggaataagggcgacacggaaatgttgaatactcatactcttcctttttcaatattattgaagcatttatcagggttattgtctcatgagcggatacatatttgaatgtatttagaaaaataaacaaataggggttccgcgcacatttccccgaaaagtgccacctgacgtcgacggatcgggagatctggagagggggtaaaaaaatgctgcactgtgcggctaggccggtgagtgagcggcgcggagccaatcagcgctcgccgttccgaaagttgccttttatggctcgagtggccgctgtggcgtcctataaaacccggcggcgcaacgcgcagccactgtcgagtccgcgtccacccgcgagcacaggcctttcgcagctctttcttcgccgctccacacccgccaccaggtaagcagggacaacaggcccagccggccacagccctcccgtgggcagtgaccgcgctgcagggtcgcgggggacactcggcgcggacaccggggaaggctggagggtggtgccgggccgcggagcggacactttcagatccaactttcagtccagggtgtagaccctttacagccgcattgccacggtgtagacaccggtggacccgctctggctcagagcacgcggcttgggggaacccattagggtcgcagtgtgggcgctatgagagccgatgcagctttcgggtgttgaaccgtatctgcccaccttggggggaggacacaaggtcgggagccaaacgccacgatcatgccttggtggcccatgggtctttgtctaaaccggtttgcccatttggcttgccgggcgggcgggcgcggcgggcccggctcggccgggttgggggctgggttgccactgcgcttgcgcgctctatggctgggtattggggcgcgtgcacgctggggagggagcccttcctcttccccctctcccaagttaaacttgcgcgtgcgtattgagacttggagcgcggccaccggggttgggcgagggcggggccgttgtccggaaggggcggggtcgcagcggcttcggggcgcctgctcgcgcttcctgctgggtgtggtcgcctcccgcgcgcgcactagccgcccgccggcggggcgaaggcggggcttgcgcccgtttggggagggggcggaggcctggcttcctgccgtggggccgcctccggaccagcgtttgcctcttatggtaataacgcggccggcctgggcttcctttgtcccctgagtttgggcgcgcgccccctggcggcccgaggccgcggcttgccggaagtgggcagggcggcagcggctgcgcctagtggcccgccagtgaccgcgaccctcttttgtgccctgatatagttcgccgaattcgctagcagaacaggatgttctgatcaaagagatccaaagtcagaacacgttgttctagctaaaataacacattcagagaacatgctgttctgatcaaagagatccaaagtcagaacaaggtgttctagctaaaataacacattcagagaacatgatgttctgatcaaagagatccaaagtcgcggccgcgttgacattgattattgactagttattaatagtaatcaattacggggtcattagttcatagcccatatatggagttccgcgttacataacttacggtaaatggcccgcctggctgaccgcccaacgacccccgcccattgacgtcaataatgacgtatgttcccatagtaacgccaatagggactttccattgacgtcaatgggtggagtatttacggtaaactgcccacttggcagtacatcaagtgtatcatatgccaagtacgccccctattgacgtcaatgacggtaaatggcccgcctggcattatgcccagtacatgaccttatgggactttcctacttggcagtacatctacgtattagtcatcgctattaccatggtgatgcggttttggcagtacatcaatgggcgtggatagcggtttgactcacggggatttccaagtctccaccccattgacgtcaatgggagtttgttttggcaccaaaatcaacgggactttccaaaatgtcgtaacaactccgccccattgacgcaaatgggcggtaggcgtgtacggtgggaggtctatataagcagagctctctggctaactagagaacccactgcttactggcttatcgaaagcttctctggctaactagagaacccactgcttactggcttatcgaaattaatacgactcactatagggagacccaagctggctagcaagatggattcacaggcccaggttcttatattgctgctgctatgggtatctggtacctgtggggacattgtgatgtcacagtctccatcctccctggctgtgtcagcaggagagaaggtcactatgagctgcaaatccagtcagagtctgctcaacagtagaacccgaaagaactacttggcttggtaccagcagaaaccagggcagtctcctaaactgctgatctactgggcatccattagggaatctggggtccctgatcgcttcacaggcagtggatctgggacagatttcactctcaccatcagcagtgtgcaggctgaagacctggcagtttattactgcaagcaatcttataatctgtggacgttcggtggaggcaccaagctggaaatcaaacggactgttgcggcaccatctgtcttcatcttcccgccatctgatgagcagttgaaatctggaactgcctctgttgtgtgcctgctgaataacttctatcccagagaggccaaagtacagtggaaggtggataacgccctccaatcgggtaactcccaggagagtgtcacagagcaggacagcaaggacagcacctacagcctcagcagcaccctgacgctgagcaaagcagactacgagaaacacaaagtctacgcctgcgaagtcacccatcagggcctgagctcgcccgtcacaaagagcttcaacaggggagagtgttgaggatcc

SEQ ID NO: 26 - DNA, 564 bp, Artificial Sequence
  dhfr sequence
atggttcgaccattgaactgcatcgtcgccgtgtcccaaaatatggggattggcaagaacggagacctaccctggcctccgctcaggaacgagttcaagtacttccaaagaatgaccacaacctcttcagtggaaggtaaacagaatctggtgattatgggtaggaaaacctggttctccattcctgagaagaatcgacctttaaaggacagaattaatatagttctcagtagagaactcaaagaaccaccacgaggagctcattttcttgccaaaagtttggatgatgccttaagacttattgaacaaccggaattggcaagtaaagtagacatggtttggatagtcggaggcagttctgtttaccaggaagccatgaatcaaccaggccacctcagactctttgtgacaaggatcatgcaggaatttgaaagtgacacgtttttcccagaaattgatttggggaaatataaacttctcccagaatacccaggcgtcctctctgaggtccaggaggaaaaaggcatcaagtataagtttgaagtctacgagaagaaagactaa

SEQ ID NO: 27 - DNA, 31 bp, Artificial Sequence
  Oligonucleotide
aaaaagatctggagagggggtaaaaaaatga

SEQ ID NO: 28 - DNA, 45 bp, Artificial Sequence
  Oligonucleotide
tcaacgcggccgcaaaaaagaattcggcgaactatatcagggcac

SEQ ID NO: 29 - DNA, 534 bp, Artificial Sequence
  Enhancer promoter
gttgacattgattattgactagttattaatagtaatcaattacggggtcattagttcatagcccatatatggagttccgcgttacataacttacggtaaatggcccgcctggctgaccgcccaacgacccccgcccattgacgtcaataatgacgtatgttcccatagtaacgccaatagggactttccattgacgtcaatgggtggagtatttacggtaaactgcccacttggcagtacatcaagtgtatcatatgccaagtacgccccctattgacgtcaatgacggtaaatggcccgcctggcattatgcccagtacatgaccttatgggactttcctacttggcagtacatctacgtattagtcatcgctattaccatggtgatgcggttttggcagtacatcaatgggcgtggatagcggtttgactcacggggatttccaagtctccaccccattgacgtcaatgggagtttgttttggcaccaaaatcaacgggactttccaaaatgtcgtaacaactccgccccat

SEQ ID NO: 30 - DNA, 89 bp, Artificial Sequence
  Core CMV
gcaaatgggcggtaggcgtgtacggtgggaggtctatataagcagagctctctggctaactagagaacccactgcttactggcttatca

SEQ ID NO: 31 - protein, 239 aa, Artificial Sequence
  LAb1
MDSQAQVLILLLLWVSGTCGDIVMSQSPSSLAVSAGEKVTMSCKSSQSLLNSRTRKNYLAWYQQKPGQSPKLLIYWASIRESGVPDRFTGSGSGTDFTLTISSVQAEDLAVYYCKQSYNLWTFGGGTKLEIKRTVAAPSVFIFPPSDEQLKSGTASVVCLLNNFYPREAKVQWKVDNALQSGNSQESVTEQDSKDSTYSLSSTLTLSKADYEKHKVYACEVTHQGLSSPVTKSFNRGEC

SEQ ID NO: 32 - protein, 470 aa, Artificial Sequence
  HAb1
MGWSLILLFLVAVATRVLSQVQLQQPGAELVKPGASVKMSCKASGYTFTSYNMHWVKQTPGRGLEWIGAIYPGNGDTSYNQKFKGKATLTADKSSSTAYMQLSSLTSEDSAVYYCARSTYYGGDWYFNVWGAGTTVTVSAASTKGPSVFPLAPSSKSTSGGTAALGCLVKDYFPEPVTVSWNSGALTSGVHTFPAVLQSSGLYSLSSVVTVPSSSLGTQTYICNVNHKPSNTKVDKKVEPKSCDKTHTCPPCPAPELLGGPSVFLFPPKPKDTLMISRTPEVTCVVVDVSHEDPEVKFNWYVDGVEVHNAKTKPREEQYNSTYRVVSVLTVLHQDWLNGKEYKCKVSNKALPAPIEKTISKAKGQPREPQVYTLPPSRDELTKNQVSLTCLVKGFYPSDIAVEWESNGQPENNYKTTPPVLDSDGSFFLYSKLTVDKSRWQQGNVFSCSVMHEALHNHYTQKSLSLSPGK

SEQ ID NO: 33 - protein, 239 aa, Artificial Sequence; identical to SEQ ID NO: 31
  LAb2

SEQ ID NO: 34 - protein, 471 aa, Artificial Sequence [sequence omitted]

SEQ ID NO: 35 - DNA, 6774 bp, Artificial Sequence
  Seq4-Luc
ggcctaactggccggtacctgagctcgctagcggagagggggtaaaaaaatgctgcactgtgcggctaggccggtgagtgagcggcgcggagccaatcagcgctcgccgttccgaaagttgccttttatggctcgagtggccgctgtggcgtcctataaaacccggcggcgcaacgcgcagccactgtcgagtccgcgtccacccgcgagcacaggcctttcgcagctctttcttcgccgctccacacccgccaccaggtaagcagggacaacaggcccagccggccacagccctcccgtgggcagtgaccgcgctgcagggtcgcgggggacactcggcgcggacaccggggaaggctggagggtggtgccgggccgcggagcggacactttcagatccaactttcagtccagggtgtagaccctttacagccgcattgccacggtgtagacaccggtggacccgctctggctcagagcacgcggcttgggggaacccattagggtcgcagtgtgggcgctatgagagccgatgcagctttcgggtgttgaaccgtatctgcccaccttggggggaggacacaaggtcgggagccaaacgccacgatcatgccttggtggcccatgggtctttgtctaaaccggtttgcccatttggcttgccgggcgggcgggcgcggcgggcccggctcggccgggttgggggctgggttgccactgcgcttgcgcgctctatggctgggtattggggcgcgtgcacgctggggagggagcccttcctcttccccctctcccaagttaaacttgcgcgtgcgtattgagacttggagcgcggccaccggggttgggcgagggcggggccgttgtccggaaggggcggggtcgcagcggcttcggggcgcctgctcgcgcttcctgctgggtgtggtcgcctcccgcgcgcgcactagccgcccgccggcggggcgaaggcggggcttgcgcccgtttggggagggggcggaggcctggcttcctgccgtggggccgcctccggaccagcgtttgcctcttatggtaataacgcggccggcctgggcttcctttgtcccctgagtttgggcgcgcgccccctggcggcccgaggccgcggcttgccggaagtgggcagggcggcagcggctgcgcctagtggcccgccagtgaccgcgaccctcttttgtgccctgatatagttcgccagatctggcctcggcggccaagcttggcaatccggtactgttggtaaagccaccatggaagatgccaaaaacattaagaagggcccagcgccattctacccactcgaagacgggaccgccggcgagcagctgcacaaagccatgaagcgctacgccctggtgcccggcaccatcgcctttaccgacgcacatatcgaggtggacattacctacgccgagtacttcgagatgagcgttcggctggcagaagctatgaagcgctatgggctgaatacaaaccatcggatcgtggtgtgcagcgagaatagcttgcagttcttcatgcccgtgttgggtgccctgttcatcggtgtggctgtggccccagctaacgacatctacaacgagcgcgagctgctgaacagcatgggcatcagccagcccaccgtcgtattcgtgagcaagaaagggctgcaaaagatcctcaacgtgcaaaagaagctaccgatcatacaaaagatcatcatcatggatagcaagaccgactaccagggcttccaaagcatgtacaccttcgtgacttcccatttgccacccggcttcaacgagtacgacttcgtgcccgagagcttcgaccgggacaaaaccatcgccctgatcatgaacagtagtggcagtaccggattgcccaagggcgtagccctaccgcaccgcaccgcttgtgtccgattcagtcatgcccgcgaccccatcttcggcaaccagatcatccccgacaccgctatcctcagcgtggtgccatttcaccacggcttcggcatgttcaccacgctgggctacttgatctgcggctttcgggtcgtgctcatgtaccgcttcgaggaggagctattcttgcgcagcttgcaagactataagattcaatctgccctgctggtgcccacactatttagcttcttcgctaagagcactctcatcgacaagtacgacctaagcaacttgcacgagatcgccagcggcggggcgccgctcagcaaggaggtaggtgaggccgtggccaaacgcttccacctaccaggcatccgccagggctacggcctgacagaaacaaccagcgccattctgatcacccccgaaggggacgacaagcctggcgcagtaggcaaggtggtgcccttcttcgaggctaaggtggtggacttggacaccggtaagacactgggtgtgaaccagcgcggcgagctgtgcgtccgtggccccatgatcatgagcggctacgttaacaaccccgaggctacaaacgctctcatcgacaaggacggctggctgcacagcggcgacatcgcctactgggacgaggacgagcacttcttcatcgtggaccggctgaagagcctgatcaaatacaagggctaccaggtagccccagccgaactggagagcatcctgctgcaacaccccaacatcttcgacgccggggtcgccggcctgcccgacgacgatgccggcgagctgcccgccgcagtcgtcgtgctggaacacggtaaaaccatgaccgagaaggagatcgtggactatgtggccagccaggttacaaccgccaagaagctgcgcggtggtgttgtgttcgtggacgaggtgcctaaaggactgaccggcaagttggacgcccgcaagatccgcgagattctcattaaggccaagaagggcggcaagatcgccgtgtaataattctagagtcggggcggccggccgcttcgagcagacatgataagatacattgatgagtttggacaaaccacaactagaatgcagtgaaaaaaatgctttatttgtgaaatttgtgatgctattgctttatttgtaaccattataagctgcaataaacaagttaacaacaacaattgcattcattttatgtttcaggttcagggggaggtgtgggaggttttttaaagcaagtaaaacctctacaaatgtggtaaaatcgataaggatccgtttgcgtattgggcgctcttccgctgatctgcgcagcaccatggcctgaaataacctctgaaagaggaacttggttagctaccttctgaggcggaaagaaccagctgtggaatgtgtgtcagttagggtgtggaaagtccccaggctccccagcaggcagaagtatgcaaagcatgcatctcaattagtcagcaaccaggtgtggaaagtccccaggctccccagcaggcagaagtatgcaaagcatgcatctcaattagtcagcaaccatagtcccgcccctaactccgcccatcccgcccctaactccgcccagttccgcccattctccgccccatggctgactaattttttttatttatgcagaggccgaggccgcctctgcctctgagctattccagaagtagtgaggaggcttttttggaggcctaggcttttgcaaaaagctcgattcttctgacactagcgccaccatgatcgaacaagacggcctccatgctggcagtcccgcagcttgggtcgaacgcttgttcgggtacgactgggcccagcagaccatcggatgtagcgatgcggccgtgttccgtctaagcgctcaaggccggcccgtgctgttcgtgaagaccgacctgagcggcgccctgaacgagcttcaagacgaggctgcccgcctgagctggctggccaccaccggcgtaccctgcgccgctgtgttggatgttgtgaccgaagccggccgggactggctgctgctgggcgaggtccctggccaggatctgctgagcagccaccttgcccccgctgagaaggtttctatcatggccgatgcaatgcggcgcctgcacaccctggaccccgctacctgccccttcgaccaccaggctaagcatcggatcgagcgtgctcggacccgcatggaggccggcctggtggaccaggacgacctggacgaggagcatcagggcctggcccccgctgaactgttcgcccgactgaaagcccgcatgccggacggtgaggacctggttgtcacacacggagatgcctgcctccctaacatcatggtcgagaatggccgcttctccggcttcatcgactgcggtcgcctaggagttgccgaccgctaccaggacatcgccctggccacccgcgacatcgctgaggagcttggcggcgagtgggccgaccgcttcttagtcttgtacggcatcgcagctcccgacagccagcgcatcgccttctaccgcttgctcgacgagttcttttaatgatctagaaccggtcatggccgcaataaaatatctttattttcattacatctgtgtgttggttttttgtgtgttcgaactagatgctgtcgaccgatgcccttgagagccttcaacccagtcagctccttccggtgggcgcggggcatgactatcgtcgccgcacttatgactgtcttctttatcatgcaactcgtaggacaggtgccggcagcgctcttccgcttcctcgctcactgactcgctgcgctcggtcgttcggctgcggcgagcggtatcagctcactcaaaggcggtaatacggttatccacagaatcaggggataacgcaggaaagaacatgtgagcaaaaggccagcaaaaggccaggaaccgtaaaaaggccgcgttgctggcgtttttccataggctccgcccccctgacgagcatcacaaaaatcgacgctcaagtcagaggtggcgaaacccgacaggactataaagataccaggcgtttccccctggaagctccctcgtgcgctctcctgttccgaccctgccgcttaccggatacctgtccgcctttctcccttcgggaagcgtggcgctttctcatagctcacgctgtaggtatctcagttcggtgtaggtcgttcgctccaagctgggctgtgtgcacgaaccccccgttcagcccgaccgctgcgccttatccggtaactatcgtcttgagtccaacccggtaagacacgacttatcgccactggcagcagccactggtaacaggattagcagagcgaggtatgtaggcggtgctacagagttcttgaagtggtggcctaactacggctacactagaagaacagtatttggtatctgcgctctgctgaagccagttaccttcggaaaaagagttggtagctcttgatccggcaaacaaaccaccgctggtagcggtggtttttttgtttgcaagcagcagattacgcgcagaaaaaaaggatctcaagaagatcctttgatcttttctacggggtctgacgctcagtggaacgaaaactcacgttaagggattttggtcatgagattatcaaaaaggatcttcacctagatccttttaaattaaaaatgaagttttaaatcaatctaaagtatatatgagtaaacttggtctgacagcggccgcaaatgctaaaccactgcagtggttaccagtgcttgatcagtgaggcaccgatctcagcgatctgcctatttcgttcgtccatagtggcctgactccccgtcgtgtagatcactacgattcgtgagggcttaccatcaggccccagcgcagcaatgatgccgcgagagccgcgttcaccggcccccgatttgtcagcaatgaaccagccagcagggagggccgagcgaagaagtggtcctgctactttgtccgcctccatccagtctatgagctgctgtcgtgatgctagagtaagaagttcgccagtgagtagtttccgaagagttgtggccattgctactggcatcgtggtatcacgctcgtcgttcggtatggcttcgttcaactctggttcccagcggtcaagccgggtcacatgatcacccatattatgaagaaatgcagtcagctccttagggcctccgatcgttgtcagaagtaagttggccgcggtgttgtcgctcatggtaatggcagcactacacaattctcttaccgtcatgccatccgtaagatgcttttccgtgaccggcgagtactcaaccaagtcgttttgtgagtagtgtatacggcgaccaagctgctcttgcccggcgtctatacgggacaacaccgcgccacatagcagtactttgaaagtgctcatcatcgggaatcgttcttcggggcggaaagactcaaggatcttgccgctattgagatccagttcgatatagcccactcttgcacccagttgatcttcagcatcttttactttcaccagcgtttcggggtgtgcaaaaacaggcaagcaaaatgccgcaaagaagggaatgagtgcgacacgaaaatgttggatgctcatactcgtcctttttcaatattattgaagcatttatcagggttactagtacgtctctcaaggataagtaagtaatattaaggtacgggaggtattggacaggccgcaataaaatatctttattttcattacatctgtgtgttggttttttgtgtgaatcgatagtactaacatacgctctccatcaaaacaaaacgaaacaaaacaaactagcaaaataggctgtccccagtgcaagtgcaggtgccagaacatttctct

SEQ ID NO: 36 - DNA, 5675 bp, Artificial Sequence
  Plasmid Seq5-Luc
ggcctaactggccggtacctgagctcgctagcctcgaggatatcaagatctgcaaatgggcggtaggcgtgtacggtgggaggtctatataagcagagctctctggctaactagagaacccactgcttactggcttatcaaagcttggcaatccggtactgttggtaaagccaccatggaagatgccaaaaacattaagaagggcccagcgccattctacccactcgaagacgggaccgccggcgagcagctgcacaaagccatgaagcgctacgccctggtgcccggcaccatcgcctttaccgacgcacatatcgaggtggacattacctacgccgagtacttcgagatgagcgttcggctggcagaagctatgaagcgctatgggctgaatacaaaccatcggatcgtggtgtgcagcgagaatagcttgcagttcttcatgcccgtgttgggtgccctgttcatcggtgtggctgtggccccagctaacgacatctacaacgagcgcgagctgctgaacagcatgggcatcagccagcccaccgtcgtattcgtgagcaagaaagggctgcaaaagatcctcaacgtgcaaaagaagctaccgatcatacaaaagatcatcatcatggatagcaagaccgactaccagggcttccaaagcatgtacaccttcgtgacttcccatttgccacccggcttcaacgagtacgacttcgtgcccgagagcttcgaccgggacaaaaccatcgccctgatcatgaacagtagtggcagtaccggattgcccaagggcgtagccctaccgcaccgcaccgcttgtgtccgattcagtcatgcccgcgaccccatcttcggcaaccagatcatccccgacaccgctatcctcagcgtggtgccatttcaccacggcttcggcatgttcaccacgctgggctacttgatctgcggctttcgggtcgtgctcatgtaccgcttcgaggaggagctattcttgcgcagcttgcaagactataagattcaatctgccctgctggtgcccacactatttagcttcttcgctaagagcactctcatcgacaagtacgacctaagcaacttgcacgagatcgccagcggcggggcgccgctcagcaaggaggtaggtgaggccgtggccaaacgcttccacctaccaggcatccgccagggctacggcctgacagaaacaaccagcgccattctgatcacccccgaaggggacgacaagcctggcgcagtaggcaaggtggtgcccttcttcgaggctaaggtggtggacttggacaccggtaagacactgggtgtgaaccagcgcggcgagctgtgcgtccgtggccccatgatcatgagcggctacgttaacaaccccgaggctacaaacgctctcatcgacaaggacggctggctgcacagcggcgacatcgcctactgggacgaggacgagcacttcttcatcgtggaccggctgaagagcctgatcaaatacaagggctaccaggtagccccagccgaactggagagcatcctgctgcaacaccccaacatcttcgacgccggggtcgccggcctgcccgacgacgatgccggcgagctgcccgccgcagtcgtcgtgctggaacacggtaaaaccatgaccgagaaggagatcgtggactatgtggccagccaggttacaaccgccaagaagctgcgcggtggtgttgtgttcgtggacgaggtgcctaaaggactgaccggcaagttggacgcccgcaagatccgcgagattctcattaaggccaagaagggcggcaagatcgccgtgtaataattctagagtcggggcggccggccgcttcgagcagacatgataagatacattgatgagtttggacaaaccacaactagaatgcagtgaaaaaaatgctttatttgtgaaatttgtgatgctattgctttatttgtaaccattataagctgcaataaacaagttaacaacaacaattgcattcattttatgtttcaggttcagggggaggtgtgggaggttttttaaagcaagtaaaacctctacaaatgtggtaaaatcgataaggatccgtttgcgtattgggcgctcttccgctgatctgcgcagcaccatggcctgaaataacctctgaaagaggaacttggttagctaccttctgaggcggaaagaaccagctgtggaatgtgtgtcagttagggtgtggaaagtccccaggctccccagcaggcagaagtatgcaaagcatgcatctcaattagtcagcaaccaggtgtggaaagtccccaggctccccagcaggcagaagtatgcaaagcatgcatctcaattagtcagcaaccatagtcccgcccctaactccgcccatcccgcccctaactccgcccagttccgcccattctccgccccatggctgactaattttttttatttatgcagaggccgaggccgcctctgcctctgagctattccagaagtagtgaggaggcttttttggaggcctaggcttttgcaaaaagctcgattcttctgacactagcgccaccatgatcgaacaagacggcctccatgctggcagtcccgcagcttgggtcgaacgcttgttcgggtacgactgggcccagcagaccatcggatgtagcgatgcggccgtgttccgtctaagcgctcaaggccggcccgtgctgttcgtgaagaccgacctgagcggcgccctgaacgagcttcaagacgaggctgcccgcctgagctggctggccaccaccggcgtaccctgcgccgctgtgttggatgttgtgaccgaagccggccgggactggctgctgctgggcgaggtccctggccaggatctgctgagcagccaccttgcccccgctgagaaggtttctatcatggccgatgcaatgcggcgcctgcacaccctggaccccgctacctgccccttcgaccaccaggctaagcatcggatcgagcgtgctcggacccgcatggaggccggcctggtggaccaggacgacctggacgaggagcatcagggcctggcccccgctgaactgttcgcccgactgaaagcccgcatgccggacggtgaggacctggttgtcacacacggagatgcctgcctccctaacatcatggtcgagaatggccgcttctccggcttcatcgactgcggtcgcctaggagttgccgaccgctaccaggacatcgccctggccacccgcgacatcgctgaggagcttggcggcgagtgggccgaccgcttcttagtcttgtacggcatcgcagctcccgacagccagcgcatcgccttctaccgcttgctcgacgagttcttttaatgatctagaaccggtcatggccgcaataaaatatctttattttcattacatctgtgtgttggttttttgtgtgttcgaactagatgctgtcgaccgatgcccttgagagccttcaacccagtcagctccttccggtgggcgcggggcatgactatcgtcgccgcacttatgactgtcttctttatcatgcaactcgtaggacaggtgccggcagcgctcttccgcttcctcgctcactgactcgctgcgctcggtcgttcggctgcggcgagcggtatcagctcactcaaaggcggtaatacggttatccacagaatcaggggataacgcaggaaagaacatgtgagcaaaaggccagcaaaaggccaggaaccgtaaaaaggccgcgttgctggcgtttttccataggctccgcccccctgacgagcatcacaaaaatcgacgctcaagtcagaggtggcgaaacccgacaggactataaagataccaggcgtttccccctggaagctccctcgtgcgctctcctgttccgaccctgccgcttaccggatacctgtccgcctttctcccttcgggaagcgtggcgctttctcatagctcacgctgtaggtatctcagttcggtgtaggtcgttcgctccaagctgggctgtgtgcacgaaccccccgttcagcccgaccgctgcgccttatccggtaactatcgtcttgagtccaacccggtaagacacgacttatcgccactggcagcagccactggtaacaggattagcagagcgaggtatgtaggcggtgctacagagttcttgaagtggtggcctaactacggctacactagaagaacagtatttggtatctgcgctctgctgaagccagttaccttcggaaaaagagttggtagctcttgatccggcaaacaaaccaccgctggtagcggtggtttttttgtttgcaagcagcagattacgcgcagaaaaaaaggatctcaagaagatcctttgatcttttctacggggtctgacgctcagtggaacgaaaactcacgttaagggattttggtcatgagattatcaaaaaggatcttcacctagatccttttaaattaaaaatgaagttttaaatcaatctaaagtatatatgagtaaacttggtctgacagcggccgcaaatgctaaaccactgcagtggttaccagtgcttgatcagtgaggcaccgatctcagcgatctgcctatttcgttcgtccatagtggcctgactccccgtcgtgtagatcactacgattcgtgagggcttaccatcaggccccagcgcagcaatgatgccgcgagagccgcgttcaccggcccccgatttgtcagcaatgaaccagccagcagggagggccgagcgaagaagtggtcctgctactttgtccgcctccatccagtctatgagctgctgtcgtgatgctagagtaagaagttcgccagtgagtagtttccgaagagttgtggccattgctactggcatcgtggtatcacgctcgtcgttcggtatggcttcgttcaactctggttcccagcggtcaagccgggtcacatgatcacccatattatgaagaaatgcagtcagctccttagggcctccgatcgttgtcagaagtaagttggccgcggtgttgtcgctcatggtaatggcagcactacacaattctcttaccgtcatgccatccgtaagatgcttttccgtgaccggcgagtactcaaccaagtcgttttgtgagtagtgtatacggcgaccaagctgctcttgcccggcgtctatacgggacaacaccgcgccacatagcagtactttgaaagtgctcatcatcgggaatcgttcttcggggcggaaagactcaaggatcttgccgctattgagatccagttcgatatagcccactcttgcacccagttgatcttcagcatcttttactttcaccagcgtttcggggtgtgcaaaaacaggcaagcaaaatgccgcaaagaagggaatgagtgcgacacgaaaatgttggatgctcatactcgtcctttttcaatattattgaagcatttatcagggttactagtacgtctctcaaggataagtaagtaatattaaggtacgggaggtattggacaggccgcaataaaatatctttattttcattacatctgtgtgttggttttttgtgtgaatcgatagtactaacatacgctctccatcaaaacaaaacgaaacaaaacaaactagcaaaataggctgtccccagtgcaagtgcaggtgccagaacatttctct

SEQ ID NO: 37 - DNA, 52 bp, Artificial Sequence
  Oligonucleotide PARIC1fw
agcttgacgtaaacgcgttcgcgaccatatgtgatcaggaattctccggaag

SEQ ID NO: 38 - DNA, 52 bp, Artificial Sequence
  Oligonucleotide PARIC1rv
gatccttccggagaattcctgatcacatatggtcgcgaacgcgtttacgtca

SEQ ID NO: 39 - DNA, 32 bp, Artificial Sequence
  Oligonucleotide PoA-Fw
ttttttgaattcgtgtaataattctagagtcg

SEQ ID NO: 40 - DNA, 22 bp, Artificial Sequence
  Oligonucleotide PoA-Rv
ccaatacgcaaacggatcctta

SEQ ID NO: 41 - DNA, 6325 bp, Artificial Sequence
  Plasmid Seq3a-IC
gttggttttttgtgtgaatcgatagtactaacatacgctctccatcaaaacaaaacgaaacaaaacaaactagcaaaataggctgtccccagtgcaagtgcaggtgccagaacatttctctggcctaactggccggtaccggagagggggtaaaaaaatgctgcactgtgcggctaggccggtgagtgagcggcgcggagccaatcagcgctcgccgttccgaaagttgccttttatggctcgagtggccgctgtggcgtcctataaaacccggcggcgcaacgcgcagccactgtcgagtccgcgtccacccgcgagcacaggcctttcgcagctctttcttcgccgctccacacccgccaccaggtaagcagggacaacaggcccagccggccacagccctcccgtgggcagtgaccgcgctgcagggtcgcgggggacactcggcgcggacaccggggaaggctggagggtggtgccgggccgcggagcggacactttcagatccaactttcagtccagggtgtagaccctttacagccgcattgccacggtgtagacaccggtggacccgctctggctcagagcacgcggcttgggggaacccattagggtcgcagtgtgggcgctatgagagccgatgcagctttcgggtgttgaaccgtatctgcccaccttggggggaggacacaaggtcgggagccaaacgccacgatcatgccttggtggcccatgggtctttgtctaaaccggtttgcccatttggcttgccgggcgggcgggcgcggcgggcccggctcggccgggttgggggctgggttgccactgcgcttgcgcgctctatggctgggtattggggcgcgtgcacgctggggagggagcccttcctcttccccctctcccaagttaaacttgcgcgtgcgtattgagacttggagcgcggccaccggggttgggcgagggcggggccgttgtccggaaggggcggggtcgcagcggcttcggggcgcctgctcgcgcttcctgctgggtgtggtcgcctcccgcgcgcgcactagccgcccgccggcggggcgaaggcggggcttgcgcccgtttggggagggggcggaggcctggcttcctgccgtggggccgcctccggaccagcgtttgcctcttatggtaataacgcggccggcctgggcttcctttgtcccctgagtttgggcgcgcgccccctggcggcccgaggccgcggcttgccggaagtgggcagggcggcagcggctgcgcctagtggcccgccagtgaccgcgaccctcttttgtgccctgatatagttcgccgaattcgctagcagaacaggatgttctgatcaaagagatccaaagtcagaacacgttgttctagctaaaataacacattcagagaacatgctgttctgatcaaagagatccaaagtcagaacaaggtgttctagctaaaataacacattcagagaacatgatgttctgatcaaagagatccaaagtcgcggccgcgttgacattgattattgactagttattaatagtaatcaattacggggtcattagttcatagcccatatatggagttccgcgttacataacttacggtaaatggcccgcctggctgaccgcccaacgacccccgcccattgacgtcaataatgacgtatgttcccatagtaacgccaatagggactttccattgacgtcaatgggtggagtatttacggtaaactgcccacttggcagtacatcaagtgtatcatatgccaagtacgccccctattgacgtcaatgacggtaaatggcccgcctggcattatgcccagtacatgaccttatgggactttcctacttggcagtacatctacgtattagtcatcgctattaccatggtgatgcggttttggcagtacatcaatgggcgtggatagcggtttgactcacggggatttccaagtctccaccccattgacgtcaatgggagtttgttttggcaccaaaatcaacgggactttccaaaatgtcgtaacaactccgccccattgacgcaaatgggcggtaggcgtgtacggtgggaggtctatataagcagagctctctggctaactagagaacccactgcttactggcttatcgaaagcttgacgtaaacgcgttcgcgaccatatgtgatcaggaattcgtgtaataattctagagtcggggcggccggccgcttcgagcagacatgataagatacattgatgagtttggacaaaccacaactagaatgcagtgaaaaaaatgctttatttgtgaaatttgtgatgctattgctttatttgtaaccattataagctgcaataaacaagttaacaacaacaattgcattcattttatgtttcaggttcagggggaggtgtgggaggttttttaaagcaagtaaaacctctacaaatgtggtaaaatcgataaggatccgtttgcgtattgggcgctcttccgctgatctgcgtaataattctagagtcggggcggccggccgcttcgagcagacatgataagatacattgatgagtttggacaaaccacaactagaatgcagtgaaaaaaatgctttatttgtgaaatttgtgatgctattgctttatttgtaaccattataagctgcaataaacaagttaacaacaacaattgcattcattttatgtttcaggttcagggggaggtgtgggaggttttttaaagcaagtaaaacctctacaaatgtggtaaaatcgataaggatccgcagcaccatggcctgaaataacctctgaaagaggaacttggttagctaccttctgaggcggaaagaaccagctgtggaatgtgtgtcagttagggtgtggaaagtccccaggctccccagcaggcagaagtatgcaaagcatgcatctcaattagtcagcaaccaggtgtggaaagtccccaggctccccagcaggcagaagtatgcaaagcatgcatctcaattagtcagcaaccatagtcccgcccctaactccgcccatcccgcccctaactccgcccagttccgcccattctccgccccatggctgactaattttttttatttatgcagaggccgaggccgcctctgcctctgagctattccagaagtagtgaggaggcttttttggaggcctaggcttttgcaaaaagctcgattcttctgacactagcgccaccatgatcgaacaagacggcctccatgctggcagtcccgcagcttgggtcgaacgcttgttcgggtacgactgggcccagcagaccatcggatgtagcgatgcggccgtgttccgtctaagcgctcaaggccggcccgtgctgttcgtgaagaccgacctgagcggcgccctgaacgagcttcaagacgaggctgcccgcctgagctggctggccaccaccggcgtaccctgcgccgctgtgttggatgttgtgaccgaagccggccgggactggctgctgctgggcgaggtccctggccaggatctgctgagcagccaccttgcccccgctgagaaggtttctatcatggccgatgcaatgcggcgcctgcacaccctggaccccgctacctgccccttcgaccaccaggctaagcatcggatcgagcgtgctcggacccgcatggaggccggcctggtggaccaggacgacctggacgaggagcatcagggcctggcccccgctgaactgttcgcccgactgaaagcccgcatgccggacggtgaggacctggttgtcacacacggagatgcctgcctccctaacatcatggtcgagaatggccgcttctccggcttcatcgactgcggtcgcctaggagttgccgaccgctaccaggacatcgccctggccacccgcgacatcgctgaggagcttggcggcgagtgggccgaccgcttcttagtcttgtacggcatcgcagctcccgacagccagcgcatcgccttctaccgcttgctcgacgagttcttttaatgatctagaaccggtcatggccgcaataaaatatctttattttcattacatctgtgtgttggttttttgtgtgttcgaactagatgctgtcgaccgatgcccttgagagccttcaacccagtcagctccttccggtgggcgcggggcatgactatcgtcgccgcacttatgactgtcttctttatcatgcaactcgtaggacaggtgccggcagcgctcttccgcttcctcgctcactgactcgctgcgctcggtcgttcggctgcggcgagcggtatcagctcactcaaaggcggtaatacggttatccacagaatcaggggataacgcaggaaagaacatgtgagcaaaaggccagcaaaaggccaggaaccgtaaaaaggccgcgttgctggcgtttttccataggctccgcccccctgacgagcatcacaaaaatcgacgctcaagtcagaggtggcgaaacccgacaggactataaagataccaggcgtttccccctggaagctccctcgtgcgctctcctgttccgaccctgccgcttaccggatacctgtccgcctttctcccttcgggaagcgtggcgctttctcatagctcacgctgtaggtatctcagttcggtgtaggtcgttcgctccaagctgggctgtgtgcacgaaccccccgttcagcccgaccgctgcgccttatccggtaactatcgtcttgagtccaacccggtaagacacgacttatcgccactggcagcagccactggtaacaggattagcagagcgaggtatgtaggcggtgctacagagttcttgaagtggtggcctaactacggctacactagaagaacagtatttggtatctgcgctctgctgaagccagttaccttcggaaaaagagttggtagctcttgatccggcaaacaaaccaccgctggtagcggtggtttttttgtttgcaagcagcagattacgcgcagaaaaaaaggatctcaagaagatcctttgatcttttctacggggtctgacgctcagtggaacgaaaactcacgttaagggattttggtcatgagattatcaaaaaggatcttcacctagatccttttaaattaaaaatgaagttttaaatcaatctaaagtatatatgagtaaacttggtctgacagcggccgcaaatgctaaaccactgcagtggttaccagtgcttgatcagtgaggcaccgatctcagcgatctgcctatttcgttcgtccatagtggcctgactccccgtcgtgtagatcactacgattcgtgagggcttaccatcaggccccagcgcagcaatgatgccgcgagagccgcgttcaccggcccccgatttgtcagcaatgaaccagccagcagggagggccgagcgaagaagtggtcctgctactttgtccgcctccatccagtctatgagctgctgtcgtgatgctagagtaagaagttcgccagtgagtagtttccgaagagttgtggccattgctactggcatcgtggtatcacgctcgtcgttcggtatggcttcgttcaactctggttcccagcggtcaagccgggtcacatgatcacccatattatgaagaaatgcagtcagctccttagggcctccgatcgttgtcagaagtaagttggccgcggtgttgtcgctcatggtaatggcagcactacacaattctcttaccgtcatgccatccgtaagatgcttttccgtgaccggcgagtactcaaccaagtcgttttgtgagtagtgtatacggcgaccaagctgctcttgcccggcgtctatacgggacaacaccgcgccacatagcagtactttgaaagtgctcatcatcgggaatcgttcttcggggcggaaagactcaaggatcttgccgctattgagatccagttcgatatagcccactcttgcacccagttgatcttcagcatcttttactttcaccagcgtttcggggtgtgcaaaaacaggcaagcaaaatgccgcaaagaagggaatgagtgcgacacgaaaatgttggatgctcatactcgtcctttttcaatattattgaagcatttatcagggttactagtacgtctctcaaggataagtaagtaatattaaggtacgggaggtattggacaggccgcaataaaatatctttattttcattacatctgtgtgttggttttttgtgtgaatcgatagtactaacatacgctctccatcaaaacaaaacgaaacaaaacaaactagcaaaataggctgtccccagtgcaagtgcaggtgccagaacatttctct

SEQ ID NO: 42 - DNA, 30 bp, Artificial Sequence
  Oligonucleotide HTNFHind3-Fv
aagctgaagcttcaccatggcctgggtgtg

SEQ ID NO: 43 - DNA, 30 bp, Artificial Sequence
  Oligonucleotide RitH-Mlu1Rv
gagctcacgcgttcatttacccggagacag

SEQ ID NO: 44 - DNA, 6794 bp, Artificial Sequence
  Plasmid pHQG9
gacggatcgggagatctcccgatcccctatggtgcactctcagtacaatctgctctgatgccgcatagttaagccagtatctgctccctgcttgtgtgttggaggtcgctgagtagtgcgcgagcaaaatttaagctacaacaaggcaaggcttgaccgacaattgcatgaagaatctgcttagggttaggcgttttgcgctgcttcgcgatgtacgggccagatatacgcgttgacattgattattgactagttattaatagtaatcaattacggggtcattagttcatagcccatatatggagttccgcgttacataacttacggtaaatggcccgcctggctgaccgcccaacgacccccgcccattgacgtcaataatgacgtatgttcccatagtaacgccaatagggactttccattgacgtcaatgggtggagtatttacggtaaactgcccacttggcagtacatcaagtgtatcatatgccaagtacgccccctattgacgtcaatgacggtaaatggcccgcctggcattatgcccagtacatgaccttatgggactttcctacttggcagtacatctacgtattagtcatcgctattaccatggtgatgcggttttggcagtacatcaatgggcgtggatagcggtttgactcacggggatttccaagtctccaccccattgacgtcaatgggagtttgttttggcaccaaaatcaacgggactttccaaaatgtcgtaacaactccgccccattgacgcaaatgggcggtaggcgtgtacggtgggaggtctatataagcagagctctctggctaactagagaacccactgcttactggcttatcgaaattaatacgactcactatagggagacccaagctggctagccaccatggcctgggtgtggaccttgcttttcctgatgacagctgcccagagtgcccaagcacagatccagttggaacagtctggacctgagctgaagaagcctggagagacagtcaagatctcctgcaaggcttctggatatatcttcacaaacaatggaatgagctgggtgaaacaggctccaggaaagggtttaaagtggatgggctgggtaaacacctacactggtaagtcaacatatgctgatgacttcaagggacggtttgccttctctttggaaacctcagccagcactgcctatttgcaaatcaacaacctcaaaaatgaggacacggctacatatttctgtgcaagagactctactacggtaatagctacgaatgctatggacttctggggtcaaggaacctcagtcaccgtctcctcagcctcaaccaagggcccatcggtcttccccctggcaccctcctccaagagcacctctgggggcacagcggccctgggctgcctggtcaaggactacttccccgaaccggtgacggtgtcgtggaactcaggcgccctgaccagcggcgtgcacaccttcccggctgtcctacagtcctcaggactctactccctcagcagcgtggtgaccgtgccctccagcagcttgggcacccagacctacatctgcaacgtgaatcacaagcccagcaacaccaaggtggacaagaaagttgagcccaaatcttgtgacaaaactcacacatgcccaccgtgcccagcacctgaactcctggggggaccgtcagtcttcctcttccccccaaaacccaaggacaccctcatgatctcccggacccctgaggtcacatgcgtggtggtggacgtgagccacgaagaccctgaggtcaagttcaactggtacgtggacggcgtggaggtgcataatgccaagacaaagccgcgggaggagcagtacaacagcacgtaccgtgtggtcagcgtcctcaccgtcctgcaccaggactggctgaatggcaaggagtacaagtgcaaggtctccaacaaagccctcccagcccccatcgagaaaaccatctccaaagccaaagggcagccccgagaaccacaggtgtacaccctgcccccatcccgggatgagctgaccaagaaccaggtcagcctgacctgcctggtcaaaggcttctatcccagcgacatcgccgtggagtgggagagcaatgggcagccggagaacaactacaagaccacgcctcccgttctggactccgacggctccttcttcctctacagcaagctcaccgtggacaagagcaggtggcagcaggggaacgtcttctcatgctccgtgatgcatgaggctctgcacaaccactacacacagaagagcctctccctgtctccgggtaaatgaggatcccaccacactggactagtggatccgagctcggtaccaagcttaagtttaaaccgctgatcagcctcgactgtgccttctagttgccagccatctgttgtttgcccctcccccgtgccttccttgaccctggaaggtgccactcccactgtcctttcctaataaaatgaggaaattgcatcgcattgtctgagtaggtgtcattctattctggggggtggggtggggcaggacagcaagggggaggattgggaagacaatagcaggcatgctggggatgcggtgggctctatggcttctgaggcggaaagaaccagctggggctctagggggtatccccacgcgccctgtagcggcgcattaagcgcggcgggtgtggtggttacgcgcagcgtgaccgctacacttgccagcgccctagcgcccgctcctttcgctttcttcccttcctttctcgccacgttcgccggctttccccgtcaagctctaaatcgggggctccctttagggttccgatttagtgctttacggcacctcgaccccaaaaaacttgattagggtgatggttcacgtagtgggccatcgccctgatagacggtttttcgccctttgacgttggagtccacgttctttaatagtggactcttgttccaaactggaacaacactcaaccctatctcggtctattcttttgatttataagggattttgccgatttcggcctattggttaaaaaatgagctgatttaacaaaaatttaacgcgaattaattctgtggaatgtgtgtcagttagggtgtggaaagtccccaggctccccagcaggcagaagtatgcaaagcatgcatctcaattagtcagcaaccaggtgtggaaagtccccaggctccccagcaggcagaagtatgcaaagcatgcatctcaattagtcagcaaccatagtcccgcccctaactccgcccatcccgcccctaactccgcccagttccgcccattctccgccccatggctgactaattttttttatttatgcagaggccgaggccgcctctgcctctgagctattccagaagtagtgaggaggcttttttggaggcctaggcttttgcaaaaagctcccgggagcttgtatatccattttcggatctgatcaagagacaggatgaggatcgtttcgcatgattgaacaagatggattgcacgcaggttctccggccgcttgggtggagaggctattcggctatgactgggcacaacagacaatcggctgctctgatgccgccgtgttccggctgtcagcgcaggggcgcccggttctttttgtcaagaccgacctgtccggtgccctgaatgaactgcaggacgaggcagcgcggctatcgtggctggccacgacgggcgttccttgcgcagctgtgctcgacgttgtcactgaagcgggaagggactggctgctattgggcgaagtgccggggcaggatctcctgtcatctcaccttgctcctgccgagaaagtatccatcatggctgatgcaatgcggcggctgcatacgcttgatccggctacctgcccattcgaccaccaagcgaaacatcgcatcgagcgagcacgtactcggatggaagccggtcttgtcgatcaggatgatctggacgaagagcatcaggggctcgcgccagccgaactgttcgccaggctcaaggcgcgcatgcccgacggcgaggatctcgtcgtgacccatggcgatgcctgcttgccgaatatcatggtggaaaatggccgcttttctggattcatcgactgtggccggctgggtgtggcggaccgctatcaggacatagcgttggctacccgtgatattgctgaagagcttggcggcgaatgggctgaccgcttcctcgtgctttacggtatcgccgctcccgattcgcagcgcatcgccttctatcgccttcttgacgagttcttctgagcgggactctggggttcgaaatgaccgaccaagcgacgcccaacctgccatcacgagatttcgattccaccgccgccttctatgaaaggttgggcttcggaatcgttttccgggacgccggctggatgatcctccagcgcggggatctcatgctggagttcttcgcccaccccaacttgtttattgcagcttataatggttacaaataaagcaatagcatcacaaatttcacaaataaagcatttttttcactgcattctagttgtggtttgtccaaactcatcaatgtatcttatcatgtctgtataccgtcgacctctagctagagcttggcgtaatcatggtcatagctgtttcctgtgtgaaattgttatccgctcacaattccacacaacatacgagccggaagcataaagtgtaaagcctggggtgcctaatgagtgagctaactcacattaattgcgttgcgctcactgcccgctttccagtcgggaaacctgtcgtgccagctgcattaatgaatcggccaacgcgcggggagaggcggtttgcgtattgggcgctcttccgcttcctcgctcactgactcgctgcgctcggtcgttcggctgcggcgagcggtatcagctcactcaaaggcggtaatacggttatccacagaatcaggggataacgcaggaaagaacatgtgagcaaaaggccagcaaaaggccaggaaccgtaaaaaggccgcgttgctggcgtttttccataggctccgcccccctgacgagcatcacaaaaatcgacgctcaagtcagaggtggcgaaacccgacaggactataaagataccaggcgtttccccctggaagctccctcgtgcgctctcctgttccgaccctgccgcttaccggatacctgtccgcctttctcccttcgggaagcgtggcgctttctcatagctcacgctgtaggtatctcagttcggtgtaggtcgttcgctccaagctgggctgtgtgcacgaaccccccgttcagcccgaccgctgcgccttatccggtaactatcgtcttgagtccaacccggtaagacacgacttatcgccactggcagcagccactggtaacaggattagcagagcgaggtatgtaggcggtgctacagagttcttgaagtggtggcctaactacggctacactagaagaacagtatttggtatctgcgctctgctgaagccagttaccttcggaaaaagagttggtagctcttgatccggcaaacaaaccaccgctggtagcggtttttttgtttgcaagcagcagattacgcgcagaaaaaaaggatctcaagaagatcctttgatcttttctacggggtctgacgctcagtggaacgaaaactcacgttaagggattttggtcatgagattatcaaaaaggatcttcacctagatccttttaaattaaaaatgaagttttaaatcaatctaaagtatatatgagtaaacttggtctgacagttaccaatgcttaatcagtgaggcacctatctcagcgatctgtctatttcgttcatccatagttgcctgactccccgtcgtgtagataactacgatacgggagggcttaccatctggccccagtgctgcaatgataccgcgagacccacgctcaccggctccagatttatcagcaataaaccagccagccggaagggccgagcgcagaagtggtcctgcaactttatccgcctccatccagtctattaattgttgccgggaagctagagtaagtagttcgccagttaatagtttgcgcaacgttgttgccattgctacaggcatcgtggtgtcacgctcgtcgtttggtatggcttcattcagctccggttcccaacgatcaaggcgagttacatgatcccccatgttgtgcaaaaaagcggttagctccttcggtcctccgatcgttgtcagaagtaagttggccgcagtgttatcactcatggttatggcagcactgcataattctcttactgtcatgccatccgtaagatgcttttctgtgactggtgagtactcaaccaagtcattctgagaatagtgtatgcggcgaccgagttgctcttgcccggcgtcaatacgggataataccgcgccacatagcagaactttaaaagtgctcatcattggaaaacgttcttcggggcgaaaactctcaaggatcttaccgctgttgagatccagttcgatgtaacccactcgtgcacccaactgatcttcagcatcttttactttcaccagcgtttctgggtgagcaaaaacaggaaggcaaaatgccgcaaaaaagggaataagggcgacacggaaatgttgaatactcatactcttcctttttcaatattattgaagcatttatcagggttattgtctcatgagcggatacatatttgaatgtatttagaaaaataaacaaataggggttccgcgcacatttccccgaaaagtgccacctgacgtc

SEQ ID NO: 45 - DNA, 5775 bp, Artificial Sequence
  Plasmid pKQG9
gacggatcgggagatctcccgatcccctatggtcgactctcagtacaatctgctctgatgccgcatagttaagccagtatctgctccctgcttgtgtgttggaggtcgctgagtagtgcgcgagcaaaatttaagctacaacaaggcaaggcttgaccgacaattgcatgaagaatctgcttagggttaggcgttttgcgctgcttcgcgatgtacgggccagatatacgcgttgacattgattattgactagttattaatagtaatcaattacggggtcattagttcatagcccatatatggagttccgcgttacataacttacggtaaatggcccgcctggctgaccgcccaacgacccccgcccattgacgtcaataatgacgtatgttcccatagtaacgccaatagggactttccattgacgtcaatgggtggactatttacggtaaactgcccacttggcagtacatcaagtgtatcatatgccaagtacgccccctattgacgtcaatgacggtaaatggcccgcctggcattatgcccagtacatgaccttatgggactttcctacttggcagtacatctacgtattagtcatcgctattaccatggtgatgcggttttggcagtacatcaatgggcgtggatagcggtttgactcacggggatttccaagtctccaccccattgacgtcaatgggagtttgttttggcaccaaaatcaacgggactttccaaaatgtcgtaacaactccgccccattgacgcaaatgggcggtaggcgtgtacggtgggaggtctatataagcagagctctctggctaactagagaacccactgcttactggcttatcgaaattaatacgactcactatagggagacccaagctggctagcaacatggattcacaggcccaggttcttatattgctgctgctatgggtatctggtacctgtggggacattgtgatgtcacagtctccatcctccctggctgtgtcagcaggagagaaggtcactatgagctgcaaatccagtcagagtctgctcaacagtagaacccgaaagaactacttggcttggtaccagcagaaaccagggcagtctcctaaactgctgatctactgggcatccattagggaatctggggtccctgatcgcttcacaggcagtggatctgggacagatttcactctcaccatcagcagtgtgcaggctgaagacctggcagtttattactgcaagcaatcttataatctgtggacgttcggtggaggcaccaagctggaaatcaaacggactgttgcggcaccatctgtcttcatcttcccgccatctgatgagcagttgaaatctggaactgcctctgttgtgtgcctgctgaataacttctatcccagagaggccaaagtacagtggaaggtggataacgccctccaatcgggtaactcccaggagagtgtcacagagcaggacagcaaggacagcacctacagcctcagcagcaccctgacgctgagcaaagcagactacgagaaacacaaagtctacgcctgcgaagtcacccatcagggcctgagctcgcccgtcacaaagagcttcaacaggggagagtgttgaggatccactagtccagtgtggtggaattctgcagatatccagcacagtggcggccgctcgagtctagagggcccgaacaaaaactcatctcagaagaggatctgaatagcgccgtcgaccatcatcatcatcatcattgagtttaaacccgctgatcagcctcgactgtgccttctagttgccagccatctgttgtttgcccctcccccgtgccttccttgaccctggaaggtgccactcccactgtcctttcctaataaaatgaggaaattgcatcgcattgtctgagtaggtgtcattctattctggggggtggggtggggcaggacagcaagggggaggattgggaagacaatagcaggcatgctggggatgcggtgggctctatggcttctgaggcggaaagaaccagctggggctctagggggtatccccacgcgccctgtagcggcgcattaagcgcggcgggtgtggtggttacgcgcagcgtgaccgctacacttgccagcgccctagcgcccgctcctttcgctttcttcccttcctttctcgccacgttcgccggctttccccgtcaagctctaaatcggggcatccctttagggttccgatttagtgctttacggcacctcgaccccaaaaaacttgattagggtgatggttcacgtagtgggccatcgccctgatagacggtttttcgccctttgacgttggagtccacgttctttaatagtggactcttgttccaaactggaacaacactcaaccctatctcggtctattcttttgatttataagggattttggggatttcggcctattggttaaaaaatgagctgatttaacaaaaatttaacgcgaattaattctgtggaatgtgtgtcagttagggtgtggaaagtccccaggctccccagcaggcagaagtatgcaaagcatgcatctcaattagtcagcaaccaggtgtggaaagtccccaggctccccagcaggcagaagtatgcaaagcatgcatctcaattagtcagcaaccatagtcccgcccctaactccgcccatcccgcccctaactccgcccagttccgcccattctccgccccatggctgactaattttttttatttatgcagaggccgaggccgcctctgcctctgagctattccagaagtagtgaggaggcttttttggaggcctaggcttttgcaaaaagctcccgggagcttgtatatccattttcggatctgatcagcacgtgttgacaattaatcatcggcatagtatatcggcatagtataatacgacaaggtgaggaactaaaccatggccaagttgaccagtgccgttccggtgctcaccgcgcgcgacgtcgccggagcggtcgagttctggaccgaccggctcgggttctcccgggacttcgtggaggacgacttcgccggtgtggtccgggacgacgtgaccctgttcatcagcgcggtccaggaccaggtggtgccggacaacaccctggcctgggtgtgggtgcgcggcctggacgagctgtacgccgagtggtcggaggtcgtgtccacgaacttccgggacgcctccgggccggccatgaccgagatcggcgagcagccgtgggggcgggagttcgccctgcgcgacccggccggcaactgcgtgcacttcgtggccgaggagcaggactgacacgtgctacgagatttcgattccaccgccgccttctatgaaaggttgggcttcggaatcgttttccgggacgccggctggatgatcctccagcgcggggatctcatgctggagttcttcgcccaccccaacttgtttattgcagcttataatggttacaaataaagcaatagcatcacaaatttcacaaataaagcatttttttcactgcattctagttgtggtttgtccaaactcatcaatgtatcttatcatgtctgtataccgtcgacctctagctagagcttggcgtaatcatggtcatagctgtttcctgtgtgaaattgttatccgctcacaattccacacaacatacgagccggaagcataaagtgtaaagcctggggtgcctaatgagtgagctaactcacattaattgcgttgcgctcactgcccgctttccagtcgggaaacctgtcgtgccagctgcattaatgaatcggccaacgcgcggggagaggcggtttgcgtattgggcgctcttccgcttcctcgctcactgactcgctgcgctcggtcgttcggctgcggcgagcggtatcagctcactcaaaggcggtaatacggttatccacagaatcaggggataacgcaggaaagaacatgtgagcaaaaggccagcaaaaggccaggaaccgtaaaaaggccgcgttgctggcgtttttccataggctccgcccccctgacgagcatcacaaaaatcgacgctcaagtcagaggtggcgaaacccgacaggactataaagataccaggcgtttccccctggaagctccctcgtgcgctctcctgttccgaccctgccgcttaccggatacctgtccgcctttctcccttcgggaagcgtggcgctttctcaatgctcacgctgtaggtatctcagttcggtgtaggtcgttcgctccaagctgggctgtgtgcacgaaccccccgttcagcccgaccgctgcgccttatccggtaactatcgtcttgagtccaacccggtaagacacgacttatcgccactggcagcagccactggtaacaggattagcagagcgaggtatgtaggcggtgctacagagttcttgaagtggtggcctaactacggctacactagaaggacagtatttggtatctgcgctctgctgaagccagttaccttcggaaaaagagttggtagctcttgatccggcaaacaaaccaccgctggtagcggtggtttttttgtttgcaagcagcagattacgcgcagaaaaaaaggatctcaagaagatcctttgatcttttctacggggtctgacgctcagtggaacgaaaactcacgttaagggattttggtcatgagattatcaaaaaggatcttcacctagatccttttaaattaaaaatgaagttttaaatcaatctaaagtatatatgagtaaacttggtctgacagttaccaatgcttaatcagtgaggcacctatctcagcgatctgtctatttcgttcatccatagttgcctgactccccgtcgtgtagataactacgatacgggagggcttaccatctggccccagtgctgcaatgataccgcgagacccacgctcaccggctccagatttatcagcaataaaccagccagccggaagggccgagcgcagaagtggtcctgcaactttatccgcctccatccagtctattaattgttgccgggaagctagagtaagtagttcgccagttaatagtttgcgcaacgttgttgccattgctacaggcatcgtggtgtcacgctcgtcgtttggtatggcttcattcagctccggttcccaacgatcaaggcgagttacatgatcccccatgttgtgcaaaaaagcggttagctccttcggtcctccgatcgttgtcagaagtaagttggccgcagtgttatcactcatggttatggcagcactgcataattctcttactgtcatgccatccgtaagatgcttttctgtgactggtgagtactcaaccaagtcattctgagaatagtgtatgcggcgaccgagttgctcttgcccggcgtcaatacgggataataccgcgccacatagcagaactttaaaagtgctcatcattggaaaacgttcttcggggcgaaaactctcaaggatcttaccgctgttgagatccagttcgatgtaacccactcgtgcacccaactgatcttcagcatcttttactttcaccagcgtttctgggtgagcaaaaacaggaaggcaaaatgccgcaaaaaagggaataagggcgacacggaaatgttgaatactcatactcttcctttttcaatattattgaagcatttatcagggttattgtctcatgagcggatacatatttgaatgtatttagaaaaataaacaaataggggttccgcgcacatttccccgaaaagtgccacctgacgtc